European Patent Specification EP 3 417 880 B1, published February 19, 2025. Title: RNA-GUIDED GENE EDITING AND GENE REGULATION. Applicant: DUKE UNIVERSITY. Application not yet assigned. The sequence listing filed with the application follows.

SEQUENCE LISTING (750 sequences)

SEQ ID NO: 1 - protein, 1483 aa, Artificial Sequence
  Description of Artificial Sequence: Synthetic polypeptide
MDYKDHDGDYKDHDIDYKDDDDKMAPKKKRKVGRGMDKKYSIGLAIGTNSVGWAVITDEYKVPSKKFKVLGNTDRHSIKKNLIGALLFDSGETAEATRLKRTARRRYTRRKNRICYLQEIFSNEMAKVDDSFFHRLEESFLVEEDKKHERHPIFGNIVDEVAYHEKYPTIYHLRKKLVDSTDKADLRLIYLALAHMIKFRGHFLIEGDLNPDNSDVDKLFIQLVQTYNQLFEENPINASGVDAKAILSARLSKSRRLENLIAQLPGEKKNGLFGNLIALSLGLTPNFKSNFDLAEDAKLQLSKDTYDDDLDNLLAQIGDQYADLFLAAKNLSDAILLSDILRVNTEITKAPLSASMIKRYDEHHQDLTLLKALVRQQLPEKYKEIFFDQSKNGYAGYIDGGASQEEFYKFIKPILEKMDGTEELLVKLNREDLLRKQRTFDNGSIPHQIHLGELHAILRRQEDFYPFLKDNREKIEKILTFRIPYYVGPLARGNSRFAWMTRKSEETITPWNFEEVVDKGASAQSFIERMTNFDKNLPNEKVLPKHSLLYEYFTVYNELTKVKYVTEGMRKPAFLSGEQKKAIVDLLFKTNRKVTVKQLKEDYFKKIECFDSVEISGVEDRFNASLGTYHDLLKIIKDKDFLDNEENEDILEDIVLTLTLFEDREMIEERLKTYAHLFDDKVMKQLKRRRYTGWGRLSRKLINGIRDKQSGKTILDFLKSDGFANRNFMQLIHDDSLTFKEDIQKAQVSGQGDSLHEHIANLAGSPAIKKGILQTVKVVDELVKVMGRHKPENIVIEMARENQTTQKGQKNSRERMKRIEEGIKELGSQILKEHPVENTQLQNEKLYLYYLQNGRDMYVDQELDINRLSDYDVDAIVPQSFLKDDSIDNKVLTRSDKNRGKSDNVPSEEVVKKMKNYWRQLLNAKLITQRKFDNLTKAERGGLSELDKAGFIKRQLVETRQITKHVAQILDSRMNTKYDENDKLIREVKVITLKSKLVSDFRKDFQFYKVREINNYHHAHDAYLNAVVGTALIKKYPKLESEFVYGDYKVYDVRKMIAKSEQEIGKATAKYFFYSNIMNFFKTEITLANGEIRKRPLIETNGETGEIVWDKGRDFATVRKVLSMPQVNIVKKTEVQTGGFSKESILPKRNSDKLIARKKDWDPKKYGGFDSPTVAYSVLVVAKVEKGKSKKLKSVKELLGITIMERSSFEKNPIDFLEAKGYKEVKKDLIIKLPKYSLFELENGRKRMLASAGELQKGNELALPSKYVNFLYLASHYEKLKGSPEDNEQKQLFVEQHKHYLDEIIEQISEFSKRVILADANLDKVLSAYNKHRDKPIREQAENIIHLFTLTNLGAPAAFKYFDTTIDRKRYTSTKEVLDATLIHQSITGLYETRIDLSQLGGDPIAGSKASPKKKRKVGRADALDDFDLDMLGSDALDDFDLDMLGSDALDDFDLDMLGSDALDDFDLDMLINYPYDVPDYAS

SEQ ID NO: 2 - DNA, 350 bp, Artificial Sequence
  Description of Artificial Sequence: Synthetic polynucleotide
gagggcctatttcccatgattccttcatatttgcatatacgatacaaggctgttagagagataattggaattaatttgactgtaaacacaaagatattagtacaaaatacgtgacgtagaaagtaataatttcttgggtagtttgcagttttaaaattatgttttaaaatggactatcatatgcttatcgtaacttgaaagtatttcgatttcttggctttatatatcttgtggaaaggacgaaacaccgggtcttcgagaagacctgttttagagctagaaatagcaagttaaaataaggctagtccgttatcaacttgaaaaagtggcaccgagtcggtgcttttttt

SEQ ID NO: 3 - DNA, 338 bp, Homo sapiens
acccccggcagcagcccgccccgagcgcgccgcctgtttattcagccgggagtccggcacgcgccaggcgcacgcactgcaacaacaaacccagctgaatggagagtttgcaaggagcgggagaaaggaacgggagggggggagaggagaggaggagggggagtttagggagtgggtgggaggaagaggtaagaggaggggggggagtgggggctgcagccgctcgctgcagcagcggggagtggggggcgaggcggggccagggctgcgcgtggggctgggtgtcccattgaaaaggcggacgcactccggcagcccagcactctctcacttctggc

SEQ ID NO: 4 - DNA, 305 bp, Mus musculus
ccgccccgagcgcgcggcctgtttattcagccgggagtccggcacgcgccgggcgcacgcactgcaacaacaaaccaggctgaatggagagtttgcaaggagcgggcgcgggcaactggagggggggggggcgagagggagggagctgaggaggtgggggaagaggaggggtagtgggggctgcagccgctcgctgcagcagcggggagtggggggcgaggcggggccagggctgcgcgtggggctgggtgtcccattgaaaaggcggccgcaccgcagccgcccagcagtctctcacttctggc

SEQ ID NO: 5 - DNA, 19 bp, Artificial Sequence
  Description of Artificial Sequence: Synthetic oligonucleotide
gctgggtgtcccattgaaa

SEQ ID NO: 6 - DNA, 19 bp, Artificial Sequence
  Description of Artificial Sequence: Synthetic oligonucleotide
cagccgctcgctgcagcag

SEQ ID NO: 7 - DNA, 19 bp, Artificial Sequence
  Description of Artificial Sequence: Synthetic oligonucleotide
tggagagtttgcaaggagc

SEQ ID NO: 8 - DNA, 19 bp, Artificial Sequence
  Description of Artificial Sequence: Synthetic oligonucleotide
gtttattcagccgggagtc

SEQ ID NO: 9 - DNA, 20 bp, Artificial Sequence
  Description of Artificial Sequence: Synthetic oligonucleotide
cgccaggaggggtgggtcta

SEQ ID NO: 10 - DNA, 19 bp, Artificial Sequence
  Description of Artificial Sequence: Synthetic oligonucleotide
ccttggtgagactggtaga

SEQ ID NO: 11 - DNA, 19 bp, Artificial Sequence
  Description of Artificial Sequence: Synthetic oligonucleotide
gtcttcaggttctgttgct

SEQ ID NO: 12 - DNA, 19 bp, Artificial Sequence
  Description of Artificial Sequence: Synthetic oligonucleotide
atattcctgatttaaaagt

SEQ ID NO: 13 - DNA, 19 bp, Artificial Sequence
  Description of Artificial Sequence: Synthetic oligonucleotide
ttaaaagtcggctggtagc

SEQ ID NO: 14 - DNA, 19 bp, Artificial Sequence
  Description of Artificial Sequence: Synthetic oligonucleotide
cgggccgggggcggggtcc

SEQ ID NO: 15 - DNA, 19 bp, Artificial Sequence
  Description of Artificial Sequence: Synthetic oligonucleotide
gcccgagccgcgtgtggaa

SEQ ID NO: 16 - DNA, 19 bp, Artificial Sequence
  Description of Artificial Sequence: Synthetic oligonucleotide
ccttcattgcggcgggctg

SEQ ID NO: 17 - DNA, 19 bp, Artificial Sequence
  Description of Artificial Sequence: Synthetic oligonucleotide
ccgacccctcccgggtccc

SEQ ID NO: 18 - DNA, 19 bp, Artificial Sequence
  Description of Artificial Sequence: Synthetic oligonucleotide
caggaccgcgcttcccacg

SEQ ID NO: 19 - DNA, 19 bp, Artificial Sequence
  Description of Artificial Sequence: Synthetic oligonucleotide
tgcaccctgggagcgcgag

SEQ ID NO: 20 - DNA, 19 bp, Artificial Sequence
  Description of Artificial Sequence: Synthetic oligonucleotide
ccgcacgcacctgttccca

SEQ ID NO: 21 - DNA, 19 bp, Artificial Sequence
  Description of Artificial Sequence: Synthetic oligonucleotide
aaaacagcgagggagaaac

SEQ ID NO: 22 - DNA, 19 bp, Artificial Sequence
  Description of Artificial Sequence: Synthetic oligonucleotide
ttaacttgattgtgaaatc

SEQ ID NO: 23 - DNA, 19 bp, Artificial Sequence
  Description of Artificial Sequence: Synthetic oligonucleotide
aaaacaatgcatatttgca

SEQ ID NO: 24 - DNA, 19 bp, Artificial Sequence
  Description of Artificial Sequence: Synthetic oligonucleotide
aaaatccagtattttaatg

SEQ ID NO: 25 - DNA, 19 bp, Artificial Sequence
  Description of Artificial Sequence: Synthetic oligonucleotide
acccagcactgcagcctgg

SEQ ID NO: 26 - DNA, 19 bp, Artificial Sequence
  Description of Artificial Sequence: Synthetic oligonucleotide
aacttatgcggcgtttcct

SEQ ID NO: 27 - DNA, 19 bp, Artificial Sequence
  Description of Artificial Sequence: Synthetic oligonucleotide
tcactttaaaaccacctct

SEQ ID NO: 28 - DNA, 19 bp, Artificial Sequence
  Description of Artificial Sequence: Synthetic oligonucleotide
gcatctttttctctttaat

SEQ ID NO: 29 - DNA, 19 bp, Artificial Sequence
  Description of Artificial Sequence: Synthetic oligonucleotide
tgtactctctgaggtgctc

SEQ ID NO: 30 - DNA, 19 bp, Artificial Sequence
  Description of Artificial Sequence: Synthetic oligonucleotide
acgcagataagaaccagtt

SEQ ID NO: 31 - DNA, 19 bp, Artificial Sequence
  Description of Artificial Sequence: Synthetic oligonucleotide
catcaagtcagccatcagc

SEQ ID NO: 32 - DNA, 19 bp, Artificial Sequence
  Description of Artificial Sequence: Synthetic oligonucleotide
gagtcaccctcctggaaac

SEQ ID NO: 33 - DNA, 19 bp, Artificial Sequence
  Description of Artificial Sequence: Synthetic oligonucleotide
gctagggatgaagaataaa

SEQ ID NO: 34 - DNA, 19 bp, Artificial Sequence
  Description of Artificial Sequence: Synthetic oligonucleotide
ttgaccaatagccttgaca

SEQ ID NO: 35 - DNA, 19 bp, Artificial Sequence
  Description of Artificial Sequence: Synthetic oligonucleotide
tgcaaatatctgtctgaaa

SEQ ID NO: 36 - DNA, 19 bp, Artificial Sequence
  Description of Artificial Sequence: Synthetic oligonucleotide
aaattagcagtatcctctt

SEQ ID NO: 37 - DNA, 19 bp, Artificial Sequence
  Description of Artificial Sequence: Synthetic oligonucleotide
cctgggctccggggcgttt

SEQ ID NO: 38 - DNA, 19 bp, Artificial Sequence
  Description of Artificial Sequence: Synthetic oligonucleotide
ggcccctgcggccaccccg

SEQ ID NO: 39 - DNA, 19 bp, Artificial Sequence
  Description of Artificial Sequence: Synthetic oligonucleotide
ctccctccctgcccggtag

SEQ ID NO: 40 - DNA, 19 bp, Artificial Sequence
  Description of Artificial Sequence: Synthetic oligonucleotide
aggtttggaaagggcgtgc

SEQ ID NO: 41 - DNA, 20 bp, Artificial Sequence
  Description of Artificial Sequence: Synthetic primer
ggagcttctcgacttcacca

SEQ ID NO: 42 - DNA, 20 bp, Artificial Sequence
  Description of Artificial Sequence: Synthetic primer
gatttgtgggcctgaagaaa

SEQ ID NO: 43 - DNA, 20 bp, Artificial Sequence
  Description of Artificial Sequence: Synthetic primer
aaggaggagggcagaatcat

SEQ ID NO: 44 - DNA, 21 bp, Artificial Sequence
  Description of Artificial Sequence: Synthetic primer
aaaccttcctcagctatgccc

SEQ ID NO: 45 - DNA, 20 bp, Artificial Sequence
  Description of Artificial Sequence: Synthetic primer
agctgatggccctaaacaga

SEQ ID NO: 46 - DNA, 20 bp, Artificial Sequence
  Description of Artificial Sequence: Synthetic primer
caggaggactctggcaccta

SEQ ID NO: 47 - DNA, 20 bp, Artificial Sequence
  Description of Artificial Sequence: Synthetic primer
ggaatccatggagggaagat

SEQ ID NO: 48 - DNA, 21 bp, Artificial Sequence
  Description of Artificial Sequence: Synthetic primer
gctgagtgaactgcactgtga

SEQ ID NO: 49 - DNA, 20 bp, Artificial Sequence
  Description of Artificial Sequence: Synthetic primer
ctctctgctcctttgccaca

SEQ ID NO: 50 - DNA, 20 bp, Artificial Sequence
  Description of Artificial Sequence: Synthetic primer
caatgaccccttcattgacc

SEQ ID NO: 51 - DNA, 20 bp, Artificial Sequence
  Description of Artificial Sequence: Synthetic primer
ggaacaagagctgctggact

SEQ ID NO: 52 - DNA, 20 bp, Artificial Sequence
  Description of Artificial Sequence: Synthetic primer
aactttggcattgtggaagg

SEQ ID NO: 53 - DNA, 20 bp, Artificial Sequence
  Description of Artificial Sequence: Synthetic primer
aacgccactgacaagaaagc

SEQ ID NO: 54 - DNA, 20 bp, Artificial Sequence
  Description of Artificial Sequence: Synthetic primer
cagatccatggaggaaggaa

SEQ ID NO: 55 - DNA, 21 bp, Artificial Sequence
  Description of Artificial Sequence: Synthetic primer
gggtactcctggaagatgtcc

SEQ ID NO: 56 - DNA, 20 bp, Artificial Sequence
  Description of Artificial Sequence: Synthetic primer
gtttgcgacgcatgttcctc

SEQ ID NO: 57 - DNA, 20 bp, Artificial Sequence
  Description of Artificial Sequence: Synthetic primer
aagcccttgctgtagtggtg

SEQ ID NO: 58 - DNA, 20 bp, Artificial Sequence
  Description of Artificial Sequence: Synthetic primer
cggcaggaaagcatctgtat

SEQ ID NO: 59 - DNA, 20 bp, Artificial Sequence
  Description of Artificial Sequence: Synthetic primer
tgttctcgctcaggtcagtg

SEQ ID NO: 60 - DNA, 20 bp, Artificial Sequence
  Description of Artificial Sequence: Synthetic primer
gaattctttgccgaaatgga

SEQ ID NO: 61 - DNA, 20 bp, Artificial Sequence
  Description of Artificial Sequence: Synthetic primer
gtgctcttcgggtttcagga

SEQ ID NO: 62 - DNA, 20 bp, Artificial Sequence
  Description of Artificial Sequence: Synthetic primer
ttgattttggagggatctcg

SEQ ID NO: 63 - DNA, 20 bp, Artificial Sequence
  Description of Artificial Sequence: Synthetic primer
gtttttctgcctccccattt

SEQ ID NO: 64 - DNA, 20 bp, Artificial Sequence
  Description of Artificial Sequence: Synthetic primer
ggatgcagggatgatgttct

SEQ ID NO: 65 - DNA, 20 bp, Artificial Sequence
  Description of Artificial Sequence: Synthetic oligonucleotide
gattggctttgatttcccta

SEQ ID NO: 66 - DNA, 23 bp, Artificial Sequence
  Description of Artificial Sequence: Synthetic oligonucleotide
gtgtagagtaagtcagcctatgg

SEQ ID NO: 67 - DNA, 20 bp, Artificial Sequence
  Description of Artificial Sequence: Synthetic oligonucleotide
gcctactcagactgttactc

SEQ ID NO: 68 - DNA, 23 bp, Artificial Sequence
  Description of Artificial Sequence: Synthetic oligonucleotide
gttggacagaacttaccgactgg

SEQ ID NO: 69 - DNA, 20 bp, Artificial Sequence
  Description of Artificial Sequence: Synthetic oligonucleotide
gcagttgcctaagaactggt

SEQ ID NO: 70 - DNA, 20 bp, Artificial Sequence
  Description of Artificial Sequence: Synthetic oligonucleotide
ggggctccaccctcacgagt

SEQ ID NO: 71 - DNA, 23 bp, Artificial Sequence
  Description of Artificial Sequence: Synthetic oligonucleotide
gtttgcttcgctataaaacgagg

SEQ ID NO: 72 - DNA, 23 bp, Artificial Sequence
  Description of Artificial Sequence: Synthetic oligonucleotide
gtctgaggatggggccgcaatgg

SEQ ID NO: 73 - DNA, 23 bp, Artificial Sequence
  Description of Artificial Sequence: Synthetic oligonucleotide
ggatctgtcaaatcgcctgcagg

SEQ ID NO: 74 - DNA, 23 bp, Artificial Sequence
  Description of Artificial Sequence: Synthetic oligonucleotide
gccaggatggcattgggcagcgg

SEQ ID NO: 75 - DNA, 23 bp, Artificial Sequence
  Description of Artificial Sequence: Synthetic oligonucleotide
gctgaatctgcggtggcaggagg

SEQ ID NO: 76 - DNA, 23 bp, Artificial Sequence
  Description of Artificial Sequence: Synthetic oligonucleotide
gttcttttgttcttctagcctgg

SEQ ID NO: 77 - DNA, 23 bp, Artificial Sequence
  Description of Artificial Sequence: Synthetic oligonucleotide
ggaaaagcttgagcaagtcaagg

SEQ ID NO: 78 - DNA, 23 bp, Artificial Sequence
  Description of Artificial Sequence: Synthetic oligonucleotide
ggaagagttgcccctgcgccagg

SEQ ID NO: 79 - DNA, 23 bp, Artificial Sequence
  Description of Artificial Sequence: Synthetic oligonucleotide
gacaaatctccagtggataaagg

SEQ ID NO: 80 - DNA, 23 bp, Artificial Sequence
  Description of Artificial Sequence: Synthetic oligonucleotide
gtgtttctcaggtaaagctctgg

SEQ ID NO: 81 - DNA, 23 bp, Artificial Sequence
  Description of Artificial Sequence: Synthetic oligonucleotide
ggaaggaccatttgacgttaagg

SEQ ID NO: 82 - DNA, 23 bp, Artificial Sequence
  Description of Artificial Sequence: Synthetic oligonucleotide
gaactgctatttcagtttcctgg

SEQ ID NO: 83 - DNA, 23 bp, Artificial Sequence
  Description of Artificial Sequence: Synthetic oligonucleotide
gccagccactcagccagtgaagg

SEQ ID NO: 84 - DNA, 23 bp, Artificial Sequence
  Description of Artificial Sequence: Synthetic oligonucleotide
ggtatgcttttctgttaaagagg

SEQ ID NO: 85 - DNA, 23 bp, Artificial Sequence
  Description of Artificial Sequence: Synthetic oligonucleotide
gctcctggactgaccactattgg

SEQ ID NO: 86 - DNA, 23 bp, Artificial Sequence
  Description of Artificial Sequence: Synthetic oligonucleotide
ggaacagaggcgtccccagttgg

SEQ ID NO: 87 - DNA, 23 bp, Artificial Sequence
  Description of Artificial Sequence: Synthetic oligonucleotide
ggaggctagaacaatcattacgg

SEQ ID NO: 88 - DNA, 23 bp, Artificial Sequence
  Description of Artificial Sequence: Synthetic oligonucleotide
gacaagaacaccttcagaaccgg

SEQ ID NO: 89 - DNA, 23 bp, Artificial Sequence
  Description of Artificial Sequence: Synthetic oligonucleotide
gggtttctgtgattttcttttgg

SEQ ID NO: 90 - DNA, 23 bp, Artificial Sequence
  Description of Artificial Sequence: Synthetic oligonucleotide
gggccaaagacctccgccagtgg

SEQ ID NO: 91 - DNA, 23 bp, Artificial Sequence
  Description of Artificial Sequence: Synthetic oligonucleotide
gttggagaagcattcataaaagg

SEQ ID NO: 92 - DNA, 23 bp, Artificial Sequence
  Description of Artificial Sequence: Synthetic oligonucleotide
gtcgctcactcaccctgcaaagg

SEQ ID NO: 93 - DNA, 23 bp, Artificial Sequence
  Description of Artificial Sequence: Synthetic oligonucleotide
gaaaagagctgatgaaacaatgg

SEQ ID NO: 94 - DNA, 23 bp, Artificial Sequence
  Description of Artificial Sequence: Synthetic oligonucleotide
gtacacttttcaaaatgctttgg

SEQ ID NO: 95 - DNA, 23 bp, Artificial Sequence
  Description of Artificial Sequence: Synthetic oligonucleotide
ggagatgatcatcaagcagaagg

SEQ ID NO: 96 - DNA, 23 bp, Artificial Sequence
  Description of Artificial Sequence: Synthetic oligonucleotide
gctttgaaagagcaataaaatgg

SEQ ID NO: 97 - DNA, 23 bp, Artificial Sequence
  Description of Artificial Sequence: Synthetic oligonucleotide
gcacaaaagtcaaatcggaatgg

SEQ ID NO: 98 - DNA, 23 bp, Artificial Sequence
  Description of Artificial Sequence: Synthetic oligonucleotide
gatttcaatataagattcggagg

SEQ ID NO: 99 - DNA, 23 bp, Artificial Sequence
  Description of Artificial Sequence: Synthetic oligonucleotide
gcttaagcaatcccgaactctgg

SEQ ID NO: 100 - DNA, 20 bp, Artificial Sequence
  Description of Artificial Sequence: Synthetic oligonucleotide
gccttctttatcccctatcg

SEQ ID NO: 101-103 - skipped (3 entries)

SEQ ID NO: 104 - DNA, 25 bp, Artificial Sequence
  Description of Artificial Sequence: Synthetic oligonucleotide
  modified_base (21)..(22): a, c, t, g, unknown or other
gaggccaaacctcggcttacnngrr

SEQ ID NO: 105 - DNA, 25 bp, Artificial Sequence
  Description of Artificial Sequence: Synthetic oligonucleotide
  modified_base (21)..(22): a, c, t, g, unknown or other
gttcgaaaatttcaggtaagnngrr

SEQ ID NO: 106 - DNA, 26 bp, Artificial Sequence
  Description of Artificial Sequence: Synthetic oligonucleotide
  modified_base (21)..(22): a, c, t, g, unknown or other
ggcagaacaggagataacagnngrrt

SEQ ID NO: 107 - DNA, 26 bp, Artificial Sequence
  Description of Artificial Sequence: Synthetic oligonucleotide
ggcggccctcgcccttctctggggat

SEQ ID NO: 108 - DNA, 23 bp, Artificial Sequence
  Description of Artificial Sequence: Synthetic oligonucleotide
gtagtgatcgtggatacgagagg

SEQ ID NO: 109 - DNA, 23 bp, Artificial Sequence
  Description of Artificial Sequence: Synthetic oligonucleotide
gtacagccctcggtgtatattgg

SEQ ID NO: 110 - DNA, 23 bp, Artificial Sequence
  Description of Artificial Sequence: Synthetic oligonucleotide
gggaaggaattaagcccgaatgg

SEQ ID NO: 111 - DNA, 23 bp, Artificial Sequence
  Description of Artificial Sequence: Synthetic oligonucleotide
gggaacagctttcgtagttgagg

SEQ ID NO: 112 - DNA, 23 bp, Artificial Sequence
  Description of Artificial Sequence: Synthetic oligonucleotide
gataaagtccagtgtcgatcagg

SEQ ID NO: 113 - DNA, 23 bp, Artificial Sequence
  Description of Artificial Sequence: Synthetic oligonucleotide
gaaaaccagagcttcggtcaagg

SEQ ID NO: 114 - DNA, 34 bp, Artificial Sequence
  Description of Artificial Sequence: Synthetic oligonucleotide
ggagtcttctgggcaggcttaaaggctaacctgg

SEQ ID NO: 115 - DNA, 34 bp, Artificial Sequence
  Description of Artificial Sequence: Synthetic oligonucleotide
gtcgggtgagcatgtctttaatctacctcgatgg

SEQ ID NO: 116 - DNA, 26 bp, Artificial Sequence
  Description of Artificial Sequence: Synthetic oligonucleotide
ggtgtcaccagagtaacagtctgagt

SEQ ID NO: 117 - DNA, 25 bp, Artificial Sequence
  Description of Artificial Sequence: Synthetic oligonucleotide
gtgatcatcaagcagaaggtatgag

SEQ ID NO: 118 - DNA, 29 bp, Artificial Sequence
  Description of Artificial Sequence: Synthetic oligonucleotide
gaacttcgaaaatttcaggtaagccgagg

SEQ ID NO: 119 - DNA, 29 bp, Artificial Sequence
  Description of Artificial Sequence: Synthetic oligonucleotide
ggaaactcatcaaatatgcgtgttagtgt

SEQ ID NO: 120 - DNA, 29 bp, Artificial Sequence
  Description of Artificial Sequence: Synthetic oligonucleotide
gtcatttacactaacacgcatatttgatg

SEQ ID NO: 121 - DNA, 29 bp, Artificial Sequence
  Description of Artificial Sequence: Synthetic oligonucleotide
ggaatgaaactcatcaaatatgcgtgtta

SEQ ID NO: 122 - DNA, 29 bp, Artificial Sequence
  Description of Artificial Sequence: Synthetic oligonucleotide
gtcatcaatatctttgaaggactctgggt

SEQ ID NO: 123 - DNA, 29 bp, Artificial Sequence
  Description of Artificial Sequence: Synthetic oligonucleotide
gtgttttcataggaaaaataggcaagttg

SEQ ID NO: 124 - DNA, 29 bp, Artificial Sequence
  Description of Artificial Sequence: Synthetic oligonucleotide
gaattggaaaatgtgatgggaaacagata

SEQ ID NO: 125 - DNA, 29 bp, Artificial Sequence
  Description of Artificial Sequence: Synthetic oligonucleotide
gatgatcatcaagcagaaggtatgagaaa

SEQ ID NO: 126 - DNA, 29 bp, Artificial Sequence
  Description of Artificial Sequence: Synthetic oligonucleotide
gagatgatcatcaagcagaaggtatgaga

SEQ ID NO: 127 - DNA, 29 bp, Artificial Sequence
  Description of Artificial Sequence: Synthetic oligonucleotide
gcattttttctcataccttctgcttgatg

SEQ ID NO: 128 - DNA, 29 bp, Artificial Sequence
  Description of Artificial Sequence: Synthetic oligonucleotide
gtcctactcagactgttactctggtgaca

SEQ ID NO: 129 - DNA, 29 bp, Artificial Sequence
  Description of Artificial Sequence: Synthetic oligonucleotide
gacaggttgtgtcaccagagtaacagtct

SEQ ID NO: 130 - DNA, 29 bp, Artificial Sequence
  Description of Artificial Sequence: Synthetic oligonucleotide
gttatcattttttctcataccttctgctt

SEQ ID NO: 131 - DNA, 29 bp, Artificial Sequence
  Description of Artificial Sequence: Synthetic oligonucleotide
gttgcctaagaactggtgggaaatggtct

SEQ ID NO: 132 - DNA, 29 bp, Artificial Sequence
  Description of Artificial Sequence: Synthetic oligonucleotide
gaaacagttgcctaagaactggtgggaaa

SEQ ID NO: 133 - DNA, 29 bp, Artificial Sequence
  Description of Artificial Sequence: Synthetic oligonucleotide
gtttcccaccagttcttaggcaactgttt

SEQ ID NO: 134 - DNA, 29 bp, Artificial Sequence
  Description of Artificial Sequence: Synthetic oligonucleotide
gtggctttgatttccctagggtccagctt

SEQ ID NO: 135 - DNA, 29 bp, Artificial Sequence
  Description of Artificial Sequence: Synthetic oligonucleotide
gtagggaaatcaaagccaatgaaacgttc

SEQ ID NO: 136 - DNA, 29 bp, Artificial Sequence
  Description of Artificial Sequence: Synthetic oligonucleotide
ggaccctagggaaatcaaagccaatgaaa

SEQ ID NO: 137 - DNA, 29 bp, Artificial Sequence
  Description of Artificial Sequence: Synthetic oligonucleotide
gtgagggctccaccctcacgagtgggttt

SEQ ID NO: 138 - DNA, 29 bp, Artificial Sequence
  Description of Artificial Sequence: Synthetic oligonucleotide
gaaggattgagggctccaccctcacgagt

SEQ ID NO: 139 - DNA, 29 bp, Artificial Sequence
  Description of Artificial Sequence: Synthetic oligonucleotide
ggctccaccctcacgagtgggtttggttc

SEQ ID NO: 140 - DNA, 29 bp, Artificial Sequence
  Description of Artificial Sequence: Synthetic oligonucleotide
gtatcccctatcgaggaaaccacgagttt

SEQ ID NO: 141 - DNA, 29 bp, Artificial Sequence
  Description of Artificial Sequence: Synthetic oligonucleotide
ggataaagaaggcctatttcatagagttg

SEQ ID NO: 142 - DNA, 29 bp, Artificial Sequence
  Description of Artificial Sequence: Synthetic oligonucleotide
gaggccttctttatcccctatcgaggaaa

SEQ ID NO: 143 - DNA, 27 bp, Artificial Sequence
  Description of Artificial Sequence: Synthetic oligonucleotide
gtgagggctccaccctcacgagtgggt

SEQ ID NO: 144 - DNA, 27 bp, Artificial Sequence
  Description of Artificial Sequence: Synthetic oligonucleotide
ggataaagaaggcctatttcatagagt

SEQ ID NO: 145 - DNA, 4932 bp, Artificial Sequence
  Description of Artificial Sequence: Synthetic polynucleotide
gccaccatggacaagaagtactccattgggctcgatatcggcacaaacagcgtcggctgggccgtcattacggacgagtacaaggtgccgagcaaaaaattcaaagttctgggcaataccgatcgccacagcataaagaagaacctcattggcgccctcctgttcgactccggggagacggccgaagccacgcggctcaaaagaacagcacggcgcagatatacccgcagaaagaatcggatctgctacctgcaggagatctttagtaatgagatggctaaggtggatgactctttcttccataggctggaggagtcctttttggtggaggaggataaaaagcacgagcgccacccaatctttggcaatatcgtggacgaggtggcgtaccatgaaaagtacccaaccatatatcatctgaggaagaagcttgtagacagtactgataaggctgacttgcggttgatctatctcgcgctggcgcatatgatcaaatttcggggacacttcctcatcgagggggacctgaacccagacaacagcgatgtcgacaaactctttatccaactggttcagacttacaatcagcttttcgaagagaacccgatcaacgcatccggagttgacgccaaagcaatcctgagcgctaggctgtccaaatcccggcggctcgaaaacctcatcgcacagctccctggggagaagaagaacggcctgtttggtaatcttatcgccctgtcactcgggctgacccccaactttaaatctaacttcgacctggccgaagatgccaagcttcaactgagcaaagacacctacgatgatgatctcgacaatctgctggcccagatcggcgaccagtacgcagacctttttttggcggcaaagaacctgtcagacgccattctgctgagtgatattctgcgagtgaacacggagatcaccaaagctccgctgagcgctagtatgatcaagcgctatgatgagcaccaccaagacttgactttgctgaaggcccttgtcagacagcaactgcctgagaagtacaaggaaattttcttcgatcagtctaaaaatggctacgccggatacattgacggcggagcaagccaggaggaattttacaaatttattaagcccatcttggaaaaaatggacggcaccgaggagctgctggtaaagcttaacagagaagatctgttgcgcaaacagcgcactttcgacaatggaagcatcccccaccagattcacctgggcgaactgcacgctatcctcaggcggcaagaggatttctacccctttttgaaagataacagggaaaagattgagaaaatcctcacatttcggataccctactatgtaggccccctcgcccggggaaattccagattcgcgtggatgactcgcaaatcagaagagaccatcactccctggaacttcgaggaagtcgtggataagggggcctctgcccagtccttcatcgaaaggatgactaactttgataaaaatctgcctaacgaaaaggtgcttcctaaacactctctgctgtacgagtacttcacagtttataacgagctcaccaaggtcaaatacgtcacagaagggatgagaaagccagcattcctgtctggagagcagaagaaagctatcgtggacctcctcttcaagacgaaccggaaagttaccgtgaaacagctcaaagaagactatttcaaaaagattgaatgtttcgactctgttgaaatcagcggagtggaggatcgcttcaacgcatccctgggaacgtatcacgatctcctgaaaatcattaaagacaaggacttcctggacaatgaggagaacgaggacattcttgaggacattgtcctcacccttacgttgtttgaagatagggagatgattgaagaacgcttgaaaacttacgctcatctcttcgacgacaaagtcatgaaacagctcaagaggcgccgatatacaggatgggggcggctgtcaagaaaactgatcaatgggatccgagacaagcagagtggaaagacaatcctggattttcttaagtccgatggatttgccaaccggaacttcatgcagttgatccatgatgactctctcacctttaaggaggacatccagaaagcacaagtttctggccagggggacagtcttcacgagcacatcgctaatcttgcaggtagcccagctatcaaaaagggaatactgcagaccgttaaggtcgtggatgaactcgtcaaagtaatgggaaggcataagcccgagaatatcgttatcgagatggcccgagagaaccaaactacccagaagggacagaagaacagtagggaaaggatgaagaggattgaagagggtataaaagaactggggtcccaaatccttaaggaacacccagttgaaaacacccagcttcagaatgagaagctctacctgtactacctgcagaacggcagggacatgtacgtggatcaggaactggacatcaatcggctctccgactacgacgtggatcatatcgtgccccagtcttttctcaaagatgattctattgataataaagtgttgacaagatccgataaaaatagagggaagagtgataacgtcccctcagaagaagttgtcaagaaaatgaaaaattattggcggcagctgctgaacgccaaactgatcacacaacggaagttcgataatctgactaaggctgaacgaggtggcctgtctgagttggataaagccggcttcatcaaaaggcagcttgttgagacacgccagatcaccaagcacgtggcccaaattctcgattcacgcatgaacaccaagtacgatgaaaatgacaaactgattcgagaggtgaaagttattactctgaagtctaagctggtctcagatttcagaaaggactttcagttttataaggtgagagagatcaacaattaccaccatgcgcatgatgcctacctgaatgcagtggtaggcactgcacttatcaaaaaatatcccaagcttgaatctgaatttgtttacggagactataaagtgtacgatgttaggaaaatgatcgcaaagtctgagcaggaaataggcaaggccaccgctaagtacttcttttacagcaatattatgaattttttcaagaccgagattacactggccaatggagagattcggaagcgaccacttatcgaaacaaacggagaaacaggagaaatcgtgtgggacaagggtagggatttcgcgacagtccggaaggtcctgtccatgccgcaggtgaacatcgttaaaaagaccgaagtacagaccggaggcttctccaaggaaagtatcctcccgaaaaggaacagcgacaagctgatcgcacgcaaaaaagattgggaccccaagaaatacggcggattcgattctcctacagtcgcttacagtgtactggttgtggccaaagtggagaaagggaagtctaaaaaactcaaaagcgtcaaggaactgctgggcatcacaatcatggagcgatcaagcttcgaaaaaaaccccatcgactttctcgaggcgaaaggatataaagaggtcaaaaaagacctcatcattaagcttcccaagtactctctctttgagcttgaaaacggccggaaacgaatgctcgctagtgcgggcgagctgcagaaaggtaacgagctggcactgccctctaaatacgttaatttcttgtatctggccagccactatgaaaagctcaaagggtctcccgaagataatgagcagaagcagctgttcgtggaacaacacaaacactaccttgatgagatcatcgagcaaataagcgaattctccaaaagagtgatcctcgccgacgctaacctcgataaggtgctttctgcttacaataagcacagggataagcccatcagggagcaggcagaaaacattatccacttgtttactctgaccaacttgggcgcgcctgcagccttcaagtacttcgacaccaccatagacagaaagcggtacacctctacaaaggaggtcctggacgccacactgattcatcagtcaattacggggctctatgaaacaagaatcgacctctctcagctcggtggagacagcagggctgaccccaagaagaagaggaaggtggctagcgagggcagaggaagtcttctaacatgcggtgacgtggaggagaatcccggccctggtaccgtgagcaagggcgaggagctgttcaccggggtggtgcccatcctggtcgagctggacggcgacgtaaacggccacaagttcagcgtgtccggcgagggcgagggcgatgccacctacggcaagctgaccctgaagttcatctgcaccaccggcaagctgcccgtgccctggcccaccctcgtgaccaccctgacctacggcgtgcagtgcttcagccgctaccccgaccacatgaagcagcacgacttcttcaagtccgccatgcccgaaggctacgtccaggagcgcaccatcttcttcaaggacgacggcaactacaagacccgcgccgaggtgaagttcgagggcgacaccctggtgaaccgcatcgagctgaagggcatcgacttcaaggaggacggcaacatcctggggcacaagctggagtacaactacaacagccacaacgtctatatcatggccgacaagcagaagaacggcatcaaggtgaacttcaagatccgccacaacatcgaggacggcagcgtgcagctcgccgaccactaccagcagaacacccccatcggcgacggccccgtgctgctgcccgacaaccactacctgagcacccagtccgccctgagcaaagaccccaacgagaagcgcgatcacatggtcctgctggagttcgtgaccgccgccgggatcactctcggcatggacgagctgtacaagaccggttag

SEQ ID NO: 146-149 - skipped (4 entries)

SEQ ID NO: 150 - DNA, 23 bp, Artificial Sequence
  Description of Artificial Sequence: Synthetic oligonucleotide
tcctactcagactgttactctgg

SEQ ID NO: 151 - DNA, 23 bp, Artificial Sequence
  Description of Artificial Sequence: Synthetic oligonucleotide
tcctactcacactgttactcagg

SEQ ID NO: 152 - DNA, 23 bp, Artificial Sequence
  Description of Artificial Sequence: Synthetic oligonucleotide
acctgctcacactgttactccag

SEQ ID NO: 153 - DNA, 23 bp, Artificial Sequence
  Description of Artificial Sequence: Synthetic oligonucleotide
gcattctcaaactgttactcagg

SEQ ID NO: 154 - DNA, 23 bp, Artificial Sequence
  Description of Artificial Sequence: Synthetic oligonucleotide
ggattctcacactgttactcggg

SEQ ID NO: 155 - DNA, 23 bp, Artificial Sequence
  Description of Artificial Sequence: Synthetic oligonucleotide
acatacttatactgttactctag

SEQ ID NO: 156 - DNA, 23 bp, Artificial Sequence
  Description of Artificial Sequence: Synthetic oligonucleotide
tattcctaagactgttactcaag

SEQ ID NO: 157 - DNA, 23 bp, Artificial Sequence
  Description of Artificial Sequence: Synthetic oligonucleotide
aaggactaagactgttactcggg

SEQ ID NO: 158 - DNA, 23 bp, Artificial Sequence
  Description of Artificial Sequence: Synthetic oligonucleotide
gagctctcatactgttactctag

SEQ ID NO: 159 - DNA, 23 bp, Artificial Sequence
  Description of Artificial Sequence: Synthetic oligonucleotide
gcaaaatgagactgttactccag

SEQ ID NO: 160 - DNA, 23 bp, Artificial Sequence
  Description of Artificial Sequence: Synthetic oligonucleotide
cctcattcagactgttactcaag

SEQ ID NO: 161 - DNA, 23 bp, Artificial Sequence
  Description of Artificial Sequence: Synthetic oligonucleotide
cattggctttgatttccctaggg

SEQ ID NO: 162 - DNA, 23 bp, Artificial Sequence
  Description of Artificial Sequence: Synthetic oligonucleotide
aattggcattgatttccctagag

SEQ ID NO: 163 - DNA, 23 bp, Artificial Sequence
  Description of Artificial Sequence: Synthetic oligonucleotide
cattggctttaatttccctatag

SEQ ID NO: 164 - DNA, 23 bp, Artificial Sequence
  Description of Artificial Sequence: Synthetic oligonucleotide
gataggctgtgatttccctagag

SEQ ID NO: 165 - DNA, 23 bp, Artificial Sequence
  Description of Artificial Sequence: Synthetic oligonucleotide
gaatagccttgatttccctaaag

SEQ ID NO: 166 - DNA, 23 bp, Artificial Sequence
  Description of Artificial Sequence: Synthetic oligonucleotide
aatttgctttgatttccctgagg

SEQ ID NO: 167 - DNA, 23 bp, Artificial Sequence
  Description of Artificial Sequence: Synthetic oligonucleotide
gatgtgctttgatttcccttggg

SEQ ID NO: 168 - DNA, 23 bp, Artificial Sequence
  Description of Artificial Sequence: Synthetic oligonucleotide
aattggttttaatttccctaaag

SEQ ID NO: 169 - DNA, 23 bp, Artificial Sequence
  Description of Artificial Sequence: Synthetic oligonucleotide
aattgggtttgatttccctttgg

SEQ ID NO: 170 - DNA, 23 bp, Artificial Sequence
  Description of Artificial Sequence: Synthetic oligonucleotide
gatgggtttttatttccctagag

SEQ ID NO: 171 - DNA, 23 bp, Artificial Sequence
  Description of Artificial Sequence: Synthetic oligonucleotide
gaatggttttgatttccctggag

SEQ ID NO: 172 - DNA, 23 bp, Artificial Sequence
  Description of Artificial Sequence: Synthetic oligonucleotide
acagttgcctaagaactggtggg

SEQ ID NO: 173 - DNA, 23 bp, Artificial Sequence
  Description of Artificial Sequence: Synthetic oligonucleotide
ccagttgtctaagaactggggag

SEQ ID NO: 174 - DNA, 23 bp, Artificial Sequence
  Description of Artificial Sequence: Synthetic oligonucleotide
gcagttgcctgtgaactggtagg

SEQ ID NO: 175 - DNA, 23 bp, Artificial Sequence
  Description of Artificial Sequence: Synthetic oligonucleotide
gcagatgcagaagaactggtgag

SEQ ID NO: 176 - DNA, 23 bp, Artificial Sequence
  Description of Artificial Sequence: Synthetic oligonucleotide
gcagttccagaagaactggtgag

SEQ ID NO: 177 - DNA, 23 bp, Artificial Sequence
  Description of Artificial Sequence: Synthetic oligonucleotide
caacttgcctatgaactggtagg

SEQ ID NO: 178 - DNA, 23 bp, Artificial Sequence
  Description of Artificial Sequence: Synthetic oligonucleotide
acacctgcctaagaactggaggg

SEQ ID NO: 179 - DNA, 23 bp, Artificial Sequence
  Description of Artificial Sequence: Synthetic oligonucleotide
tcaggtggctaagaactgggtgg

SEQ ID NO: 180 - DNA, 23 bp, Artificial Sequence
  Description of Artificial Sequence: Synthetic oligonucleotide
gaagttggccaagaactggagag

SEQ ID NO: 181 - DNA, 23 bp, Artificial Sequence
  Description of Artificial Sequence: Synthetic oligonucleotide
gctgctgcccaagaactggcagg

SEQ ID NO: 182 - DNA, 23 bp, Artificial Sequence
  Description of Artificial Sequence: Synthetic oligonucleotide
tcagctggctaagaacgggtaag

SEQ ID NO: 183 - DNA, 23 bp, Artificial Sequence
  Description of Artificial Sequence: Synthetic oligonucleotide
agggctccaccctcacgagtggg

SEQ ID NO: 184 - DNA, 23 bp, Artificial Sequence
  Description of Artificial Sequence: Synthetic oligonucleotide
gcagctcagccctcacgagtcag

SEQ ID NO: 185 - DNA, 23 bp, Artificial Sequence
  Description of Artificial Sequence: Synthetic oligonucleotide
ggggcttcagcatcacgagtgag

SEQ ID NO: 186 - DNA, 23 bp, Artificial Sequence
  Description of Artificial Sequence: Synthetic oligonucleotide
ggggctctcccctcactagtgag

SEQ ID NO: 187 - DNA, 23 bp, Artificial Sequence
  Description of Artificial Sequence: Synthetic oligonucleotide
ggggatccaccttcaccagtcag

SEQ ID NO: 188 - DNA, 23 bp, Artificial Sequence
  Description of Artificial Sequence: Synthetic oligonucleotide
agggctggaccctcacaagtaag

SEQ ID NO: 189 - DNA, 23 bp, Artificial Sequence
  Description of Artificial Sequence: Synthetic oligonucleotide
tggtctcctcccccacgagtggg

SEQ ID NO: 190 - DNA, 23 bp, Artificial Sequence
  Description of Artificial Sequence: Synthetic oligonucleotide
agggctcccaccccacgagtgag

SEQ ID NO: 191 - DNA, 23 bp, Artificial Sequence
  Description of Artificial Sequence: Synthetic oligonucleotide
gaggctccatactcaccagtgag

SEQ ID NO: 192 - DNA, 23 bp, Artificial Sequence
  Description of Artificial Sequence: Synthetic oligonucleotide
ggagctgccccttcacgagtggg

SEQ ID NO: 193 - DNA, 23 bp, Artificial Sequence
  Description of Artificial Sequence: Synthetic oligonucleotide
atgactccaccctcaagagtaag

SEQ ID NO: 194 - DNA, 23 bp, Artificial Sequence
  Description of Artificial Sequence: Synthetic oligonucleotide
gccttctttatcccctatcgagg

SEQ ID NO: 195 - DNA, 23 bp, Artificial Sequence
  Description of Artificial Sequence: Synthetic oligonucleotide
gtctgctgtgtcccctatcgggg

SEQ ID NO: 196 - DNA, 23 bp, Artificial Sequence
  Description of Artificial Sequence: Synthetic oligonucleotide
cccttctctatcccctgtcgtgg

SEQ ID NO: 197 - DNA, 23 bp, Artificial Sequence
  Description of Artificial Sequence: Synthetic oligonucleotide
gccttctttatcccctctcttgg

SEQ ID NO: 198 - DNA, 23 bp, Artificial Sequence
  Description of Artificial Sequence: Synthetic oligonucleotide
gcgctctttttcccctatcttag

SEQ ID NO: 199 - DNA, 23 bp, Artificial Sequence
  Description of Artificial Sequence: Synthetic oligonucleotide
gccctctgtctcccctgtcgcag

SEQ ID NO: 200 - DNA, 23 bp, Artificial Sequence
  Description of Artificial Sequence: Synthetic oligonucleotide
tccatctttgtcccctattgagg

SEQ ID NO: 201 - DNA, 23 bp, Artificial Sequence
  Description of Artificial Sequence: Synthetic oligonucleotide
accttctctctcccctatagagg

SEQ ID NO: 202 - DNA, 23 bp, Artificial Sequence
  Description of Artificial Sequence: Synthetic oligonucleotide
gttttctttttcccctatgggag

SEQ ID NO: 203 - DNA, 23 bp, Artificial Sequence
  Description of Artificial Sequence: Synthetic oligonucleotide
tgcttcttaatcccctatcaaag

SEQ ID NO: 204 - DNA, 23 bp, Artificial Sequence
  Description of Artificial Sequence: Synthetic oligonucleotide
accttcttactcccctatccggg

SEQ ID NO: 205 - DNA, 22 bp, Artificial Sequence
  Description of Artificial Sequence: Synthetic primer
gagaggttatgtggctttacca

SEQ ID NO: 206 - DNA, 20 bp, Artificial Sequence
  Description of Artificial Sequence: Synthetic primer
aaaaatgcttcccactttgc

SEQ ID NO: 207 - DNA, 20 bp, Artificial Sequence
  Description of Artificial Sequence: Synthetic primer
ctcattctcatgcctggaca

SEQ ID NO: 208 - DNA, 25 bp, Artificial Sequence
  Description of Artificial Sequence: Synthetic primer
gagtttggctcaaattgttactctt

SEQ ID NO: 209 - DNA, 25 bp, Artificial Sequence
  Description of Artificial Sequence: Synthetic primer
gggaaatggtctaggagagtaaagt

SEQ ID NO: 210 - DNA, 25 bp, Artificial Sequence
  Description of Artificial Sequence: Synthetic primer
gtttggctcaaattgttactcttca

SEQ ID NO: 211 - DNA, 25 bp, Artificial Sequence
  Description of Artificial Sequence: Synthetic primer
gtgagagtaatgtgtttgctgagag

SEQ ID NO: 212 - DNA, 20 bp, Artificial Sequence
  Description of Artificial Sequence: Synthetic primer
cgggcttggacagaacttac

SEQ ID NO: 213 - DNA, 20 bp, Artificial Sequence
  Description of Artificial Sequence: Synthetic primer
ctgcgtagtgccaaaacaaa

SEQ ID NO: 214 - DNA, 24 bp, Artificial Sequence
  Description of Artificial Sequence: Synthetic primer
taatttcattgaagagtggctgaa

SEQ ID NO: 215 - DNA, 24 bp, Artificial Sequence
  Description of Artificial Sequence: Synthetic primer
aagccctgtgtggtagtagtcagt

SEQ ID NO: 216 - DNA, 24 bp, Artificial Sequence
  Description of Artificial Sequence: Synthetic primer
tgagtcatgttggataaccagtct

SEQ ID NO: 217 - DNA, 24 bp, Artificial Sequence
  Description of Artificial Sequence: Synthetic primer
gaaggtcaggaacatacaattcaa

SEQ ID NO: 218 - DNA, 24 bp, Artificial Sequence
  Description of Artificial Sequence: Synthetic primer
gatatgggcatgtcagtttcatag

SEQ ID NO: 219 - DNA, 24 bp, Artificial Sequence
  Description of Artificial Sequence: Synthetic primer
tgctgttgattaatggttgatagg

SEQ ID NO: 220 - DNA, 23 bp, Artificial Sequence
  Description of Artificial Sequence: Synthetic primer
ttttaaattgccatgtttgtgtc

SEQ ID NO: 221 - DNA, 24 bp, Artificial Sequence
  Description of Artificial Sequence: Synthetic primer
atgaataacctaatgggcagaaaa

SEQ ID NO: 222 - DNA, 24 bp, Artificial Sequence
  Description of Artificial Sequence: Synthetic primer
tcaagtcgcttcattttgatagac

SEQ ID NO: 223 - DNA, 24 bp, Artificial Sequence
  Description of Artificial Sequence: Synthetic primer
cacaacaaaacatatagccaaagc

SEQ ID NO: 224 - DNA, 25 bp, Artificial Sequence
  Description of Artificial Sequence: Synthetic primer
tgctgctaaaataacacaaatcagt

SEQ ID NO: 225 - DNA, 23 bp, Artificial Sequence
  Description of Artificial Sequence: Synthetic primer
ctgtgcctattgtggttatcctg

SEQ ID NO: 226 - DNA, 24 bp, Artificial Sequence
  Description of Artificial Sequence: Synthetic primer
attgatctgcaatacatgtggagt

SEQ ID NO: 227 - DNA, 24 bp, Artificial Sequence
  Description of Artificial Sequence: Synthetic primer
tttgcctctgctattacagtatgg

SEQ ID NO: 228 - DNA, 24 bp, Artificial Sequence
  Description of Artificial Sequence: Synthetic primer
tgtagggtggttggctaaaataat

SEQ ID NO: 229 - DNA, 24 bp, Artificial Sequence
  Description of Artificial Sequence: Synthetic primer
tttttgcacagtcaataacacaaa

SEQ ID NO: 230 - DNA, 24 bp, Artificial Sequence
  Description of Artificial Sequence: Synthetic primer
ggctggtctcacaattgtacttta

SEQ ID NO: 231 - DNA, 24 bp, Artificial Sequence
  Description of Artificial Sequence: Synthetic primer
cattatggactgaaaatctcagca

SEQ ID NO: 232 - DNA, 24 bp, Artificial Sequence
  Description of Artificial Sequence: Synthetic primer
atcatcctagccataacacaatga

SEQ ID NO: 233 - DNA, 24 bp, Artificial Sequence
  Description of Artificial Sequence: Synthetic primer
ttcagctttaacgtgattttctgt

SEQ ID NO: 234 - DNA, 24 bp, Artificial Sequence
  Description of Artificial Sequence: Synthetic primer
ggattcagaagctgtttacgaagt

SEQ ID NO: 235 - DNA, 24 bp, Artificial Sequence
  Description of Artificial Sequence: Synthetic primer
tttagctggattggaaaaacaaat

SEQ ID NO: 236 - DNA, 24 bp, Artificial Sequence
  Description of Artificial Sequence: Synthetic primer
aactcaccccattgttggtatatt

SEQ ID NO: 237 - DNA, 24 bp, Artificial Sequence
  Description of Artificial Sequence: Synthetic primer
ccttgtccaaataccgaaatacat

SEQ ID NO: 238 - DNA, 24 bp, Artificial Sequence
  Description of Artificial Sequence: Synthetic primer
cacataattcatgaacttggcttc

SEQ ID NO: 239 - DNA, 24 bp, Artificial Sequence
  Description of Artificial Sequence: Synthetic primer
tagtagctggggaggaagatacag

SEQ ID NO: 240 - DNA, 24 bp, Artificial Sequence
  Description of Artificial Sequence: Synthetic primer
tttttgttttaattgcgactgtgt

SEQ ID NO: 241 - DNA, 24 bp, Artificial Sequence
  Description of Artificial Sequence: Synthetic primer
agaaaaggggttttcttttgactt

SEQ ID NO: 242 - DNA, 24 bp, Artificial Sequence
  Description of Artificial Sequence: Synthetic primer
cattgtgactggatgagaagaaac

SEQ ID NO: 243 - DNA, 24 bp, Artificial Sequence
  Description of Artificial Sequence: Synthetic primer
aacggctgttattaaagtcctcag

SEQ ID NO: 244 - DNA, 24 bp, Artificial Sequence
  Description of Artificial Sequence: Synthetic primer
caagtcagaagtcacttgctttgt

SEQ ID NO: 245 - DNA, 24 bp, Artificial Sequence
  Description of Artificial Sequence: Synthetic primer
ttttatgtgcaggaatcagtctgt

SEQ ID NO: 246 - DNA, 18 bp, Artificial Sequence
  Description of Artificial Sequence: Synthetic primer
tggcggcgttttcattat

SEQ ID NO: 247 - DNA, 26 bp, Artificial Sequence
  Description of Artificial Sequence: Synthetic primer
ttcgatccgtaatgattgttctagcc

SEQ ID NO: 248 - DNA, 20 bp, Artificial Sequence
  Description of Artificial Sequence: Synthetic primer
ggtcttccagagtgctgagg

SEQ ID NO: 249 - DNA, 24 bp, Artificial Sequence
  Description of Artificial Sequence: Synthetic primer
tgtgtgcttctgtacacatcatct

SEQ ID NO: 250 - DNA, 24 bp, Artificial Sequence
  Description of Artificial Sequence: Synthetic primer
agatttcaaccctcaaaaactgag

SEQ ID NO: 251 - DNA, 24 bp, Artificial Sequence
  Description of Artificial Sequence: Synthetic primer
taaactctttcttttccgcaattc

SEQ ID NO: 252 - DNA, 24 bp, Artificial Sequence
  Description of Artificial Sequence: Synthetic primer
caaggtgacctgctacctaaaaat

SEQ ID NO: 253 - DNA, 24 bp, Artificial Sequence
  Description of Artificial Sequence: Synthetic primer
tatgaccaaggctatgtgttcact

SEQ ID NO: 254 - DNA, 24 bp, Artificial Sequence
  Description of Artificial Sequence: Synthetic primer
acagcctctctccagtaacattct

SEQ ID NO: 255 - DNA, 24 bp, Artificial Sequence
  Description of Artificial Sequence: Synthetic primer
tattcttgcagtggtttcacattt

SEQ ID NO: 256 - DNA, 24 bp, Artificial Sequence
  Description of Artificial Sequence: Synthetic primer
atattttaagccaagacccaacaa

SEQ ID NO: 257 - DNA, 24 bp, Artificial Sequence
  Description of Artificial Sequence: Synthetic primer
ctttcaactgtctgtctgattgct

SEQ ID NO: 258 - DNA, 24 bp, Artificial Sequence
  Description of Artificial Sequence: Synthetic primer
aacagcctctcttcattgttctct

SEQ ID NO: 259 - DNA, 24 bp, Artificial Sequence
  Description of Artificial Sequence: Synthetic primer
ctctggaacttgtctctgtcttga

SEQ ID NO: 260 - DNA, 24 bp, Artificial Sequence
  Description of Artificial Sequence: Synthetic primer
ctttcctgcgttctcatgttacta

SEQ ID NO: 261 - DNA, 24 bp, Artificial Sequence
  Description of Artificial Sequence: Synthetic primer
ccttatatccgtatcgctcactct

SEQ ID NO: 262 - DNA, 24 bp, Artificial Sequence
  Description of Artificial Sequence: Synthetic primer
catatctgtctaacttccgcacac

SEQ ID NO: 263 - DNA, 24 bp, Artificial Sequence
  Description of Artificial Sequence: Synthetic primer
acaggtgttatgttgtctgcatct

SEQ ID NO: 264 - DNA, 24 bp, Artificial Sequence
  Description of Artificial Sequence: Synthetic primer
actccattcccagattagttatgc

SEQ ID NO: 265 - DNA, 24 bp, Artificial Sequence
  Description of Artificial Sequence: Synthetic primer
ctgttttctttgtgagagtggaga

SEQ ID NO: 266 - DNA, 24 bp, Artificial Sequence
  Description of Artificial Sequence: Synthetic primer
tgtaaggtggtcaaacttgctcta

SEQ ID NO: 267 - DNA, 25 bp, Artificial Sequence
  Description of Artificial Sequence: Synthetic primer
tttttcctagtacccacagattttt

SEQ ID NO: 268 - DNA, 24 bp, Artificial Sequence
  Description of Artificial Sequence: Synthetic primer
tccctgattctctcatttgtgtta

SEQ ID NO: 269 - DNA, 24 bp, Artificial Sequence
  Description of Artificial Sequence: Synthetic primer
ttgggaacatcagagaaagtatga

SEQ ID NO: 270 - DNA, 24 bp, Artificial Sequence
  Description of Artificial Sequence: Synthetic primer
acaaattacagtctcctgggaaag

SEQ ID NO: 271 - DNA, 24 bp, Artificial Sequence
  Description of Artificial Sequence: Synthetic primer
agtagcttaccttggcagagaaaa

SEQ ID NO: 272 - DNA, 24 bp, Artificial Sequence
  Description of Artificial Sequence: Synthetic primer
tgacatactgttaccctttgcagt

SEQ ID NO: 273 - DNA, 23 bp, Artificial Sequence
  Description of Artificial Sequence: Synthetic primer
gaaaggctcagtgaatgtttgtt

SEQ ID NO: 274 - DNA, 24 bp, Artificial Sequence
  Description of Artificial Sequence: Synthetic primer
cactgcatcatctcattaaatcaa

SEQ ID NO: 275 - DNA, 24 bp, Artificial Sequence
  Description of Artificial Sequence: Synthetic primer
cccatatattcatgattacccaca

SEQ ID NO: 276 - DNA, 24 bp, Artificial Sequence
  Description of Artificial Sequence: Synthetic primer
tatcagaacgagcactaaaagcac

SEQ ID NO: 277 - DNA, 20 bp, Artificial Sequence
  Description of Artificial Sequence: Synthetic primer
ttgggaggctgaggtacaag

SEQ ID NO: 278 - DNA, 24 bp, Artificial Sequence
  Description of Artificial Sequence: Synthetic primer
gaatgaaaaacaaacagaaggtga

SEQ ID NO: 279 - DNA, 24 bp, Artificial Sequence
  Description of Artificial Sequence: Synthetic primer
ctcctcatctgtacccttcaatct

SEQ ID NO: 280 - DNA, 24 bp, Artificial Sequence
  Description of Artificial Sequence: Synthetic primer
agagtggcatctagtgtcagtgag

SEQ ID NO: 281 - DNA, 24 bp, Artificial Sequence
  Description of Artificial Sequence: Synthetic primer
taccaaaagcttctcctgtttacc

SEQ ID NO: 282 - DNA, 24 bp, Artificial Sequence
  Description of Artificial Sequence: Synthetic primer
gtaagttggatggcctattctttg

SEQ ID NO: 283 - DNA, 24 bp, Artificial Sequence
  Description of Artificial Sequence: Synthetic primer
gaaggaaatgcaaggatacaagat

SEQ ID NO: 284 - DNA, 24 bp, Artificial Sequence
  Description of Artificial Sequence: Synthetic primer
tgattgaaagaatcattccagaaa

SEQ ID NO: 285 - DNA, 24 bp, Artificial Sequence
  Description of Artificial Sequence: Synthetic primer
tcagaaggaaaattgaaattggtt

SEQ ID NO: 286 - DNA, 24 bp, Artificial Sequence
  Description of Artificial Sequence: Synthetic primer
cagatgtgttcttcatcattcctc

SEQ ID NO: 287 - DNA, 24 bp, Artificial Sequence
  Description of Artificial Sequence: Synthetic primer
ttctctttagggaaagctctcaaa

SEQ ID NO: 288 - DNA, 24 bp, Artificial Sequence
  Description of Artificial Sequence: Synthetic primer
gggtatagatcatatggagggaag

SEQ ID NO: 289 - DNA, 20 bp, Artificial Sequence
  Description of Artificial Sequence: Synthetic primer
agatgatctgcccacctcag

SEQ ID NO: 290 - DNA, 24 bp, Artificial Sequence
  Description of Artificial Sequence: Synthetic primer
ctttcttcctcatttagtggcaat

SEQ ID NO: 291 - DNA, 24 bp, Artificial Sequence
  Description of Artificial Sequence: Synthetic primer
atgaattgcagattgatggtactg

SEQ ID NO: 292 - DNA, 24 bp, Artificial Sequence
  Description of Artificial Sequence: Synthetic primer
tctcaccaagaaccaaattgtcta

SEQ ID NO: 293 - DNA, 24 bp, Artificial Sequence
  Description of Artificial Sequence: Synthetic primer
gtaggataccttggcaacagtctt

SEQ ID NO: 294 - DNA, 24 bp, Artificial Sequence
  Description of Artificial Sequence: Synthetic primer
ttaacgaattgtgagatttgctgt

SEQ ID NO: 295 - DNA, 24 bp, Artificial Sequence
  Description of Artificial Sequence: Synthetic primer
tcagaaagtcaagtagcacacaca

SEQ ID NO: 296 - DNA, 23 bp, Artificial Sequence
  Description of Artificial Sequence: Synthetic primer
agaagcacacactcaggtaaagc

SEQ ID NO: 297 - DNA, 24 bp, Artificial Sequence
  Description of Artificial Sequence: Synthetic primer
tctttgggggaataatgactaaaa

SEQ ID NO: 298 - DNA, 24 bp, Artificial Sequence
  Description of Artificial Sequence: Synthetic primer
tttggcatttatgggaataaaact

SEQ ID NO: 299 - DNA, 23 bp, Artificial Sequence
  Description of Artificial Sequence: Synthetic primer
actaattctggtcaagcccatca

SEQ ID NO: 300 - DNA, 24 bp, Artificial Sequence
  Description of Artificial Sequence: Synthetic primer
ttaagacatcggatgaacagaaag

SEQ ID NO: 301 - DNA, 23 bp, Artificial Sequence
  Description of Artificial Sequence: Synthetic primer
agaagctttctgacatgatctgc

SEQ ID NO: 302 - DNA, 24 bp, Artificial Sequence
  Description of Artificial Sequence: Synthetic primer
tcaattgcattaggacttagacca

SEQ ID NO: 303 - DNA, 24 bp, Artificial Sequence
  Description of Artificial Sequence: Synthetic primer
gttaaattacctgtgaagcccttg

SEQ ID NO: 304 - DNA, 24 bp, Artificial Sequence
  Description of Artificial Sequence: Synthetic primer
cggaaaacagatccactttatgat

SEQ ID NO: 305 - DNA, 24 bp, Artificial Sequence
  Description of Artificial Sequence: Synthetic primer
aaatccactggaaacatcttgagt

SEQ ID NO: 306 - DNA, 24 bp, Artificial Sequence
  Description of Artificial Sequence: Synthetic primer
agtctcttcagaatcatgccctat

SEQ ID NO: 307 - DNA, 22 bp, Artificial Sequence
  Description of Artificial Sequence: Synthetic primer
gcttggtggcacatacctgtag

SEQ ID NO: 308 - DNA, 24 bp, Artificial Sequence
  Description of Artificial Sequence: Synthetic primer
ggtaggtagatttgcttgcttgtt

SEQ ID NO: 309 - DNA, 24 bp, Artificial Sequence
  Description of Artificial Sequence: Synthetic primer
agctctcagcagagtagggattta

SEQ ID NO: 310 - DNA, 21 bp, Artificial Sequence
  Description of Artificial Sequence: Synthetic primer
gtgagtctactgcaccccatc

SEQ ID NO: 311 - DNA, 24 bp, Artificial Sequence
  Description of Artificial Sequence: Synthetic primer
tgacactgtgaagtcaattctgtc

SEQ ID NO: 312 - DNA, 24 bp, Artificial Sequence
  Description of Artificial Sequence: Synthetic primer
tcaagaacttgacaatgagcaaat

SEQ ID NO: 313 - DNA, 22 bp, Artificial Sequence
  Description of Artificial Sequence: Synthetic primer
tatccgatccactgttgtgtgt

SEQ ID NO: 314 - DNA, 23 bp, Artificial Sequence
  Description of Artificial Sequence: Synthetic primer
caggagacccaaaaccactctac

SEQ ID NO: 315 - DNA, 24 bp, Artificial Sequence
  Description of Artificial Sequence: Synthetic primer
ttgttctacaaatagggcttcctt

SEQ ID NO: 316 - DNA, 24 bp, Artificial Sequence
  Description of Artificial Sequence: Synthetic primer
tgttaagtttgggcttatgttcct

SEQ ID NO: 317 - DNA, 23 bp, Artificial Sequence
  Description of Artificial Sequence: Synthetic primer
cacaagtctcactgcacaaacat

SEQ ID NO: 318 - DNA, 24 bp, Artificial Sequence
  Description of Artificial Sequence: Synthetic primer
tgacccatgattatctctctttga

SEQ ID NO: 319 - DNA, 24 bp, Artificial Sequence
  Description of Artificial Sequence: Synthetic primer
ttcagcttctgattggttttaatg

SEQ ID NO: 320 - DNA, 24 bp, Artificial Sequence
  Description of Artificial Sequence: Synthetic primer
ccaattccttaattttccctacag

SEQ ID NO: 321 - DNA, 21 bp, Artificial Sequence
  Description of Artificial Sequence: Synthetic primer
atctcagaccaggagggagac

SEQ ID NO: 322 - DNA, 24 bp, Artificial Sequence
  Description of Artificial Sequence: Synthetic primer
cctcagggtcagtacatttttcag

SEQ ID NO: 323 - DNA, 24 bp, Artificial Sequence
  Description of Artificial Sequence: Synthetic primer
ttcttaggacattgctccacatac

SEQ ID NO: 324 - DNA, 24 bp, Artificial Sequence
  Description of Artificial Sequence: Synthetic primer
gcaaacataatgcaactcgtaatc

SEQ ID NO: 325 - DNA, 21 bp, Artificial Sequence
  Description of Artificial Sequence: Synthetic primer
gcaagggagtctgtgtctttg

SEQ ID NO: 326 - DNA, 24 bp, Artificial Sequence
  Description of Artificial Sequence: Synthetic primer
tcatttaagtggctgttctgtgtt

SEQ ID NO: 327 - DNA, 24 bp, Artificial Sequence
  Description of Artificial Sequence: Synthetic primer
acaaaacagagagaaaaggcagag

SEQ ID NO: 328 - DNA, 23 bp, Artificial Sequence
  Description of Artificial Sequence: Synthetic primer
gttttgatttctggtgcctacag

SEQ ID NO: 329 - DNA, 20 bp, Artificial Sequence
  Description of Artificial Sequence: Synthetic primer
actgaagctgaagcccagtc

SEQ ID NO: 330 - DNA, 23 bp, Artificial Sequence
  Description of Artificial Sequence: Synthetic primer
acatgagctctcaggtttctgac

SEQ ID NO: 331 - DNA, 25 bp, Artificial Sequence
  Description of Artificial Sequence: Synthetic primer
tcaaacttagatggttccctatgtt

SEQ ID NO: 332 - DNA, 24 bp, Artificial Sequence
  Description of Artificial Sequence: Synthetic primer
gtaccctgaaaatgtagggtgact

SEQ ID NO: 333 - DNA, 20 bp, Artificial Sequence
  Description of Artificial Sequence: Synthetic primer
cacttcccaagtgaggcaat

SEQ ID NO: 334 - DNA, 24 bp, Artificial Sequence
  Description of Artificial Sequence: Synthetic primer
ctatacttggggctgacttgctac

SEQ ID NO: 335 - DNA, 24 bp, Artificial Sequence
  Description of Artificial Sequence: Synthetic primer
tcgtataggttactttggctcaca

SEQ ID NO: 336 - DNA, 24 bp, Artificial Sequence
  Description of Artificial Sequence: Synthetic primer
agggatctttactcctcagtgtgt

SEQ ID NO: 337 - DNA, 24 bp, Artificial Sequence
  Description of Artificial Sequence: Synthetic primer
tgtagaagttggaatatcctgctg

SEQ ID NO: 338 - DNA, 24 bp, Artificial Sequence
  Description of Artificial Sequence: Synthetic primer
gtcaacaatttgatctcaggcttc

SEQ ID NO: 339 - DNA, 24 bp, Artificial Sequence
  Description of Artificial Sequence: Synthetic primer
ctcagtactaaagatggacgcttg

SEQ ID NO: 340 - DNA, 24 bp, Artificial Sequence
  Description of Artificial Sequence: Synthetic primer
aatcatttcagtcttcccaacaat

SEQ ID NO: 341 - DNA, 24 bp, Artificial Sequence
  Description of Artificial Sequence: Synthetic primer
gggaatcacagtagatgtttgtca

SEQ ID NO: 342 - DNA, 24 bp, Artificial Sequence
  Description of Artificial Sequence: Synthetic primer
agaccaggaggtaagaacattttg

SEQ ID NO: 343 - DNA, 24 bp, Artificial Sequence
  Description of Artificial Sequence: Synthetic primer
ccacatagaaagagacttgcagaa

SEQ ID NO: 344 - DNA, 24 bp, Artificial Sequence
  Description of Artificial Sequence: Synthetic primer
agagatgccaaaagaacagtcaat

SEQ ID NO: 345 - DNA, 24 bp, Artificial Sequence
  Description of Artificial Sequence: Synthetic primer
tgtgccttaggctatgtaaactgt

SEQ ID NO: 346 - DNA, 24 bp, Artificial Sequence
  Description of Artificial Sequence: Synthetic primer
aaacccttgtaaccaaaattacca

SEQ ID NO: 347 - DNA, 24 bp, Artificial Sequence
  Description of Artificial Sequence: Synthetic primer
taactgcatcagaagtccttgcta

SEQ ID NO: 348 - DNA, 22 bp, Artificial Sequence
  Description of Artificial Sequence: Synthetic primer
ggagaccaagctgctaaagtca

SEQ ID NO: 349 - DNA, 37 bp, Artificial Sequence
  Description of Artificial Sequence: Synthetic primer
gtggtgccgcgggagtttggctcaaattgttactctt

SEQ ID NO: 350 - DNA, 37 bp, Artificial Sequence
  Description of Artificial Sequence: Synthetic primer
gtggtgccgcgggggaaatggtctaggagagtaaagt

SEQ ID NO: 351 - DNA, 34 bp, Artificial Sequence
  Description of Artificial Sequence: Synthetic primer
gtggtgccgcgggagaggttatgtggctttacca

SEQ ID NO: 352 - DNA, 32 bp, Artificial Sequence
  Description of Artificial Sequence: Synthetic primer
gtggtgccgcggctcattctcatgcctggaca

SEQ ID NO: 353 - DNA, 32 bp, Artificial Sequence
  Description of Artificial Sequence: Synthetic primer
gtggtgccgcggcgggcttggacagaacttac

SEQ ID NO: 354 - DNA, 32 bp, Artificial Sequence
  Description of Artificial Sequence: Synthetic primer
gtggtgccgcggctgcgtagtgccaaaacaaa

SEQ ID NO: 355 - DNA, 36 bp, Artificial Sequence
  Description of Artificial Sequence: Synthetic primer
gtggtgccgcggtaatttcattgaagagtggctgaa

SEQ ID NO: 356 - DNA, 36 bp, Artificial Sequence
  Description of Artificial Sequence: Synthetic primer
gtggtgccgcggaagccctgtgtggtagtagtcagt

SEQ ID NO: 357 - DNA, 36 bp, Artificial Sequence
  Description of Artificial Sequence: Synthetic primer
gtggtgccgcggcaagtcagaagtcacttgctttgt

SEQ ID NO: 358 - DNA, 36 bp, Artificial Sequence
  Description of Artificial Sequence: Synthetic primer
gtggtgccgcggttttatgtgcaggaatcagtctgt

SEQ ID NO: 359 - DNA, 36 bp, Artificial Sequence
  Description of Artificial Sequence: Synthetic primer
gtggtgccgcggtgtgtgcttctgtacacatcatct

SEQ ID NO: 360 - DNA, 36 bp, Artificial Sequence
  Description of Artificial Sequence: Synthetic primer
gtggtgccgcggagatttcaaccctcaaaaactgag

SEQ ID NO: 361 - DNA, 36 bp, Artificial Sequence
  Description of Artificial Sequence: Synthetic primer
gtggtgccgcggttgggaacatcagagaaagtatga

SEQ ID NO: 362 - DNA, 36 bp, Artificial Sequence
  Description of Artificial Sequence: Synthetic primer
gtggtgccgcggacaaattacagtctcctgggaaag

SEQ ID NO: 363 - DNA, 32 bp, Artificial Sequence
  Description of Artificial Sequence: Synthetic primer
gtggtgccgcggcacttcccaagtgaggcaat

SEQ ID NO: 364 - DNA, 36 bp, Artificial Sequence
  Description of Artificial Sequence: Synthetic primer
gtggtgccgcggctatacttggggctgacttgctac

SEQ ID NO: 365 - DNA, 34 bp, Artificial Sequence
  Description of Artificial Sequence: Synthetic primer
gtggtgccgcggttggctctttagcttgtgtttc

SEQ ID NO: 366 - DNA, 32 bp, Artificial Sequence
  Description of Artificial Sequence: Synthetic primer
gtggtgccgcggtgagactcccaaaggcaatc

SEQ ID NO: 367 - DNA, 34 bp, Artificial Sequence; identical to SEQ ID NO: 365
  Description of Artificial Sequence: Synthetic primer

SEQ ID NO: 368 - DNA, 32 bp, Artificial Sequence
  Description of Artificial Sequence: Synthetic primer
gtggtgccgcggactgaggggtgatcttggtg

SEQ ID NO: 369 - DNA, 32 bp, Artificial Sequence
  Description of Artificial Sequence: Synthetic primer
gtggtgccgcgggcagagaaagccagtcggta

SEQ ID NO: 370 - DNA, 32 bp, Artificial Sequence; identical to SEQ ID NO: 366
  Description of Artificial Sequence: Synthetic primer

SEQ ID NO: 371 - DNA, 32 bp, Artificial Sequence; identical to SEQ ID NO: 369
  Description of Artificial Sequence: Synthetic primer

SEQ ID NO: 372 - DNA, 32 bp, Artificial Sequence; identical to SEQ ID NO: 368
  Description of Artificial Sequence: Synthetic primer

SEQ ID NO: 373 - DNA, 32 bp, Artificial Sequence
  Description of Artificial Sequence: Synthetic primer
gtggtgccgcggccagagttcctagggcagag

SEQ ID NO: 374 - DNA, 32 bp, Artificial Sequence
  Description of Artificial Sequence: Synthetic primer
gtggtgccgcggagctagtccccacattccac

SEQ ID NO: 375 - DNA, 32 bp, Artificial Sequence; identical to SEQ ID NO: 373
  Description of Artificial Sequence: Synthetic primer

SEQ ID NO: 376 - DNA, 32 bp, Artificial Sequence
  Description of Artificial Sequence: Synthetic primer
gtggtgccgcggggtggagggaaactttaggc

SEQ ID NO: 377 - DNA, 32 bp, Artificial Sequence; identical to SEQ ID NO: 352
  Description of Artificial Sequence: Synthetic primer

SEQ ID NO: 378 - DNA, 32 bp, Artificial Sequence; identical to SEQ ID NO: 374
  Description of Artificial Sequence: Synthetic primer

SEQ ID NO: 379 - DNA, 34 bp, Artificial Sequence
  Description of Artificial Sequence: Synthetic primer
gtggtgccgcggtctcatgcctggacaagtaact

SEQ ID NO: 380 - DNA, 32 bp, Artificial Sequence; identical to SEQ ID NO: 376
  Description of Artificial Sequence: Synthetic primer

SEQ ID NO: 381 - DNA, 32 bp, Artificial Sequence
  Description of Artificial Sequence: Synthetic primer
gtggtgccgcggggcttggacagaacttaccg

SEQ ID NO: 382 - DNA, 32 bp, Artificial Sequence
  Description of Artificial Sequence: Synthetic primer
gtggtgccgcggcaccactgtctgcctaagga

SEQ ID NO: 383 - DNA, 32 bp, Artificial Sequence; identical to SEQ ID NO: 381
  Description of Artificial Sequence: Synthetic primer

SEQ ID NO: 384 - DNA, 32 bp, Artificial Sequence; identical to SEQ ID NO: 376
  Description of Artificial Sequence: Synthetic primer

SEQ ID NO: 385 - DNA, 33 bp, Artificial Sequence
  Description of Artificial Sequence: Synthetic primer
gtggtgccgcggcgtagtgccaaaacaaacagt

SEQ ID NO: 386 - DNA, 32 bp, Artificial Sequence; identical to SEQ ID NO: 382
  Description of Artificial Sequence: Synthetic primer

SEQ ID NO: 387 - DNA, 33 bp, Artificial Sequence; identical to SEQ ID NO: 385
  Description of Artificial Sequence: Synthetic primer

SEQ ID NO: 388 - DNA, 32 bp, Artificial Sequence; identical to SEQ ID NO: 376
  Description of Artificial Sequence: Synthetic primer

SEQ ID NO: 389 - DNA, 32 bp, Artificial Sequence
  Description of Artificial Sequence: Synthetic primer
gtggtgccgcgggcgagggcctacttgatatg

SEQ ID NO: 390 - DNA, 32 bp, Artificial Sequence
  Description of Artificial Sequence: Synthetic primer
gtggtgccgcggcttcccaagtgaggcaatgc

SEQ ID NO: 391 - DNA, 33 bp, Artificial Sequence
  Description of Artificial Sequence: Synthetic primer
gtggtgccgcggacgttttgtgctgctgtaaca

SEQ ID NO: 392 - DNA, 32 bp, Artificial Sequence
  Description of Artificial Sequence: Synthetic primer
gtggtgccgcggctgcaggcacattctcttcc

SEQ ID NO: 393 - DNA, 32 bp, Artificial Sequence
  Description of Artificial Sequence: Synthetic primer
gtggtgccgcgggccctgtgtggtagtagtca

SEQ ID NO: 394 - DNA, 32 bp, Artificial Sequence; identical to SEQ ID NO: 390
  Description of Artificial Sequence: Synthetic primer

SEQ ID NO: 395 - DNA, 33 bp, Artificial Sequence
  Description of Artificial Sequence: Synthetic primer
gtggtgccgcggcagtattaaggggtgggagct

SEQ ID NO: 396 - DNA, 32 bp, Artificial Sequence
  Description of Artificial Sequence: Synthetic primer
gtggtgccgcggtctcttcctcacacagctga

SEQ ID NO: 397 - DNA, 32 bp, Artificial Sequence
  Description of Artificial Sequence: Synthetic primer
gtggtgccgcggggagcttggagggaagagaa

SEQ ID NO: 398 - DNA, 32 bp, Artificial Sequence; identical to SEQ ID NO: 390
  Description of Artificial Sequence: Synthetic primer

SEQ ID NO: 399 - DNA, 32 bp, Artificial Sequence
  Description of Artificial Sequence: Synthetic primer
gtggtgccgcggatggatggggaagacactgg

SEQ ID NO: 400 - DNA, 32 bp, Artificial Sequence; identical to SEQ ID NO: 392
  Description of Artificial Sequence: Synthetic primer

SEQ ID NO: 401 - DNA, 32 bp, Artificial Sequence
  Description of Artificial Sequence: Synthetic primer
gtggtgccgcggggatgaaacagggcaggaac

SEQ ID NO: 402 - DNA, 31 bp, Artificial Sequence
  Description of Artificial Sequence: Synthetic primer
gtggtgccgcggttcccaagtgaggcaatgc

SEQ ID NO: 403 - DNA, 32 bp, Artificial Sequence
  Description of Artificial Sequence: Synthetic primer
gtggtgccgcggtttgcagagccatgatgagg

SEQ ID NO: 404 - DNA, 30 bp, Artificial Sequence
  Description of Artificial Sequence: Synthetic primer
gtggtgccgcggcgacagccaaaacagccg

SEQ ID NO: 405 - DNA, 44 bp, Artificial Sequence
  Description of Artificial Sequence: Synthetic oligonucleotide
aaaatattttagctcctactcagactgttactctggtgacacaa

SEQ ID NO: 406 - DNA, 44 bp, Artificial Sequence
  Description of Artificial Sequence: Synthetic oligonucleotide
ttgtgtcaccagagtaacagtctgagtaggagctaaaatatttt

SEQ ID NO: 407 - DNA, 36 bp, Artificial Sequence
  Description of Artificial Sequence: Synthetic oligonucleotide
tagctcctactcagactgttactctggtgacacaac

SEQ ID NO: 408 - DNA, 28 bp, Artificial Sequence
  Description of Artificial Sequence: Synthetic oligonucleotide
tagctcctactcagactggtgacccaac

SEQ ID NO: 409 - DNA, 24 bp, Artificial Sequence
  Description of Artificial Sequence: Synthetic oligonucleotide
tagctcctactctggtgacacaac

SEQ ID NO: 410 - DNA, 28 bp, Artificial Sequence
  Description of Artificial Sequence: Synthetic oligonucleotide
tagctcctactcagactggtgacacaac

SEQ ID NO: 411 - DNA, 16 bp, Artificial Sequence
  Description of Artificial Sequence: Synthetic oligonucleotide
tagctcctactcagac

SEQ ID NO: 412 - DNA, 27 bp, Artificial Sequence
  Description of Artificial Sequence: Synthetic oligonucleotide
tagctcctactcagactgttacacaac

SEQ ID NO: 413 - DNA, 30 bp, Artificial Sequence
  Description of Artificial Sequence: Synthetic oligonucleotide
tagctcctactcagactgtggtgaggtgac

SEQ ID NO: 414 - DNA, 32 bp, Artificial Sequence
  Description of Artificial Sequence: Synthetic oligonucleotide
tagctcctactcagactctctggtgacacaac

SEQ ID NO: 415 - DNA, 31 bp, Artificial Sequence
  Description of Artificial Sequence: Synthetic oligonucleotide
tagctcctactcagacctctggtgacacaac

SEQ ID NO: 416 - DNA, 32 bp, Artificial Sequence
  Description of Artificial Sequence: Synthetic oligonucleotide
tagctcctactcaggctgtctggtgacacaac

SEQ ID NO: 417 - DNA, 33 bp, Artificial Sequence
  Description of Artificial Sequence: Synthetic oligonucleotide
tagctcctactcagactactctggtgacacaac

SEQ ID NO: 418 - DNA, 28 bp, Artificial Sequence
  Description of Artificial Sequence: Synthetic oligonucleotide
tagctcctactcagactgttgacacaac

SEQ ID NO: 419 - DNA, 13 bp, Artificial Sequence
  Description of Artificial Sequence: Synthetic oligonucleotide
ctggtgacacaac

SEQ ID NO: 420 - DNA, 29 bp, Artificial Sequence
  Description of Artificial Sequence: Synthetic oligonucleotide
tagctcctactcagactgttagacacaac

SEQ ID NO: 421 - DNA, 33 bp, Artificial Sequence
  Description of Artificial Sequence: Synthetic oligonucleotide
tagctcctactcagactgctctggtgacacaac

SEQ ID NO: 422 - DNA, 20 bp, Artificial Sequence
  Description of Artificial Sequence: Synthetic oligonucleotide
cagactgttactctggtgac

SEQ ID NO: 423 - DNA, 29 bp, Artificial Sequence
  Description of Artificial Sequence: Synthetic oligonucleotide
cagaccacctgtggtctcctactggtgac

SEQ ID NO: 424 - DNA, 18 bp, Artificial Sequence
  Description of Artificial Sequence: Synthetic oligonucleotide
gctttgatttccctaggg

SEQ ID NO: 425 - DNA, 25 bp, Artificial Sequence
  Description of Artificial Sequence: Synthetic oligonucleotide
gctttgatttccagttcttaggcaa

SEQ ID NO: 426 - DNA, 18 bp, Artificial Sequence
  Description of Artificial Sequence: Synthetic oligonucleotide
gctttgattcttaggcaa

SEQ ID NO: 427 - DNA, 62 bp, Artificial Sequence
  Description of Artificial Sequence: Synthetic oligonucleotide
  modified_base (13)..(53): a, c, t, g, unknown or other
gctttgatttccnnnnnnnnnnnnnnnnnnnnnnnnnnnnnnnnnnnnnnnnncttaggcaa

SEQ ID NO: 428 - DNA, 18 bp, Artificial Sequence
  Description of Artificial Sequence: Synthetic oligonucleotide
tcttaaccattaccatag

SEQ ID NO: 429 - DNA, 32 bp, Artificial Sequence
  Description of Artificial Sequence: Synthetic oligonucleotide
tcttaaccattaccatagagttcttaggcaac

SEQ ID NO: 430 - DNA, 30 bp, Artificial Sequence
  Description of Artificial Sequence: Synthetic oligonucleotide
tcttaaccattaccaaagttcttaggcaac

SEQ ID NO: 431 - DNA, 31 bp, Artificial Sequence
  Description of Artificial Sequence: Synthetic oligonucleotide
tcttaaccattaccataggttcttaggcaac

SEQ ID NO: 432 - DNA, 14 bp, Artificial Sequence
  Description of Artificial Sequence: Synthetic oligonucleotide
gaaccaaacccact

SEQ ID NO: 433 - DNA, 24 bp, Artificial Sequence
  Description of Artificial Sequence: Synthetic oligonucleotide
gaaccaaacccacttaggggataa

SEQ ID NO: 434 - DNA, 2328 bp, Artificial Sequence
  Description of Artificial Sequence: Synthetic polynucleotide
atgaggtctgactacaaagaccatgacggtgattataaagatcatgacatcgattacaaggatgacgatgacaagatggcccccaagaagaagaggaaggtgggcctcgagcccggagaaaaaccgtacaagtgccctgagtgcgggaaatcattctccgaccctggggcgctcgtccggcaccaaaggacgcatacaggggaaaagccgtataagtgccccgagtgtggaaagagcttctcgcagagagcccaccttgaacgacaccaaagaacacacactggtgagaaaccctataagtgtccagagtgcggcaaatcgtttagcagatccgatgacttggtgcgccaccagcggacacacacgggtgaaaagccctacaaatgcccggagtgtgggaagtcgttttcaaggtcggatcatctgactacccatcagcgcacccatacgggagcggccgcccgcgccctggtgaagagcgagctggaggagaagaagtccgagctgcggcacaagctgaagtacgtgccccacgagtacatcgagctgatcgagatcgccaggaaccccacccaggaccgcatcctggagatgaaggtgatggagttcttcatgaaggtgtacggctacaggggagagcacctgggcggaagcagaaagcctgacggcgccatctatacagtgggcagccccatcgattacggcgtgatcgtggacacaaaggcctacagcggcggctacaatctgcctatcggccaggccgacgagatgcagagatacgtgaaggagaaccagacccggaataagcacatcaaccccaacgagtggtggaaggtgtaccctagcagcgtgaccgagttcaagttcctgttcgtgagcggccacttcaagggcaactacaaggcccagctgaccaggctgaaccgcaaaaccaactgcaatggcgccgtgctgagcgtggaggagctgctgatcggcggcgagatgatcaaagccggcaccctgacactggaggaggtgcggcgcaagttcaacaacggcgagatcaacttcgagggcagaggaagtcttctaacatgcggtgacgtggaggagaatcccggccctagatctgactacaaagaccatgacggtgattataaagatcatgacatcgattacaaggatgacgatgacaagatggcccccaagaagaagaggaaggtgggcctcgagccgggagagaagccgtacaagtgtcccgaatgtggaaagagcttctcacagtcgggggaccttcggcgccaccagcgcacacatactggtgaaaagccgtataagtgtccagaatgtggcaaatcattctccacatcagggagcctggtcaggcaccagcgaacccacacgggtgagaagccctataagtgccccgaatgcgggaagtccttttcgcagagagcccacttggagaggcaccagaggacccatacgggggagaaaccttacaagtgccctgaatgcggaaagtcgttctcgacccatctggatctcatcagacatcagagaacgcacactggagagaaaccctacaaatgtcccgagtgtgggaagtcgtttagccgaaaggacaatctcaaaaaccatcaacggacacacacgggtgaaaaaccatacaaatgcccggagtgcggcaaatcgttttcccaacttgcgcacttgcgggcacaccaacgcacgcatactggagcggccgcccgcgccctggtgaagagcgagctggaggagaagaagtccgagctgcggcacaagctgaagtacgtgccccacgagtacatcgagctgatcgagatcgccaggaaccccacccaggaccgcatcctggagatgaaggtgatggagttcttcatgaaggtgtacggctacaggggagagcacctgggcggaagcagaaagcctgacggcgccatctatacagtgggcagccccatcgattacggcgtgatcgtggacacaaaggcctacagcggcggctacaatctgcctatcggccaggccgacgagatggagagatacgtggaggagaaccagacacgggataagcacctcaaccccaacgagtggtggaaggtgtaccctagcagcgtgaccgagttcaagttcctgttcgtgagcggccacttcaagggcaactacaaggcccagctgaccaggctgaaccacatcaccaactgcaatggcgccgtgctgagcgtggaggagctgctgatcggcggcgagatgatcaaagccggcaccctgacactggaggaggtgcggcgcaagttcaacaacggcgagatcaacttctga

SEQ ID NO: 435 - protein, 775 aa, Artificial Sequence
  Description of Artificial Sequence: Synthetic polypeptide
MRSDYKDHDGDYKDHDIDYKDDDDKMAPKKKRKVGLEPGEKPYKCPECGKSFSDPGALVRHQRTHTGEKPYKCPECGKSFSQRAHLERHQRTHTGEKPYKCPECGKSFSRSDDLVRHQRTHTGEKPYKCPECGKSFSRSDHLTTHQRTHTGAAARALVKSELEEKKSELRHKLKYVPHEYIELIEIARNPTQDRILEMKVMEFFMKVYGYRGEHLGGSRKPDGAIYTVGSPIDYGVIVDTKAYSGGYNLPIGQADEMQRYVKENQTRNKHINPNEWWKVYPSSVTEFKFLFVSGHFKGNYKAQLTRLNRKTNCNGAVLSVEELLIGGEMIKAGTLTLEEVRRKFNNGEINFEGRGSLLTCGDVEENPGPRSDYKDHDGDYKDHDIDYKDDDDKMAPKKKRKVGLEPGEKPYKCPECGKSFSQSGDLRRHQRTHTGEKPYKCPECGKSFSTSGSLVRHQRTHTGEKPYKCPECGKSFSQRAHLERHQRTHTGEKPYKCPECGKSFSTHLDLIRHQRTHTGEKPYKCPECGKSFSRKDNLKNHQRTHTGEKPYKCPECGKSFSQLAHLRAHQRTHTGAAARALVKSELEEKKSELRHKLKYVPHEYIELIEIARNPTQDRILEMKVMEFFMKVYGYRGEHLGGSRKPDGAIYTVGSPIDYGVIVDTKAYSGGYNLPIGQADEMERYVEENQTRDKHLNPNEWWKVYPSSVTEFKFLFVSGHFKGNYKAQLTRLNHITNCNGAVLSVEELLIGGEMIKAGTLTLEEVRRKFNNGEINF

SEQ ID NO: 436 - DNA, 4725 bp, Artificial Sequence
  Description of Artificial Sequence: Synthetic polynucleotide
tggccactccctctatgcgcactcgctcgctcggtggggcctggcgaccaaaggtcgccagacggacgtgctttgcacgtccggccccaccgagcgagcgagtgcgcatagagggagtggccaactccatcactagaggtatggcagtgacgtaacgcgaagcgcgcgaagcgagaccacgcctaccagctgcgtcagcagtcaggtgacccttttgcgacagtttgcgacaccacgtggccgctgagggtatatattctcgagtgagcgaaccaggagctccattttgaccgcgaaatttgaacgagcagcagccatgccggggttctacgagattgtcctgaaggtcccgagtgacctggacgagcacctgccgggcatttctaactcgtttgttaactgggtggccgagaaggaatgggagctgccgccggattctgacatggatccgaatctgattgagcaggcacccctgaccgtggccgaaaagcttcagcgcgagttcctggtggagtggcgccgcgtgagtaaggccccggaggccctcttttttgtccagttcgaaaagggggagacctacttccacctgcacgtgctgattgagaccatcggggtcaaatccatggtggtcggccgctacgtgagccagattaaagagaagctggtgacccgcatctaccgcggggtcgagccgcagcttccgaactggttcgcggtgaccaaaacgcgaaatggcgccgggggcgggaacaaggtggtggacgactgctacatccccaactacctgctccccaagacccagcccgagctccagtgggcgtggactaacatggaccagtatttaagcgcctgtttgaatctcgcggagcgtaaacggctggtggcgcagcatctgacgcacgtgtcgcagacgcaggagcagaacaaagagaatcagaaccccaattctgacgcgccggtcatcaggtcaaaaacctcagccaggtacatggagctggtcgggtggctggtggaccgcgggatcacgtcagaaaagcaatggattcaggaggaccaggcctcgtacatctccttcaacgccgcctccaactcgcggtcccagatcaaggccgcgctggacaatgcctccaagatcatgagcctgacaaagacggctccggactacctggtgggcagcaacccgccggaggacattaccaaaaatcggatctaccaaatcctggagctgaacgggtacgatccgcagtacgcggcctccgtcttcctgggctgggcgcaaaagaagttcgggaagaggaacaccatctggctctttgggccggccacgacgggtaaaaccaacatcgcggaagccatcgcccacgccgtgcccttctacggctgcgtaaactggaccaatgagaactttcccttcaacgattgcgtcgacaagatggtgatctggtgggaggagggcaagatgacggccaaggtcgtggagagcgccaaggccattctgggcggaagcaaggtgcgcgtggaccaaaagtgcaagtcatcggcccagatcgaacccactcccgtgatcgtcacctccaacaccaacatgtgcgccgtgattgacgggaacagcaccaccttcgagcatcagcagccgctgcaggaccggatgtttaaatttgaacttacccgccgtttggaccatgactttgggaaggtcaccaaacaggaagtaaaggactttttccggtgggcttccgatcacgtgactgacgtggctcatgagttctacgtcagaaagggtggagctaagaaacgccccgcctccaatgacgcggatgtaagcgagccaaaacggcagtgcacgtcacttgcgcagccgacaacgtcagacgcggaagcaccggcggactacgcggacaggtaccaaaacaaatgttctcgtcacgtgggcatgaatctgatgctttttccctgtaaaacatgcgagagaatgaatcaaatttccaatgtctgttttacgcatggtcaaagagactgtggggaatgcttccctggaatgtcagaatctcaacccgtttctgtcgtcaaaaagaagacttatcagaaactgtgtccaattcatcatatcctgggaagggcacccgagattgcctgttcggcctgcgatttggccaatgtggacttggatgactgtgtttctgagcaataaatgacttaaaccaggtatggctgctgacggttatcttccagattggctcgaggacaacctttctgaaggcattcgtgagtggtgggctctgaaacctggagtccctcaacccaaagcgaaccaacaacaccaggacaaccgtcggggtcttgtgcttccgggttacaaatacctcggacccggtaacggactcgacaaaggagagccggtcaacgaggcggacgcggcagccctcgaacacgacaaagcttacgaccagcagctcaaggccggtgacaacccgtacctcaagtacaaccacgccgacgccgagtttcaggagcgtcttcaagaagatacgtcttttgggggcaaccttggcagagcagtcttccaggccaaaaagaggatccttgagcctcttggtctggttgaggaagcagctaaaacggctcctggaaagaagaggcctgtagatcagtctcctcaggaaccggactcatcatctggtgttggcaaatcgggcaaacagcctgccagaaaaagactaaatttcggtcagactggcgactcagagtcagtcccagaccctcaacctctcggagaaccaccagcagcccccacaagtttgggatctaatacaatggcttcaggcggtggcgcaccaatggcagacaataacgagggtgccgatggagtgggtaattcctcaggaaattggcattgcgattcccaatggctgggcgacagagtcatcaccaccagcaccagaacctgggccctgcccacttacaacaaccatctctacaagcaaatctccagcgcttcaacgggagcttcaaacgacaaccactactttggctacagcaccccttgggggtattttgactttaacagattccactgccacttctcaccacgtgactggcagcgactcattaacaacaactggggattccggcccaagaaactcagcttcaagctcttcaacatccaagttaaagaggtcacgcagaacgatggcacgacgactattgccaataaccttaccagcacggttcaagtgtttacggactcggagtatcagctcccgtacgtgctcgggtcggcgcaccaaggctgtctcccgccgtttccagcggacgtcttcatggtccctcagtatggatacctcaccctgaacaacggaagtcaagcggtgggacgctcatccttttactgcctggagtacttcccttcgcagatgctaaggactggaaataacttccaattcagctataccttcgaggatgtaccttttcacagcagctacgctcacagccagagtttggatcgcttgatgaatcctcttattgatcagtatctgtactacctgaacagaacgcaaggaacaacctctggaacaaccaaccaatcacggctgctttttagccaggctgggcctcagtctatgtctttgcaggccagaaattggctacctgggccctgctaccggcaacagagactttcaaagactgctaacgacaacaacaacagtaactttccttggacagcggccagcaaatatcatctcaatggccgcgactcgctggtgaatccaggaccagctatggccagtcacaaggacgatgaagaaaaatttttccctatgcacggcaatctaatatttggcaaagaagggacaacggcaagtaacgcagaattagataatgtaatgattacggatgaagaagagattcgtaccaccaatcctgtggcaacagagcagtatggaactgtggcaaataacttgcagagctcaaatacagctcccacgactagaactgtcaatgatcagggggccttacctggcatggtgtggcaagatcgtgacgtgtaccttcaaggacctatctgggcaaagattcctcacacggatggacactttcatccttctcctctgatgggaggctttggactgaaacatccgcctcctcaaatcatgatcaaaaatactccggtaccggcaaatcctccgacgactttcagcccggccaagtttgcttcatttatcactcagtactccactggacaggtcagcgtggaaattgagtgggagctacagaaagaaaacagcaaacgttggaatccagagattcagtacacttccaactacaacaagtctgttaatgtggactttactgtagacactaatggtgtttatagtgaacctcgccctattggaacccggtatctcacacgaaacttgtaatcctggttaatcaataaaccgtttaattcgtttcagttgaactttggctcttgtgcacttcttatcttatcttgtttccatggctactgcgtagataagcagcggcctgcggcgcttgcgcttcgcggtttacaactgctggttaatatttaactctcgccatacctctagtgatggagttggccactccctctatgcgcactcgctcgctcggtggggccggacgtgcaaagcacgtccgtctggcgacctttggtcgccaggccccaccgagcgagcgagtgcgcatagagggagtggccaa

SEQ ID NO: 437 - protein, 737 aa, Artificial Sequence
  Description of Artificial Sequence: Synthetic polypeptide
MAADGYLPDWLEDNLSEGIREWWALKPGVPQPKANQQHQDNRRGLVLPGYKYLGPGNGLDKGEPVNEADAAALEHDKAYDQQLKAGDNPYLKYNHADAEFQERLQEDTSFGGNLGRAVFQAKKRILEPLGLVEEAAKTAPGKKRPVDQSPQEPDSSSGVGKSGKQPARKRLNFGQTGDSESVPDPQPLGEPPAAPTSLGSNTMASGGGAPMADNNEGADGVGNSSGNWHCDSQWLGDRVITTSTRTWALPTYNNHLYKQISSASTGASNDNHYFGYSTPWGYFDFNRFHCHFSPRDWQRLINNNWGFRPKKLSFKLFNIQVKEVTQNDGTTTIANNLTSTVQVFTDSEYQLPYVLGSAHQGCLPPFPADVFMVPQYGYLTLNNGSQAVGRSSFYCLEYFPSQMLRTGNNFQFSYTFEDVPFHSSYAHSQSLDRLMNPLIDQYLYYLNRTQGTTSGTTNQSRLLFSQAGPQSMSLQARNWLPGPCYRQQRLSKTANDNNNSNFPWTAASKYHLNGRDSLVNPGPAMASHKDDEEKFFPMHGNLIFGKEGTTASNAELDNVMITDEEEIRTTNPVATEQYGTVANNLQSSNTAPTTRTVNDQGALPGMVWQDRDVYLQGPIWAKIPHTDGHFHPSPLMGGFGLKHPPPQIMIKNTPVPANPPTTFSPAKFASFITQYSTGQVSVEIEWELQKENSKRWNPEIQYTSNYNKSVNVDFTVDTNGVYSEPRPIGTRYLTRNL

SEQ ID NO: 438 - protein, 406 aa, Artificial Sequence
  Description of Artificial Sequence: Synthetic polypeptide
MDYKDHDGDYKDHDIDYKDDDDKMAPKKKRKVGRLEPGEKPYKCPECGKSFSRKDALRGHQRTHTGEKPYKCPECGKSFSHRTTLTNHQRTHTGEKPYKCPECGKSFSQRNALAGHQRTHTGEKPYKCPECGKSFSHKNALQNHQRTHTGEKPYKCPECGKSFSDPGHLVRHQRTHTGEKPYKCPECGKSFSTSGNLVRHQRTHTGAAARALVKSELEEKKSELRHKLKYVPHEYIELIEIARNPTQDRILEMKVMEFFMKVYGYRGEHLGGSRKPDGAIYTVGSPIDYGVIVDTKAYSGGYNLPIGQADEMERYVEENQTRDKHLNPNEWWKVYPSSVTEFKFLFVSGHFKGNYKAQLTRLNHITNCNGAVLSVEELLIGGEMIKAGTLTLEEVRRKFNNGEINF

SEQ ID NO: 439 - protein, 406 aa, Artificial Sequence
  Description of Artificial Sequence: Synthetic polypeptide
MDYKDHDGDYKDHDIDYKDDDDKMAPKKKRKVGRLEPGEKPYKCPECGKSFSQQRSLVGHQRTHTGEKPYKCPECGKSFSDKKDLTRHQRTHTGEKPYKCPECGKSFSTSGHLVRHQRTHTGEKPYKCPECGKSFSQRAHLERHQRTHTGEKPYKCPECGKSFSTSGSLVRHQRTHTGEKPYKCPECGKSFSTSGNLVRHQRTHTGAAARALVKSELEEKKSELRHKLKYVPHEYIELIEIARNPTQDRILEMKVMEFFMKVYGYRGEHLGGSRKPDGAIYTVGSPIDYGVIVDTKAYSGGYNLPIGQADEMQRYVKENQTRNKHINPNEWWKVYPSSVTEFKFLFVSGHFKGNYKAQLTRLNRKTNCNGAVLSVEELLIGGEMIKAGTLTLEEVRRKFNNGEINF

SEQ ID NO: 440 - protein, 320 aa, Artificial Sequence
  Description of Artificial Sequence: Synthetic polypeptide
MDYKDHDGDYKDHDIDYKDDDDKMAPKKKRKVGRLEPGERPFQCRICMRNFSSKQALAVHTRTHTGEKPFQCRICMRNFSQSTTLKRHLRTHTGEKPFQCRICMRNFSRSDHLSLHLKTHLRGSQLVKSELEEKKSELRHKLKYVPHEYIELIEIARNPTQDRILEMKVMEFFMKVYGYRGEHLGGSRKPDGAIYTVGSPIDYGVIVDTKAYSGGYNLPIGQADEMQRYVKENQTRNKHINPNEWWKVYPSSVTEFKFLFVSGHFKGNYKAQLTRLNRKTNCNGAVLSVEELLIGGEMIKAGTLTLEEVRRKFNNGEINF

SEQ ID NO: 441 - protein, 320 aa, Artificial Sequence
  Description of Artificial Sequence: Synthetic polypeptide
MDYKDHDGDYKDHDIDYKDDDDKMAPKKKRKVGRLEPGERPFQCRICMRNFSRRAHLQNHTRTHTGEKPFQCRICMRNFSQSTTLKRHLRTHTGEKPFQCRICMRNFSDGGHLTRHLKTHLRGSQLVKSELEEKKSELRHKLKYVPHEYIELIEIARNPTQDRILEMKVMEFFMKVYGYRGEHLGGSRKPDGAIYTVGSPIDYGVIVDTKAYSGGYNLPIGQADEMERYVEENQTRDKHLNPNEWWKVYPSSVTEFKFLFVSGHFKGNYKAQLTRLNHITNCNGAVLSVEELLIGGEMIKAGTLTLEEVRRKFNNGEINF

SEQ ID NO: 442 - DNA, 42 bp, Artificial Sequence
  Description of Artificial Sequence: Synthetic oligonucleotide
caaactagaaatgccatcttccttgatgttggaggtacctgc

SEQ ID NO: 443 - protein, 406 aa, Artificial Sequence; identical to SEQ ID NO: 438
  Description of Artificial Sequence: Synthetic polypeptide

SEQ ID NO: 444 - protein, 406 aa, Artificial Sequence; identical to SEQ ID NO: 439
  Description of Artificial Sequence: Synthetic polypeptide

SEQ ID NO: 445 - DNA, 25 bp, Artificial Sequence
  Description of Artificial Sequence: Synthetic oligonucleotide
  misc_feature (1)..(1): May or may not be present
  misc_feature (25)..(25): May or may not be present
tatctgcccatgactggcgcaggga

SEQ ID NO: 446 - protein, 320 aa, Artificial Sequence; identical to SEQ ID NO: 440
  Description of Artificial Sequence: Synthetic polypeptide

SEQ ID NO: 447 - protein, 320 aa, Artificial Sequence; identical to SEQ ID NO: 441
  Description of Artificial Sequence: Synthetic polypeptide

SEQ ID NO: 448 - DNA, 42 bp, Artificial Sequence
  Description of Artificial Sequence: Synthetic oligonucleotide
actagaaatgccatcttccttgatgttggaggtacctgctct

SEQ ID NO: 449 - protein, 406 aa, Artificial Sequence
  Description of Artificial Sequence: Synthetic polypeptide
MDYKDHDGDYKDHDIDYKDDDDKMAPKKKRKVGRLEPGEKPYKCPECGKSFSHRTTLTNHQRTHTGEKPYKCPECGKSFSQRNALAGHQRTHTGEKPYKCPECGKSFSHKNALQNHQRTHTGEKPYKCPECGKSFSDPGHLVRHQRTHTGEKPYKCPECGKSFSTSGNLVRHQRTHTGEKPYKCPECGKSFSQSSNLVRHQRTHTGAAARALVKSELEEKKSELRHKLKYVPHEYIELIEIARNPTQDRILEMKVMEFFMKVYGYRGEHLGGSRKPDGAIYTVGSPIDYGVIVDTKAYSGGYNLPIGQADEMERYVEENQTRDKHLNPNEWWKVYPSSVTEFKFLFVSGHFKGNYKAQLTRLNHITNCNGAVLSVEELLIGGEMIKAGTLTLEEVRRKFNNGEINF

SEQ ID NO: 450 - protein, 406 aa, Artificial Sequence
  Description of Artificial Sequence: Synthetic polypeptide
MDYKDHDGDYKDHDIDYKDDDDKMAPKKKRKVGRLEPGEKPYKCPECGKSFSQRNALAGHQRTHTGEKPYKCPECGKSFSQQRSLVGHQRTHTGEKPYKCPECGKSFSDKKDLTRHQRTHTGEKPYKCPECGKSFSTSGHLVRHQRTHTGEKPYKCPECGKSFSQRAHLERHQRTHTGEKPYKCPECGKSFSTSGSLVRHQRTHTGAAARALVKSELEEKKSELRHKLKYVPHEYIELIEIARNPTQDRILEMKVMEFFMKVYGYRGEHLGGSRKPDGAIYTVGSPIDYGVIVDTKAYSGGYNLPIGQADEMQRYVKENQTRNKHINPNEWWKVYPSSVTEFKFLFVSGHFKGNYKAQLTRLNRKTNCNGAVLSVEELLIGGEMIKAGTLTLEEVRRKFNNGEINF

SEQ ID NO: 451 - protein, 378 aa, Artificial Sequence
  Description of Artificial Sequence: Synthetic polypeptide
MDYKDHDGDYKDHDIDYKDDDDKMAPKKKRKVGRLEPGEKPYKCPECGKSFSQRNALAGHQRTHTGEKPYKCPECGKSFSHKNALQNHQRTHTGEKPYKCPECGKSFSDPGHLVRHQRTHTGEKPYKCPECGKSFSTSGNLVRHQRTHTGEKPYKCPECGKSFSQSSNLVRHQRTHTGAAARALVKSELEEKKSELRHKLKYVPHEYIELIEIARNPTQDRILEMKVMEFFMKVYGYRGEHLGGSRKPDGAIYTVGSPIDYGVIVDTKAYSGGYNLPIGQADEMERYVEENQTRDKHLNPNEWWKVYPSSVTEFKFLFVSGHFKGNYKAQLTRLNHITNCNGAVLSVEELLIGGEMIKAGTLTLEEVRRKFNNGEINF

SEQ ID NO: 452 - protein, 378 aa, Artificial Sequence
  Description of Artificial Sequence: Synthetic polypeptide
MDYKDHDGDYKDHDIDYKDDDDKMAPKKKRKVGRLEPGEKPYKCPECGKSFSQQRSLVGHQRTHTGEKPYKCPECGKSFSDKKDLTRHQRTHTGEKPYKCPECGKSFSTSGHLVRHQRTHTGEKPYKCPECGKSFSQRAHLERHQRTHTGEKPYKCPECGKSFSTSGSLVRHQRTHTGAAARALVKSELEEKKSELRHKLKYVPHEYIELIEIARNPTQDRILEMKVMEFFMKVYGYRGEHLGGSRKPDGAIYTVGSPIDYGVIVDTKAYSGGYNLPIGQADEMQRYVKENQTRNKHINPNEWWKVYPSSVTEFKFLFVSGHFKGNYKAQLTRLNRKTNCNGAVLSVEELLIGGEMIKAGTLTLEEVRRKFNNGEINF

SEQ ID NO: 453 - DNA, 26 bp, Artificial Sequence
  Description of Artificial Sequence: Synthetic oligonucleotide
  misc_feature (1)..(1): May or may not be present
  misc_feature (26)..(26): May or may not be present
tgccatcttccttgatgttggaggta

SEQ ID NO: 454 - protein, 322 aa, Artificial Sequence
  Description of Artificial Sequence: Synthetic polypeptide
MDYKDHDGDYKDHDIDYKDDDDKMAPKKKRKVGRLEPGERPFQCRICMRNFSSPSKLARHTRTHTGEKPFQCRICMRNFSVRHNLTRHLRTHTGEKPFQCRICMRNFSQRNNLGRHLKTHTGAAARALVKSELEEKKSELRHKLKYVPHEYIELIEIARNPTQDRILEMKVMEFFMKVYGYRGEHLGGSRKPDGAIYTVGSPIDYGVIVDTKAYSGGYNLPIGQADEMQRYVKENQTRNKHINPNEWWKVYPSSVTEFKFLFVSGHFKGNYKAQLTRLNRKTNCNGAVLSVEELLIGGEMIKAGTLTLEEVRRKFNNGEINF

SEQ ID NO: 455 - protein, 322 aa, Artificial Sequence
  Description of Artificial Sequence: Synthetic polypeptide
MDYKDHDGDYKDHDIDYKDDDDKMAPKKKRKVGRLEPGERPFQCRICMRNFSIPNHLARHTRTHTGEKPFQCRICMRNFSQSAHLKRHLRTHTGEKPFQCRICMRNFSHHNSLTRHLKTHTGAAARALVKSELEEKKSELRHKLKYVPHEYIELIEIARNPTQDRILEMKVMEFFMKVYGYRGEHLGGSRKPDGAIYTVGSPIDYGVIVDTKAYSGGYNLPIGQADEMERYVEENQTRDKHLNPNEWWKVYPSSVTEFKFLFVSGHFKGNYKAQLTRLNHITNCNGAVLSVEELLIGGEMIKAGTLTLEEVRRKFNNGEINF

SEQ ID NO: 456 - DNA, 6626 bp, Artificial Sequence
  Description of Artificial Sequence: Synthetic polynucleotide
ggggggggggggggggggttggccactccctctctgcgcgctcgctcgctcactgaggccgggcgaccaaaggtcgcccgacgcccgggctttgcccgggcggcctcagtgagcgagcgagcgcgcagagagggagtggccaactccatcactaggggttcctagatctgaattcggtacccgttacataacttacggtaaatggcccgcctggctgaccgcccaacgacccccgcccattgacgtcaataatgacgtatgttcccatagtaacgccaatagggactttccattgacgtcaatgggtggagtatttacggtaaactgcccacttggcagtacatcaagtgtatcatatgccaagtacgccccctattgacgtcaatgacggtaaatggcccgcctggcattatgcccagtacatgaccttatgggactttcctacttggcagtacatctacgtattagtcatcgctattaccatggtgatgcggttttggcagtacatcaatgggcgtggatagcggtttgactcacggggatttccaagtctccaccccattgacgtcaatgggagtttgttttggcaccaaaatcaacgggactttccaaaatgtcgtaacaactccgccccattgacgcaaatgggcggtaggcgtgtacggtgggaggtctatataagcagagctcgtttagtgaaccgtcagatcgcctggagacgccatccacgctgttttgacctccatagaagacaccgggaccgatccagcctccggactctagaggatccggtactcgaggaactgaaaaaccagaaagttaactggtaagtttagtctttttgtcttttatttcaggtcccggatccggtggtggtgcaaatcaaagaactgctcctcagtggatgttgcctttacttctaggcctgtacggaagtgttacttctgctctaaaagctgcggaattgtacccgcggcccgggatccaccggtggctagcgtctataggcccacccccttggtggaattcgccatgaggtctgactacaaagaccatgacggtgattataaagatcatgacatcgattacaaggatgacgatgacaagatggcccccaagaagaagaggaaggtgggcctcgagcccggagaaaaaccgtacaagtgccctgagtgcgggaaatcattctccgaccctggggcgctcgtccggcaccaaaggacgcatacaggggaaaagccgtataagtgccccgagtgtggaaagagcttctcgcagagagcccaccttgaacgacaccaaagaacacacactggtgagaaaccctataagtgtccagagtgcggcaaatcgtttagcagatccgatgacttggtgcgccaccagcggacacacacgggtgaaaagccctacaaatgcccggagtgtgggaagtcgttttcaaggtcggatcatctgactacccatcagcgcacccatacgggagcggccgcccgcgccctggtgaagagcgagctggaggagaagaagtccgagctgcggcacaagctgaagtacgtgccccacgagtacatcgagctgatcgagatcgccaggaaccccacccaggaccgcatcctggagatgaaggtgatggagttcttcatgaaggtgtacggctacaggggagagcacctgggcggaagcagaaagcctgacggcgccatctatacagtgggcagccccatcgattacggcgtgatcgtggacacaaaggcctacagcggcggctacaatctgcctatcggccaggccgacgagatgcagagatacgtgaaggagaaccagacccggaataagcacatcaaccccaacgagtggtggaaggtgtaccctagcagcgtgaccgagttcaagttcctgttcgtgagcggccacttcaagggcaactacaaggcccagctgaccaggctgaaccgcaaaaccaactgcaatggcgccgtgctgagcgtggaggagctgctgatcggcggcgagatgatcaaagccggcaccctgacactggaggaggtgcggcgcaagttcaacaacggcgagatcaacttcgagggcagaggaagtcttctaacatgcggtgacgtggaggagaatcccggccctagatctgactacaaagaccatgacggtgattataaagatcatgacatcgattacaaggatgacgatgacaagatggcccccaagaagaagaggaaggtgggcctcgagccgggagagaagccgtacaagtgtcccgaatgtggaaagagcttctcacagtcgggggaccttcggcgccaccagcgcacacatactggtgaaaagccgtataagtgtccagaatgtggcaaatcattctccacatcagggagcctggtcaggcaccagcgaacccacacgggtgagaagccctataagtgccccgaatgcgggaagtccttttcgcagagagcccacttggagaggcaccagaggacccatacgggggagaaaccttacaagtgccctgaatgcggaaagtcgttctcgacccatctggatctcatcagacatcagagaacgcacactggagagaaaccctacaaatgtcccgagtgtgggaagtcgtttagccgaaaggacaatctcaaaaaccatcaacggacacacacgggtgaaaaaccatacaaatgcccggagtgcggcaaatcgttttcccaacttgcgcacttgcgggcacaccaacgcacgcatactggagcggccgcccgcgccctggtgaagagcgagctggaggagaagaagtccgagctgcggcacaagctgaagtacgtgccccacgagtacatcgagctgatcgagatcgccaggaaccccacccaggaccgcatcctggagatgaaggtgatggagttcttcatgaaggtgtacggctacaggggagagcacctgggcggaagcagaaagcctgacggcgccatctatacagtgggcagccccatcgattacggcgtgatcgtggacacaaaggcctacagcggcggctacaatctgcctatcggccaggccgacgagatggagagatacgtggaggagaaccagacacgggataagcacctcaaccccaacgagtggtggaaggtgtaccctagcagcgtgaccgagttcaagttcctgttcgtgagcggccacttcaagggcaactacaaggcccagctgaccaggctgaaccacatcaccaactgcaatggcgccgtgctgagcgtggaggagctgctgatcggcggcgagatgatcaaagccggcaccctgacactggaggaggtgcggcgcaagttcaacaacggcgagatcaacttctgattaattaactaatctagagtcgactagagctcgctgatcagcctcgactgtgccttctagttgccagccatctgttgtttgcccctcccccgtgccttccttgaccctggaaggtgccactcccactgtcctttcctaataaaatgaggaaattgcatcgcattgtctgagtaggtgtcattctattctggggggtggggtggggcaggacagcaagggggaggattgggaagacaatagcaggcatgctggggagagatctaggaacccctagtgatggagttggccactccctctctgcgcgctcgctcgctcactgaggccgcccgggcaaagcccgggcgtcgggcgacctttggtcgcccggcctcagtgagcgagcgagcgcgcagagagggagtggccaacccccccccccccccccctgcagcccagctgcattaatgaatcggccaacgcgcggggagaggcggtttgcgtattgggcgctcttccgcttcctcgctcactgactcgctgcgctcggtcgttcggctgcggcgagcggtatcagctcactcaaaggcggtaatacggttatccacagaatcaggggataacgcaggaaagaacatgtgagcaaaaggccagcaaaaggccaggaaccgtaaaaaggccgcgttgctggcgtttttccataggctccgcccccctgacgagcatcacaaaaatcgacgctcaagtcagaggtggcgaaacccgacaggactataaagataccaggcgtttccccctggaagctccctcgtgcgctctcctgttccgaccctgccgcttaccggatacctgtccgcctttctcccttcgggaagcgtggcgctttctcaatgctcacgctgtaggtatctcagttcggtgtaggtcgttcgctccaagctgggctgtgtgcacgaaccccccgttcagcccgaccgctgcgccttatccggtaactatcgtcttgagtccaacccggtaagacacgacttatcgccactggcagcagccactggtaacaggattagcagagcgaggtatgtaggcggtgctacagagttcttgaagtggtggcctaactacggctacactagaaggacagtatttggtatctgcgctctgctgaagccagttaccttcggaaaaagagttggtagctcttgatccggcaaacaaaccaccgctggtagcggtggtttttttgtttgcaagcagcagattacgcgcagaaaaaaaggatctcaagaagatcctttgatcttttctacggggtctgacgctcagtggaacgaaaactcacgttaagggattttggtcatgagattatcaaaaaggatcttcacctagatccttttaaattaaaaatgaagttttaaatcaatctaaagtatatatgagtaaacttggtctgacagttaccaatgcttaatcagtgaggcacctatctcagcgatctgtctatttcgttcatccatagttgcctgactccccgtcgtgtagataactacgatacgggagggcttaccatctggccccagtgctgcaatgataccgcgagacccacgctcaccggctccagatttatcagcaataaaccagccagccggaagggccgagcgcagaagtggtcctgcaactttatccgcctccatccagtctattaattgttgccgggaagctagagtaagtagttcgccagttaatagtttgcgcaacgttgttgccattgctacaggcatcgtggtgtcacgctcgtcgtttggtatggcttcattcagctccggttcccaacgatcaaggcgagttacatgatcccccatgttgtgcaaaaaagcggttagctccttcggtcctccgatcgttgtcagaagtaagttggccgcagtgttatcactcatggttatggcagcactgcataattctcttactgtcatgccatccgtaagatgcttttctgtgactggtgagtactcaaccaagtcattctgagaatagtgtatgcggcgaccgagttgctcttgcccggcgtcaatacgggataataccgcgccacatagcagaactttaaaagtgctcatcattggaaaacgttcttcggggcgaaaactctcaaggatcttaccgctgttgagatccagttcgatgtaacccactcgtgcacccaactgatcttcagcatcttttactttcaccagcgtttctgggtgagcaaaaacaggaaggcaaaatgccgcaaaaaagggaataagggcgacacggaaatgttgaatactcatactcttcctttttcaatattattgaagcatttatcagggttattgtctcatgagcggatacatatttgaatgtatttagaaaaataaacaaataggggttccgcgcacatttccccgaaaagtgccacctgacgtctaagaaaccattattatcatgacattaacctataaaaataggcgtatcacgaggccctttcgtctcgcgcgtttcggtgatgacggtgaaaacctctgacacatgcagctcccggagacggtcacagcttgtctgtaagcggatgccgggagcagacaagcccgtcagggcgcgtcagcgggtgttggcgggtgtcggggctggcttaactatgcggcatcagagcagattgtactgagagtgcaccatatgcggtgtgaaataccgcacagatgcgtaaggagaaaataccgcatcaggaaattgtaaacgttaatattttgttaaaattcgcgttaaatttttgttaaatcagctcattttttaaccaataggccgaaatcggcaaaatcccttataaatcaaaagaatagaccgagatagggttgagtgttgttccagtttggaacaagagtccactattaaagaacgtggactccaacgtcaaagggcgaaaaaccgtctatcagggcgatggcccactacgtgaaccatcaccctaatcaagttttttggggtcgaggtgccgtaaagcactaaatcggaaccctaaagggagcccccgatttagagcttgacggggaaagccggcgaacgtggcgagaaaggaagggaagaaagcgaaaggagcgggcgctagggcgctggcaagtgtagcggtcacgctgcgcgtaaccaccacacccgccgcgcttaatgcgccgctacagggcgcgtcgcgccattcgccattcaggctacgcaactgttgggaagggcgatcggtgcgggcctcttcgctattacgccagctggctgca

SEQ ID NO: 457 - DNA, 22 bp, Artificial Sequence
  Description of Artificial Sequence: Synthetic primer
gagaggttatgtggctttacca

SEQ ID NO: 458 - DNA, 20 bp, Artificial Sequence
  Description of Artificial Sequence: Synthetic primer
ctgcgtagtgccaaaacaaa

SEQ ID NO: 459 - DNA, 3252 bp, Artificial Sequence
  Description of Artificial Sequence: Synthetic polynucleotide
atgaaaaggaactacattctggggctggacatcgggattacaagcgtggggtatgggattattgactatgaaacaagggacgtgatcgacgcaggcgtcagactgttcaaggaggccaacgtggaaaacaatgagggacggagaagcaagaggggagccaggcgcctgaaacgacggagaaggcacagaatccagagggtgaagaaactgctgttcgattacaacctgctgaccgaccattctgagctgagtggaattaatccttatgaagccagggtgaaaggcctgagtcagaagctgtcagaggaagagttttccgcagctctgctgcacctggctaagcgccgaggagtgcataacgtcaatgaggtggaagaggacaccggcaacgagctgtctacaaaggaacagatctcacgcaatagcaaagctctggaagagaagtatgtcgcagagctgcagctggaacggctgaagaaagatggcgaggtgagagggtcaattaataggttcaagacaagcgactacgtcaaagaagccaagcagctgctgaaagtgcagaaggcttaccaccagctggatcagagcttcatcgatacttatatcgacctgctggagactcggagaacctactatgagggaccaggagaagggagccccttcggatggaaagacatcaaggaatggtacgagatgctgatgggacattgcacctattttccagaagagctgagaagcgtcaagtacgcttataacgcagatctgtacaacgccctgaatgacctgaacaacctggtcatcaccagggatgaaaacgagaaactggaatactatgagaagttccagatcatcgaaaacgtgtttaagcagaagaaaaagcctacactgaaacagattgctaaggagatcctggtcaacgaagaggacatcaagggctaccgggtgacaagcactggaaaaccagagttcaccaatctgaaagtgtatcacgatattaaggacatcacagcacggaaagaaatcattgagaacgccgaactgctggatcagattgctaagatcctgactatctaccagagctccgaggacatccaggaagagctgactaacctgaacagcgagctgacccaggaagagatcgaacagattagtaatctgaaggggtacaccggaacacacaacctgtccctgaaagctatcaatctgattctggatgagctgtggcatacaaacgacaatcagattgcaatctttaaccggctgaagctggtcccaaaaaaggtggacctgagtcagcagaaagagatcccaaccacactggtggacgatttcattctgtcacccgtggtcaagcggagcttcatccagagcatcaaagtgatcaacgccatcatcaagaagtacggcctgcccaatgatatcattatcgagctggctagggagaagaacagcaaggacgcacagaagatgatcaatgagatgcagaaacgaaaccggcagaccaatgaacgcattgaagagattatccgaactaccgggaaagagaacgcaaagtacctgattgaaaaaatcaagctgcacgatatgcaggagggaaagtgtctgtattctctggaggccatccccctggaggacctgctgaacaatccattcaactacgaggtcgatcatattatccccagaagcgtgtccttcgacaattcctttaacaacaaggtgctggtcaagcaggaagagaactctaaaaagggcaataggactcctttccagtacctgtctagttcagattccaagatctcttacgaaacctttaaaaagcacattctgaatctggccaaaggaaagggccgcatcagcaagaccaaaaaggagtacctgctggaagagcgggacatcaacagattctccgtccagaaggattttattaaccggaatctggtggacacaagatacgctactcgcggcctgatgaatctgctgcgatcctatttccgggtgaacaatctggatgtgaaagtcaagtccatcaacggcgggttcacatcttttctgaggcgcaaatggaagtttaaaaaggagcgcaacaaagggtacaagcaccatgccgaagatgctctgattatcgcaaatgccgacttcatctttaaggagtggaaaaagctggacaaagccaagaaagtgatggagaaccagatgttcgaagagaagcaggccgaatctatgcccgaaatcgagacagaacaggagtacaaggagattttcatcactcctcaccagatcaagcatatcaaggatttcaaggactacaagtactctcaccgggtggataaaaagcccaacagagagctgatcaatgacaccctgtatagtacaagaaaagacgataaggggaataccctgattgtgaacaatctgaacggactgtacgacaaagataatgacaagctgaaaaagctgatcaacaaaagtcccgagaagctgctgatgtaccaccatgatcctcagacatatcagaaactgaagctgattatggagcagtacggcgacgagaagaacccactgtataagtactatgaagagactgggaactacctgaccaagtatagcaaaaaggataatggccccgtgatcaagaagatcaagtactatgggaacaagctgaatgcccatctggacatcacagacgattaccctaacagtcgcaacaaggtggtcaagctgtcactgaagccatacagattcgatgtctatctggacaacggcgtgtataaatttgtgactgtcaagaatctggatgtcatcaaaaaggagaactactatgaagtgaatagcaagtgctacgaagaggctaaaaagctgaaaaagattagcaaccaggcagagttcatcgcctccttttacaacaacgacctgattaagatcaatggcgaactgtatagggtcatcggggtgaacaatgatctgctgaaccgcattgaagtgaatatgattgacatcacttaccgagagtatctggaaaacatgaatgataagcgcccccctcgaattatcaaaacaattgcctctaagactcagagtatcaaaaagtactcaaccgacattctgggaaacctgtatgaggtgaagagcaaaaagcaccctcagattatcaaaaagggcagcggaggcaagcgtcctgctgctactaagaaagctggtcaagctaagaaaaagaaaggatcctacccatacgatgttccagattacgcttaa

SEQ ID NO: 460 - DNA, 83 bp, Artificial Sequence
  Description of Artificial Sequence: Synthetic oligonucleotide
gttttagtactctggaaacagaatctactaaaacaaggcaaaatgccgtgtttatctcgtcaacttgttggcgagattttttt

SEQ ID NO: 461 - DNA, 3333 bp, Artificial Sequence
  Description of Artificial Sequence: Synthetic polynucleotide
atggtgcctaagaagaagagaaaggtggctgccttcaaacctaattcaatcaactacatcctcggcctcgatatcggcatcgcatccgtcggctgggcgatggtagaaattgacgaagaagaaaaccccatccgcctgattgatttgggcgtgcgcgtatttgagcgtgccgaagtaccgaaaacaggcgactcccttgccatggcaaggcgtttggcgcgcagtgttcgccgcctgacccgccgtcgcgcccaccgcctgcttcggacccgccgcctattgaaacgcgaaggcgtattacaagccgccaattttgacgaaaacggcttgattaaatccttaccgaatacaccatggcaacttcgcgcagccgcattagaccgcaaactgacgcctttagagtggtcggcagtcttgttgcatttaatcaaacatcgcggctatttatcgcaacggaaaaacgagggcgaaactgccgataaggagcttggcgctttgcttaaaggcgtagccggcaatgcccatgccttacagacaggcgatttccgcacaccggccgaattggctttaaataaatttgagaaagaaagcggccatatccgcaatcagcgcagcgattattcgcatacgttcagccgcaaagatttacaggcggagctgattttgctgtttgaaaaacaaaaagaatttggcaatccgcatgtttcaggcggccttaaagaaggtattgaaaccctactgatgacgcaacgccctgccctgtccggcgatgccgttcaaaaaatgttggggcattgcaccttcgaaccggcagagccgaaagccgctaaaaacacctacacagccgaacgtttcatctggctgaccaagctgaacaacctgcgtattttagagcaaggcagcgagcggccattgaccgataccgaacgcgccacgcttatggacgagccatacagaaaatccaaactgacttacgcacaagcccgtaagctgctgggtttagaagataccgcctttttcaaaggcttgcgctatggtaaagacaatgccgaagcctcaacattgatggaaatgaaggcctaccatgccatcagccgtgcactggaaaaagaaggattgaaagacaaaaaatccccattaaacctttctcccgaattacaagacgaaatcggcacggcattctccctgttcaaaaccgatgaagacattacaggccgtctgaaagaccgtatacagcccgaaatcttagaagcgctgttgaaacacatcagcttcgataagttcgtccaaatttccttgaaagcattgcgccgaattgtgcctctaatggaacaaggcaaacgttacgatgaagcctgcgccgaaatctacggagaccattacggcaagaagaatacggaagaaaagatttatctgccgccgattcccgccgacgaaatccgcaaccccgtcgtcttgcgcgccttatctcaagcacgtaaggtcattaacggcgtggtacgccgttacggctccccagctcgtatccatattgaaactgcaagggaagtaggtaaatcgtttaaagaccgcaaagaaattgagaaacgccaagaagaaaaccgcaaagaccgggaaaaagccgccgccaaattccgagagtatttccccaattttgtcggagaacccaaatccaaagatattctgaaactgcgcctgtacgagcaacaacacggcaaatgcctgtattcgggcaaagaaatcaacttaggccgtctgaacgaaaaaggctatgtcgaaatcgaccatgccctgccgttctcgcgcacatgggacgacagtttcaacaataaagtactggtattgggcagcgaaaaccaaaacaaaggcaatcaaaccccttacgaatacttcaacggcaaagacaacagccgcgaatggcaggaatttaaagcgcgtgtcgaaaccagccgtttcccgcgcagtaaaaaacaacggattctgctgcaaaaattcgatgaagacggctttaaagaacgcaatctgaacgacacgcgctacgtcaaccgtttcctgtgtcaatttgttgccgaccgtatgcggctgacaggtaaaggcaagaaacgtgtctttgcatccaacggacaaattaccaatctgttgcgcggcttttggggattgcgcaaagtgcgtgcggaaaacgaccgccatcacgccttggacgccgtcgtcgttgcctgctcgaccgttgccatgcagcagaaaattacccgttttgtacgctataaagagatgaacgcgtttgacggtaaaaccatagacaaagaaacaggagaagtgctgcatcaaaaaacacacttcccacaaccttgggaatttttcgcacaagaagtcatgattcgcgtcttcggcaaaccggacggcaaacccgaattcgaagaagccgataccctagaaaaactgcgcacgttgcttgccgaaaaattatcatctcgccccgaagccgtacacgaatacgttacgccactgtttgtttcacgcgcgcccaatcggaagatgagcgggcaagggcatatggagaccgtcaaatccgccaaacgactggacgaaggcgtcagcgtgttgcgcgtaccgctgacacagttaaaactgaaagacttggaaaaaatggtcaatcgggagcgcgaacctaagctatacgaagcactgaaagcacggctggaagcacataaagacgatcctgccaaagcctttgccgagccgttttacaaatacgataaagcaggcaaccgcacccaacaggtaaaagccgtacgcgtagagcaagtacagaaaaccggcgtatgggtgcgcaaccataacggtattgccgacaacgcaaccatggtgcgcgtagatgtgtttgagaaaggcgacaagtattatctggtaccgatttacagttggcaggtagcgaaagggattttgccggatagggctgttgtacaaggaaaagatgaagaagattggcaacttattgatgatagtttcaactttaaattctcattacaccctaatgatttagtcgaggttataacaaaaaaagctagaatgtttggttactttgccagctgccatcgaggcacaggtaatatcaatatacgcattcatgatcttgatcataaaattggcaaaaatggaatactggaaggtatcggcgtcaaaaccgccctttcattccaaaaataccaaattgacgaactgggcaaagaaatcagaccatgccgtctgaaaaaacgcccgcctgtccgttacccatacgatgttccagattacgctgcagctccagcagcgaagaaaaagaagctggattaa

SEQ ID NO: 462 - DNA, 120 bp, Artificial Sequence
  Description of Artificial Sequence: Synthetic polynucleotide
gttgtagctccctttctcatttcggaaacgaaatgagaaccgttgctacaataaggccgtctgaaaagatgtgccgcaacgctctgccccttaaagcttctgctttaaggggcttttttt

SEQ ID NO: 463 - DNA, 144 bp, Artificial Sequence
  Description of Artificial Sequence: Synthetic polynucleotide
gttgtagctccctttctcatttcgcagtgctacaatgaaaattgtcgcactgcgaaatgagaaccgttgctacaataaggccgtctgaaaagatgtgccgcaacgctctgccccttaaagcttctgctttaaggggcttttttt

SEQ ID NO: 464 - DNA, 24 bp, Artificial Sequence
  Description of Artificial Sequence: Synthetic primer
tcgggtttattacagggacagcag

SEQ ID NO: 465 - DNA, 24 bp, Artificial Sequence
  Description of Artificial Sequence: Synthetic primer
tctaaggccgagtcttatgagcag

SEQ ID NO: 466 - DNA, 4564 bp, Artificial Sequence
  Description of Artificial Sequence: Synthetic polynucleotide
atggactacaaagaccatgacggtgattataaagatcatgacatcgattacaaggatgacgatgacaagatggcccccaagaagaagaggaaggtgggccgcggaatggacaagaagtactccattgggctcgccatcggcacaaacagcgtcggctgggccgtcattacggacgagtacaaggtgccgagcaaaaaattcaaagttctgggcaataccgatcgccacagcataaagaagaacctcattggcgccctcctgttcgactccggggaaaccgccgaagccacgcggctcaaaagaacagcacggcgcagatatacccgcagaaagaatcggatctgctacctgcaggagatctttagtaatgagatggctaaggtggatgactctttcttccataggctggaggagtcctttttggtggaggaggataaaaagcacgagcgccacccaatctttggcaatatcgtggacgaggtggcgtaccatgaaaagtacccaaccatatatcatctgaggaagaagcttgtagacagtactgataaggctgacttgcggttgatctatctcgcgctggcgcatatgatcaaatttcggggacacttcctcatcgagggggacctgaacccagacaacagcgatgtcgacaaactctttatccaactggttcagacttacaatcagcttttcgaagagaacccgatcaacgcatccggagttgacgccaaagcaatcctgagcgctaggctgtccaaatcccggcggctcgaaaacctcatcgcacagctccctggggagaagaagaacggcctgtttggtaatcttatcgccctgtcactcgggctgacccccaactttaaatctaacttcgacctggccgaagatgccaagcttcaactgagcaaagacacctacgatgatgatctcgacaatctgctggcccagatcggcgaccagtacgcagacctttttttggcggcaaagaacctgtcagacgccattctgctgagtgatattctgcgagtgaacacggagatcaccaaagctccgctgagcgctagtatgatcaagcgctatgatgagcaccaccaagacttgactttgctgaaggcccttgtcagacagcaactgcctgagaagtacaaggaaattttcttcgatcagtctaaaaatggctacgccggatacattgacggcggagcaagccaggaggaattttacaaatttattaagcccatcttggaaaaaatggacggcaccgaggagctgctggtaaagcttaacagagaagatctgttgcgcaaacagcgcactttcgacaatggaagcatcccccaccagattcacctgggcgaactgcacgctatcctcaggcggcaagaggatttctacccctttttgaaagataacagggaaaagattgagaaaatcctcacatttcggataccctactatgtaggccccctcgcccggggaaattccagattcgcgtggatgactcgcaaatcagaagagaccatcactccctggaacttcgaggaagtcgtggataagggggcctctgcccagtccttcatcgaaaggatgactaactttgataaaaatctgcctaacgaaaaggtgcttcctaaacactctctgctgtacgagtacttcacagtttataacgagctcaccaaggtcaaatacgtcacagaagggatgagaaagccagcattcctgtctggagagcagaagaaagctatcgtggacctcctcttcaagacgaaccggaaagttaccgtgaaacagctcaaagaagactatttcaaaaagattgaatgtttcgactctgttgaaatcagcggagtggaggatcgcttcaacgcatccctgggaacgtatcacgatctcctgaaaatcattaaagacaaggacttcctggacaatgaggagaacgaggacattcttgaggacattgtcctcacccttacgttgtttgaagatagggagatgattgaagaacgcttgaaaacttacgctcatctcttcgacgacaaagtcatgaaacagctcaagaggcgccgatatacaggatgggggcggctgtcaagaaaactgatcaatgggatccgagacaagcagagtggaaagacaatcctggattttcttaagtccgatggatttgccaaccggaacttcatgcagttgatccatgatgactctctcacctttaaggaggacatccagaaagcacaagtttctggccagggggacagtcttcacgagcacatcgctaatcttgcaggtagcccagctatcaaaaagggaatactgcagaccgttaaggtcgtggatgaactcgtcaaagtaatgggaaggcataagcccgagaatatcgttatcgagatggcccgagagaaccaaactacccagaagggacagaagaacagtagggaaaggatgaagaggattgaagagggtataaaagaactggggtcccaaatccttaaggaacacccagttgaaaacacccagcttcagaatgagaagctctacctgtactacctgcagaacggcagggacatgtacgtggatcaggaactggacatcaatcggctctccgactacgacgtggatgccatcgtgccccagtcttttctcaaagatgattctattgataataaagtgttgacaagatccgataaaaatagagggaagagtgataacgtcccctcagaagaagttgtcaagaaaatgaaaaattattggcggcagctgctgaacgccaaactgatcacacaacggaagttcgataatctgactaaggctgaacgaggtggcctgtctgagttggataaagccggcttcatcaaaaggcagcttgttgagacacgccagatcaccaagcacgtggcccaaattctcgattcacgcatgaacaccaagtacgatgaaaatgacaaactgattcgagaggtgaaagttattactctgaagtctaagctggtctcagatttcagaaaggactttcagttttataaggtgagagagatcaacaattaccaccatgcgcatgatgcctacctgaatgcagtggtaggcactgcacttatcaaaaaatatcccaagcttgaatctgaatttgtttacggagactataaagtgtacgatgttaggaaaatgatcgcaaagtctgagcaggaaataggcaaggccaccgctaagtacttcttttacagcaatattatgaattttttcaagaccgagattacactggccaatggagagattcggaagcgaccacttatcgaaacaaacggagaaacaggagaaatcgtgtgggacaagggtagggatttcgcgacagtccggaaggtcctgtccatgccgcaggtgaacatcgttaaaaagaccgaagtacagaccggaggcttctccaaggaaagtatcctcccgaaaaggaacagcgacaagctgatcgcacgcaaaaaagattgggaccccaagaaatacggcggattcgattctcctacagtcgcttacagtgtactggttgtggccaaagtggagaaagggaagtctaaaaaactcaaaagcgtcaaggaactgctgggcatcacaatcatggagcgatcaagcttcgaaaaaaaccccatcgactttctcgaggcgaaaggatataaagaggtcaaaaaagacctcatcattaagcttcccaagtactctctctttgagcttgaaaacggccggaaacgaatgctcgctagtgcgggcgagctgcagaaaggtaacgagctggcactgccctctaaatacgttaatttcttgtatctggccagccactatgaaaagctcaaagggtctcccgaagataatgagcagaagcagctgttcgtggaacaacacaaacactaccttgatgagatcatcgagcaaataagcgaattctccaaaagagtgatcctcgccgacgctaacctcgataaggtgctttctgcttacaataagcacagggataagcccatcagggagcaggcagaaaacattatccacttgtttactctgaccaacttgggcgcgcctgcagccttcaagtacttcgacaccaccatagacagaaagcggtacacctctacaaaggaggtcctggacgccacactgattcatcagtcaattacggggctctatgaaacaagaatcgacctctctcagctcggtggagacagcagggctgaccccaagaagaagaggaaggtggctagcgatgctaagtcactgactgcctggtcccggacactggtgaccttcaaggatgtgtttgtggacttcaccagggaggagtggaagctgctggacactgctcagcagatcctgtacagaaatgtgatgctggagaactataagaacctggtttccttgggttatcagcttactaagccagatgtgatcctccggttggagaagggagaagagccctggctggtggagagagaaattcaccaagagacccatcctgattcagagactgcatttgaaatcaaatcatcagttccgaaaaagaaacgcaaagttgctagcg

SEQ ID NO: 467 - DNA, 388 bp, Artificial Sequence
  Description of Artificial Sequence: Synthetic polynucleotide
taagcttcagtttttccttagttcctgttacatttctgtgtgtctccattagtgacctcccatagtccaagcatgagcagttctggccaggcccctgtcggggtcagtgccccacccccgccttctggttctgtgtaaccttctaagcaaaccttctggctcaagcacagcaatgctgagtcatgatgagtcatgctgaggcttagggtgtgtgcccagatgttctcagcctagagtgatgactcctatctgggtccccagcaggatgcttacagggcagatggcaaaaaaaaggagaagctgaccacctgactaaaactccacctcaaacggcatcataaagaaaatggatgcctgagacagaatgtgacatattctagaatatatt

SEQ ID NO: 468 - DNA, 19 bp, Artificial Sequence
  Description of Artificial Sequence: Synthetic oligonucleotide
cagccgctcgctgcagcag

SEQ ID NO: 469 - DNA, 19 bp, Artificial Sequence
  Description of Artificial Sequence: Synthetic oligonucleotide
ctgctgcagcgagcggctg

SEQ ID NO: 470 - DNA, 19 bp, Artificial Sequence
  Description of Artificial Sequence: Synthetic oligonucleotide
gctgggtgtcccattgaaa

SEQ ID NO: 471 - DNA, 19 bp, Artificial Sequence
  Description of Artificial Sequence: Synthetic oligonucleotide
tttcaatgggacacccagc

SEQ ID NO: 472 - DNA, 19 bp, Artificial Sequence
  Description of Artificial Sequence: Synthetic oligonucleotide
gtttattcagccgggagtc

SEQ ID NO: 473 - DNA, 19 bp, Artificial Sequence
  Description of Artificial Sequence: Synthetic oligonucleotide
gactcccggctgaataaac

SEQ ID NO: 474 - DNA, 19 bp, Artificial Sequence
  Description of Artificial Sequence: Synthetic oligonucleotide
tggagagtttgcaaggagc

SEQ ID NO: 475 - DNA, 19 bp, Artificial Sequence
  Description of Artificial Sequence: Synthetic oligonucleotide
gctccttgcaaactctcca

SEQ ID NO: 476 - DNA, 19 bp, Artificial Sequence
  Description of Artificial Sequence: Synthetic oligonucleotide
ccctccagactttccacct

SEQ ID NO: 477 - DNA, 19 bp, Artificial Sequence
  Description of Artificial Sequence: Synthetic oligonucleotide
aggtggaaagtctggaggg

SEQ ID NO: 478 - DNA, 19 bp, Artificial Sequence
  Description of Artificial Sequence: Synthetic oligonucleotide
aattttcttccaagttctc

SEQ ID NO: 479 - DNA, 19 bp, Artificial Sequence
  Description of Artificial Sequence: Synthetic oligonucleotide
gagaacttggaagaaaatt

SEQ ID NO: 480 - DNA, 19 bp, Artificial Sequence
  Description of Artificial Sequence: Synthetic oligonucleotide
ctgcggagagaagaaaggg

SEQ ID NO: 481 - DNA, 19 bp, Artificial Sequence
  Description of Artificial Sequence: Synthetic oligonucleotide
ccctttcttctctccgcag

SEQ ID NO: 482 - DNA, 19 bp, Artificial Sequence
  Description of Artificial Sequence: Synthetic oligonucleotide
agagccaccccctggctcc

SEQ ID NO: 483 - DNA, 19 bp, Artificial Sequence
  Description of Artificial Sequence: Synthetic oligonucleotide
ggagccagggggtggctct

SEQ ID NO: 484 - DNA, 19 bp, Artificial Sequence
  Description of Artificial Sequence: Synthetic oligonucleotide
cgaagccaaccgcggcggg

SEQ ID NO: 485 - DNA, 19 bp, Artificial Sequence
  Description of Artificial Sequence: Synthetic oligonucleotide
cccgccgcggttggcttcg

SEQ ID NO: 486 - DNA, 19 bp, Artificial Sequence
  Description of Artificial Sequence: Synthetic oligonucleotide
agagggaagacgatcgccc

SEQ ID NO: 487 - DNA, 19 bp, Artificial Sequence
  Description of Artificial Sequence: Synthetic oligonucleotide
gggcgatcgtcttccctct

SEQ ID NO: 488 - DNA, 19 bp, Artificial Sequence
  Description of Artificial Sequence: Synthetic oligonucleotide
cccctttaactttcctccg

SEQ ID NO: 489 - DNA, 19 bp, Artificial Sequence
  Description of Artificial Sequence: Synthetic oligonucleotide
cggaggaaagttaaagggg

SEQ ID NO: 490 - DNA, 19 bp, Artificial Sequence
  Description of Artificial Sequence: Synthetic oligonucleotide
gcagccccgcttccttcaa

SEQ ID NO: 491 - DNA, 19 bp, Artificial Sequence
  Description of Artificial Sequence: Synthetic oligonucleotide
ttgaaggaagcggggctgc

SEQ ID NO: 492 - DNA, 24 bp, Artificial Sequence
  Description of Artificial Sequence: Synthetic oligonucleotide
caccgcagccgctcgctgcagcag

SEQ ID NO: 493 - DNA, 24 bp, Artificial Sequence
  Description of Artificial Sequence: Synthetic oligonucleotide
aaacctgctgcagcgagcggctgc

SEQ ID NO: 494 - DNA, 24 bp, Artificial Sequence
  Description of Artificial Sequence: Synthetic oligonucleotide
caccggctgggtgtcccattgaaa

SEQ ID NO: 495 - DNA, 24 bp, Artificial Sequence
  Description of Artificial Sequence: Synthetic oligonucleotide
aaactttcaatgggacacccagcc

SEQ ID NO: 496 - DNA, 24 bp, Artificial Sequence
  Description of Artificial Sequence: Synthetic oligonucleotide
caccggtttattcagccgggagtc

SEQ ID NO: 497 - DNA, 24 bp, Artificial Sequence
  Description of Artificial Sequence: Synthetic oligonucleotide
aaacgactcccggctgaataaacc

SEQ ID NO: 498 - DNA, 24 bp, Artificial Sequence
  Description of Artificial Sequence: Synthetic oligonucleotide
caccgtggagagtttgcaaggagc

SEQ ID NO: 499 - DNA, 24 bp, Artificial Sequence
  Description of Artificial Sequence: Synthetic oligonucleotide
aaacgctccttgcaaactctccac

SEQ ID NO: 500 - DNA, 24 bp, Artificial Sequence
  Description of Artificial Sequence: Synthetic oligonucleotide
caccgccctccagactttccacct

SEQ ID NO: 501 - DNA, 24 bp, Artificial Sequence
  Description of Artificial Sequence: Synthetic oligonucleotide
aaacaggtggaaagtctggagggc

SEQ ID NO: 502 - DNA, 24 bp, Artificial Sequence
  Description of Artificial Sequence: Synthetic oligonucleotide
caccgaattttcttccaagttctc

SEQ ID NO: 503 - DNA, 24 bp, Artificial Sequence
  Description of Artificial Sequence: Synthetic oligonucleotide
aaacgagaacttggaagaaaattc

SEQ ID NO: 504 - DNA, 24 bp, Artificial Sequence
  Description of Artificial Sequence: Synthetic oligonucleotide
caccgctgcggagagaagaaaggg

SEQ ID NO: 505 - DNA, 24 bp, Artificial Sequence
  Description of Artificial Sequence: Synthetic oligonucleotide
aaacccctttcttctctccgcagc

SEQ ID NO: 506 - DNA, 24 bp, Artificial Sequence
  Description of Artificial Sequence: Synthetic oligonucleotide
caccgagagccaccccctggctcc

SEQ ID NO: 507 - DNA, 24 bp, Artificial Sequence
  Description of Artificial Sequence: Synthetic oligonucleotide
aaacggagccagggggtggctctc

SEQ ID NO: 508 - DNA, 24 bp, Artificial Sequence
  Description of Artificial Sequence: Synthetic oligonucleotide
caccgcgaagccaaccgcggcggg

SEQ ID NO: 509 - DNA, 24 bp, Artificial Sequence
  Description of Artificial Sequence: Synthetic oligonucleotide
aaaccccgccgcggttggcttcgc

SEQ ID NO: 510 - DNA, 24 bp, Artificial Sequence
  Description of Artificial Sequence: Synthetic oligonucleotide
caccgagagggaagacgatcgccc

SEQ ID NO: 511 - DNA, 24 bp, Artificial Sequence
  Description of Artificial Sequence: Synthetic oligonucleotide
aaacgggcgatcgtcttccctctc

SEQ ID NO: 512 - DNA, 24 bp, Artificial Sequence
  Description of Artificial Sequence: Synthetic oligonucleotide
caccgcccctttaactttcctccg

SEQ ID NO: 513 - DNA, 24 bp, Artificial Sequence
  Description of Artificial Sequence: Synthetic oligonucleotide
aaaccggaggaaagttaaaggggc

SEQ ID NO: 514 - DNA, 24 bp, Artificial Sequence
  Description of Artificial Sequence: Synthetic oligonucleotide
caccggcagccccgcttccttcaa

SEQ ID NO: 515 - DNA, 24 bp, Artificial Sequence
  Description of Artificial Sequence: Synthetic oligonucleotide
aaacttgaaggaagcggggctgcc

SEQ ID NO: 516 - DNA, 19 bp, Artificial Sequence
  Description of Artificial Sequence: Synthetic oligonucleotide
cgagagcgagaggagggag

SEQ ID NO: 517 - DNA, 19 bp, Artificial Sequence
  Description of Artificial Sequence: Synthetic oligonucleotide
ctccctcctctcgctctcg

SEQ ID NO: 518 - DNA, 19 bp, Artificial Sequence
  Description of Artificial Sequence: Synthetic oligonucleotide
gagagagcttgagagcgcg

SEQ ID NO: 519 - DNA, 19 bp, Artificial Sequence
  Description of Artificial Sequence: Synthetic oligonucleotide
cgcgctctcaagctctctc

SEQ ID NO: 520 - DNA, 19 bp, Artificial Sequence
  Description of Artificial Sequence: Synthetic oligonucleotide
ggtggagggggcggggccc

SEQ ID NO: 521 - DNA, 19 bp, Artificial Sequence
  Description of Artificial Sequence: Synthetic oligonucleotide
gggccccgccccctccacc

SEQ ID NO: 522 - DNA, 19 bp, Artificial Sequence
  Description of Artificial Sequence: Synthetic oligonucleotide
ggtatccacgtaaatcaaa

SEQ ID NO: 523 - DNA, 19 bp, Artificial Sequence
  Description of Artificial Sequence: Synthetic oligonucleotide
tttgatttacgtggatacc

SEQ ID NO: 524 - DNA, 19 bp, Artificial Sequence
  Description of Artificial Sequence: Synthetic oligonucleotide
ccaatcactggctccggtc

SEQ ID NO: 525 - DNA, 19 bp, Artificial Sequence
  Description of Artificial Sequence: Synthetic oligonucleotide
gaccggagccagtgattgg

SEQ ID NO: 526 - DNA, 19 bp, Artificial Sequence
  Description of Artificial Sequence: Synthetic oligonucleotide
ggcgcccgagggaagaaga

SEQ ID NO: 527 - DNA, 19 bp, Artificial Sequence
  Description of Artificial Sequence: Synthetic oligonucleotide
tcttcttccctcgggcgcc

SEQ ID NO: 528 - DNA, 19 bp, Artificial Sequence
  Description of Artificial Sequence: Synthetic oligonucleotide
gggtgggggtaccagagga

SEQ ID NO: 529 - DNA, 19 bp, Artificial Sequence
  Description of Artificial Sequence: Synthetic oligonucleotide
tcctctggtacccccaccc

SEQ ID NO: 530 - DNA, 19 bp, Artificial Sequence
  Description of Artificial Sequence: Synthetic oligonucleotide
ccggggacagaagagaggg

SEQ ID NO: 531 - DNA, 19 bp, Artificial Sequence
  Description of Artificial Sequence: Synthetic oligonucleotide
ccctctcttctgtccccgg

SEQ ID NO: 532 - DNA, 19 bp, Artificial Sequence
  Description of Artificial Sequence: Synthetic oligonucleotide
gagagagagtgggagaagc

SEQ ID NO: 533 - DNA, 19 bp, Artificial Sequence
  Description of Artificial Sequence: Synthetic oligonucleotide
gcttctcccactctctctc

SEQ ID NO: 534 - DNA, 19 bp, Artificial Sequence
  Description of Artificial Sequence: Synthetic oligonucleotide
aaagtaactgtcaaatgcg

SEQ ID NO: 535 - DNA, 19 bp, Artificial Sequence
  Description of Artificial Sequence: Synthetic oligonucleotide
cgcatttgacagttacttt

SEQ ID NO: 536 - DNA, 19 bp, Artificial Sequence
  Description of Artificial Sequence: Synthetic oligonucleotide
ttaaccagagcgcccagtc

SEQ ID NO: 537 - DNA, 19 bp, Artificial Sequence
  Description of Artificial Sequence: Synthetic oligonucleotide
gactgggcgctctggttaa

SEQ ID NO: 538 - DNA, 19 bp, Artificial Sequence
  Description of Artificial Sequence: Synthetic oligonucleotide
cgtcggagctgcccgctag

SEQ ID NO: 539 - DNA, 19 bp, Artificial Sequence
  Description of Artificial Sequence: Synthetic oligonucleotide
ctagcgggcagctccgacg

SEQ ID NO: 540 - DNA, 24 bp, Artificial Sequence
  Description of Artificial Sequence: Synthetic oligonucleotide
caccgcgagagcgagaggagggag

SEQ ID NO: 541 - DNA, 24 bp, Artificial Sequence
  Description of Artificial Sequence: Synthetic oligonucleotide
aaacctccctcctctcgctctcgc

SEQ ID NO: 542 - DNA, 24 bp, Artificial Sequence
  Description of Artificial Sequence: Synthetic oligonucleotide
caccggagagagcttgagagcgcg

SEQ ID NO: 543 - DNA, 24 bp, Artificial Sequence
  Description of Artificial Sequence: Synthetic oligonucleotide
aaaccgcgctctcaagctctctcc

SEQ ID NO: 544 - DNA, 24 bp, Artificial Sequence
  Description of Artificial Sequence: Synthetic oligonucleotide
caccgggtggagggggcggggccc

SEQ ID NO: 545 - DNA, 24 bp, Artificial Sequence
  Description of Artificial Sequence: Synthetic oligonucleotide
aaacgggccccgccccctccaccc

SEQ ID NO: 546 - DNA, 24 bp, Artificial Sequence
  Description of Artificial Sequence: Synthetic oligonucleotide
caccgggtatccacgtaaatcaaa

SEQ ID NO: 547 - DNA, 24 bp, Artificial Sequence
  Description of Artificial Sequence: Synthetic oligonucleotide
aaactttgatttacgtggataccc

SEQ ID NO: 548 - DNA, 24 bp, Artificial Sequence
  Description of Artificial Sequence: Synthetic oligonucleotide
caccgccaatcactggctccggtc

SEQ ID NO: 549 - DNA, 24 bp, Artificial Sequence
  Description of Artificial Sequence: Synthetic oligonucleotide
aaacgaccggagccagtgattggc

SEQ ID NO: 550 - DNA, 24 bp, Artificial Sequence
  Description of Artificial Sequence: Synthetic oligonucleotide
caccgggcgcccgagggaagaaga

SEQ ID NO: 551 - DNA, 24 bp, Artificial Sequence
  Description of Artificial Sequence: Synthetic oligonucleotide
aaactcttcttccctcgggcgccc

SEQ ID NO: 552 - DNA, 24 bp, Artificial Sequence
  Description of Artificial Sequence: Synthetic oligonucleotide
caccggggtgggggtaccagagga

SEQ ID NO: 553 - DNA, 24 bp, Artificial Sequence
  Description of Artificial Sequence: Synthetic oligonucleotide
aaactcctctggtacccccacccc

SEQ ID NO: 554 - DNA, 24 bp, Artificial Sequence
  Description of Artificial Sequence: Synthetic oligonucleotide
caccgccggggacagaagagaggg

SEQ ID NO: 555 - DNA, 24 bp, Artificial Sequence
  Description of Artificial Sequence: Synthetic oligonucleotide
aaacccctctcttctgtccccggc

SEQ ID NO: 556 - DNA, 24 bp, Artificial Sequence
  Description of Artificial Sequence: Synthetic oligonucleotide
caccggagagagagtgggagaagc

SEQ ID NO: 557 - DNA, 24 bp, Artificial Sequence
  Description of Artificial Sequence: Synthetic oligonucleotide
aaacgcttctcccactctctctcc

SEQ ID NO: 558 - DNA, 24 bp, Artificial Sequence
  Description of Artificial Sequence: Synthetic oligonucleotide
caccgaaagtaactgtcaaatgcg

SEQ ID NO: 559 - DNA, 24 bp, Artificial Sequence
  Description of Artificial Sequence: Synthetic oligonucleotide
aaaccgcatttgacagttactttc

SEQ ID NO: 560 - DNA, 24 bp, Artificial Sequence
  Description of Artificial Sequence: Synthetic oligonucleotide
caccgttaaccagagcgcccagtc

SEQ ID NO: 561 - DNA, 24 bp, Artificial Sequence
  Description of Artificial Sequence: Synthetic oligonucleotide
aaacgactgggcgctctggttaac

SEQ ID NO: 562 - DNA, 24 bp, Artificial Sequence
  Description of Artificial Sequence: Synthetic oligonucleotide
caccgcgtcggagctgcccgctag

SEQ ID NO: 563 - DNA, 24 bp, Artificial Sequence
  Description of Artificial Sequence: Synthetic oligonucleotide
aaacctagcgggcagctccgacgc

SEQ ID NO: 564 - DNA, 20 bp, Artificial Sequence
  Description of Artificial Sequence: Synthetic oligonucleotide
gagacacacagaaatgtaac

SEQ ID NO: 565 - DNA, 20 bp, Artificial Sequence
  Description of Artificial Sequence: Synthetic oligonucleotide
ggtggggcactgaccccgac

SEQ ID NO: 566 - DNA, 20 bp, Artificial Sequence
  Description of Artificial Sequence: Synthetic oligonucleotide
ctagagtgatgactcctatc

SEQ ID NO: 567 - DNA, 20 bp, Artificial Sequence
  Description of Artificial Sequence: Synthetic oligonucleotide
gactaaaactccacctcaaa

SEQ ID NO: 568 - DNA, 20 bp, Artificial Sequence
  Description of Artificial Sequence: Synthetic oligonucleotide
aatatgtcacattctgtctc

SEQ ID NO: 569 - DNA, 20 bp, Artificial Sequence
  Description of Artificial Sequence: Synthetic oligonucleotide
ggactatgggaggtcactaa

SEQ ID NO: 570 - DNA, 20 bp, Artificial Sequence
  Description of Artificial Sequence: Synthetic oligonucleotide
gctcatgcttggactatggg

SEQ ID NO: 571 - DNA, 20 bp, Artificial Sequence
  Description of Artificial Sequence: Synthetic oligonucleotide
gttctggccaggcccctgtc

SEQ ID NO: 572 - DNA, 20 bp, Artificial Sequence
  Description of Artificial Sequence: Synthetic oligonucleotide
agtgccccacccccgccttc

SEQ ID NO: 573 - DNA, 20 bp, Artificial Sequence
  Description of Artificial Sequence: Synthetic oligonucleotide
gtggggcactgaccccgaca

SEQ ID NO: 574 - DNA, 20 bp, Artificial Sequence
  Description of Artificial Sequence: Synthetic oligonucleotide
aaccttctaagcaaaccttc

SEQ ID NO: 575 - DNA, 20 bp, Artificial Sequence
  Description of Artificial Sequence: Synthetic oligonucleotide
gttacacagaaccagaaggc

SEQ ID NO: 576 - DNA, 20 bp, Artificial Sequence
  Description of Artificial Sequence: Synthetic oligonucleotide
gaaggttacacagaaccaga

SEQ ID NO: 577 - DNA, 20 bp, Artificial Sequence
  Description of Artificial Sequence: Synthetic oligonucleotide
agtcatgatgagtcatgctg

SEQ ID NO: 578 - DNA, 20 bp, Artificial Sequence
  Description of Artificial Sequence: Synthetic oligonucleotide
gatgagtcatgctgaggctt

SEQ ID NO: 579 - DNA, 20 bp, Artificial Sequence
  Description of Artificial Sequence: Synthetic oligonucleotide
actctaggctgagaacatct

SEQ ID NO: 580 - DNA, 20 bp, Artificial Sequence
  Description of Artificial Sequence: Synthetic oligonucleotide
gtccccagcaggatgcttac

SEQ ID NO: 581 - DNA, 20 bp, Artificial Sequence
  Description of Artificial Sequence: Synthetic oligonucleotide
gccctgtaagcatcctgctg

SEQ ID NO: 582 - DNA, 20 bp, Artificial Sequence
  Description of Artificial Sequence: Synthetic oligonucleotide
cagggcagatggcaaaaaaa

SEQ ID NO: 583 - DNA, 20 bp, Artificial Sequence
  Description of Artificial Sequence: Synthetic oligonucleotide
gaggtggagttttagtcagg

SEQ ID NO: 584 - DNA, 20 bp, Artificial Sequence
  Description of Artificial Sequence: Synthetic oligonucleotide
aaacggcatcataaagaaaa

SEQ ID NO: 585 - DNA, 105 bp, Artificial Sequence
  Description of Artificial Sequence: Synthetic polynucleotide
gagacacacagaaatgtaacgttttagagctagaaatagcaagttaaaataaggctagtccgttatcaacttgaaaaagtggcaccgagtcggtgctttttttcc

SEQ ID NO: 586 - DNA, 105 bp, Artificial Sequence
  Description of Artificial Sequence: Synthetic polynucleotide
ggtggggcactgaccccgacgttttagagctagaaatagcaagttaaaataaggctagtccgttatcaacttgaaaaagtggcaccgagtcggtgctttttttcc

SEQ ID NO: 587 - DNA, 105 bp, Artificial Sequence
  Description of Artificial Sequence: Synthetic polynucleotide
ctagagtgatgactcctatcgttttagagctagaaatagcaagttaaaataaggctagtccgttatcaacttgaaaaagtggcaccgagtcggtgctttttttcc

SEQ ID NO: 588 - DNA, 105 bp, Artificial Sequence
  Description of Artificial Sequence: Synthetic polynucleotide
gactaaaactccacctcaaagttttagagctagaaatagcaagttaaaataaggctagtccgttatcaacttgaaaaagtggcaccgagtcggtgctttttttcc

SEQ ID NO: 589 - DNA, 105 bp, Artificial Sequence
  Description of Artificial Sequence: Synthetic polynucleotide
aatatgtcacattctgtctcgttttagagctagaaatagcaagttaaaataaggctagtccgttatcaacttgaaaaagtggcaccgagtcggtgctttttttcc

SEQ ID NO: 590 - DNA, 105 bp, Artificial Sequence
  Description of Artificial Sequence: Synthetic polynucleotide
ggactatgggaggtcactaagttttagagctagaaatagcaagttaaaataaggctagtccgttatcaacttgaaaaagtggcaccgagtcggtgctttttttcc

SEQ ID NO: 591 - DNA, 105 bp, Artificial Sequence
  Description of Artificial Sequence: Synthetic polynucleotide
gctcatgcttggactatggggttttagagctagaaatagcaagttaaaataaggctagtccgttatcaacttgaaaaagtggcaccgagtcggtgctttttttcc

SEQ ID NO: 592 - DNA, 105 bp, Artificial Sequence
  Description of Artificial Sequence: Synthetic polynucleotide
gttctggccaggcccctgtcgttttagagctagaaatagcaagttaaaataaggctagtccgttatcaacttgaaaaagtggcaccgagtcggtgctttttttcc

SEQ ID NO: 593 - DNA, 105 bp, Artificial Sequence
  Description of Artificial Sequence: Synthetic polynucleotide
agtgccccacccccgccttcgttttagagctagaaatagcaagttaaaataaggctagtccgttatcaacttgaaaaagtggcaccgagtcggtgctttttttcc

SEQ ID NO: 594 - DNA, 105 bp, Artificial Sequence
  Description of Artificial Sequence: Synthetic polynucleotide
gtggggcactgaccccgacagttttagagctagaaatagcaagttaaaataaggctagtccgttatcaacttgaaaaagtggcaccgagtcggtgctttttttcc

SEQ ID NO: 595 - DNA, 105 bp, Artificial Sequence
  Description of Artificial Sequence: Synthetic polynucleotide
aaccttctaagcaaaccttcgttttagagctagaaatagcaagttaaaataaggctagtccgttatcaacttgaaaaagtggcaccgagtcggtgctttttttcc

SEQ ID NO: 596 - DNA, 105 bp, Artificial Sequence
  Description of Artificial Sequence: Synthetic polynucleotide
gttacacagaaccagaaggcgttttagagctagaaatagcaagttaaaataaggctagtccgttatcaacttgaaaaagtggcaccgagtcggtgctttttttcc

SEQ ID NO: 597 - DNA, 105 bp, Artificial Sequence
  Description of Artificial Sequence: Synthetic polynucleotide
gaaggttacacagaaccagagttttagagctagaaatagcaagttaaaataaggctagtccgttatcaacttgaaaaagtggcaccgagtcggtgctttttttcc

SEQ ID NO: 598 - DNA, 105 bp, Artificial Sequence
  Description of Artificial Sequence: Synthetic polynucleotide
agtcatgatgagtcatgctggttttagagctagaaatagcaagttaaaataaggctagtccgttatcaacttgaaaaagtggcaccgagtcggtgctttttttcc

SEQ ID NO: 599 - DNA, 105 bp, Artificial Sequence
  Description of Artificial Sequence: Synthetic polynucleotide
gatgagtcatgctgaggcttgttttagagctagaaatagcaagttaaaataaggctagtccgttatcaacttgaaaaagtggcaccgagtcggtgctttttttcc

SEQ ID NO: 600 - DNA, 105 bp, Artificial Sequence
  Description of Artificial Sequence: Synthetic polynucleotide
actctaggctgagaacatctgttttagagctagaaatagcaagttaaaataaggctagtccgttatcaacttgaaaaagtggcaccgagtcggtgctttttttcc

SEQ ID NO: 601 - DNA, 105 bp, Artificial Sequence
  Description of Artificial Sequence: Synthetic polynucleotide
gtccccagcaggatgcttacgttttagagctagaaatagcaagttaaaataaggctagtccgttatcaacttgaaaaagtggcaccgagtcggtgctttttttcc

SEQ ID NO: 602 - DNA, 105 bp, Artificial Sequence
  Description of Artificial Sequence: Synthetic polynucleotide
gccctgtaagcatcctgctggttttagagctagaaatagcaagttaaaataaggctagtccgttatcaacttgaaaaagtggcaccgagtcggtgctttttttcc

SEQ ID NO: 603 - DNA, 105 bp, Artificial Sequence
  Description of Artificial Sequence: Synthetic polynucleotide
cagggcagatggcaaaaaaagttttagagctagaaatagcaagttaaaataaggctagtccgttatcaacttgaaaaagtggcaccgagtcggtgctttttttcc

SEQ ID NO: 604 - DNA, 105 bp, Artificial Sequence
  Description of Artificial Sequence: Synthetic polynucleotide
gaggtggagttttagtcagggttttagagctagaaatagcaagttaaaataaggctagtccgttatcaacttgaaaaagtggcaccgagtcggtgctttttttcc

SEQ ID NO: 605 - DNA, 105 bp, Artificial Sequence
  Description of Artificial Sequence: Synthetic polynucleotide
aaacggcatcataaagaaaagttttagagctagaaatagcaagttaaaataaggctagtccgttatcaacttgaaaaagtggcaccgagtcggtgctttttttcc

SEQ ID NO: 606 - DNA, 19 bp, Artificial Sequence
  Description of Artificial Sequence: Synthetic oligonucleotide
tgtactctctgaggtgctc

SEQ ID NO: 607 - DNA, 19 bp, Artificial Sequence
  Description of Artificial Sequence: Synthetic oligonucleotide
acgcagataagaaccagtt

SEQ ID NO: 608 - DNA, 19 bp, Artificial Sequence
  Description of Artificial Sequence: Synthetic oligonucleotide
catcaagtcagccatcagc

SEQ ID NO: 609 - DNA, 19 bp, Artificial Sequence
  Description of Artificial Sequence: Synthetic oligonucleotide
gagtcaccctcctggaaac

SEQ ID NO: 610 - DNA, 19 bp, Artificial Sequence
  Description of Artificial Sequence: Synthetic oligonucleotide
cctgggctccggggcgttt

SEQ ID NO: 611 - DNA, 19 bp, Artificial Sequence
  Description of Artificial Sequence: Synthetic oligonucleotide
ggcccctgcggccaccccg

SEQ ID NO: 612 - DNA, 19 bp, Artificial Sequence
  Description of Artificial Sequence: Synthetic oligonucleotide
ctccctccctgcccggtag

SEQ ID NO: 613 - DNA, 19 bp, Artificial Sequence
  Description of Artificial Sequence: Synthetic oligonucleotide
aggtttggaaagggcgtgc

SEQ ID NO: 614 - DNA, 20 bp, Artificial Sequence
  Description of Artificial Sequence: Synthetic oligonucleotide
actccactgcactccagtct

SEQ ID NO: 615 - DNA, 20 bp, Artificial Sequence
  Description of Artificial Sequence: Synthetic oligonucleotide
tctgtgggggacctgcactg

SEQ ID NO: 616 - DNA, 20 bp, Artificial Sequence
  Description of Artificial Sequence: Synthetic oligonucleotide
ggggcgccagttgtgtctcc

SEQ ID NO: 617 - DNA, 20 bp, Artificial Sequence
  Description of Artificial Sequence: Synthetic oligonucleotide
acaccattgccaccaccatt

SEQ ID NO: 618 - DNA, 20 bp, Artificial Sequence
  Description of Artificial Sequence: Synthetic primer
caatgaccccttcattgacc

SEQ ID NO: 619 - DNA, 20 bp, Artificial Sequence
  Description of Artificial Sequence: Synthetic primer
ttgattttggagggatctcg

SEQ ID NO: 620 - DNA, 20 bp, Artificial Sequence
  Description of Artificial Sequence: Synthetic primer
ggaatccatggagggaagat

SEQ ID NO: 621 - DNA, 20 bp, Artificial Sequence
  Description of Artificial Sequence: Synthetic primer
tgttctcgctcaggtcagtg

SEQ ID NO: 622 - DNA, 20 bp, Artificial Sequence
  Description of Artificial Sequence: Synthetic primer
ctctctgctcctttgccaca

SEQ ID NO: 623 - DNA, 20 bp, Artificial Sequence
  Description of Artificial Sequence: Synthetic primer
gtgctcttcgggtttcagga

SEQ ID NO: 624 - DNA, 30 bp, Artificial Sequence
  Description of Artificial Sequence: Synthetic primer
cgaaagagaaagcgaaccagtatcgagaac

SEQ ID NO: 625 - DNA, 27 bp, Artificial Sequence
  Description of Artificial Sequence: Synthetic primer
cgttgtgcatagtcgctgcttgatcgc

SEQ ID NO: 626 - DNA, 25 bp, Artificial Sequence
  Description of Artificial Sequence: Synthetic primer
gagtttggctcaaattgttactctt

SEQ ID NO: 627 - DNA, 25 bp, Artificial Sequence
  Description of Artificial Sequence: Synthetic primer
gggaaatggtctaggagagtaaagt

SEQ ID NO: 628 - DNA, 23 bp, Artificial Sequence
  Description of Artificial Sequence: Synthetic oligonucleotide
gattggctttgatttccctaggg

SEQ ID NO: 629 - DNA, 23 bp, Artificial Sequence
  Description of Artificial Sequence: Synthetic oligonucleotide
gcctactcagactgttactctgg

SEQ ID NO: 630 - DNA, 23 bp, Artificial Sequence
  Description of Artificial Sequence: Synthetic oligonucleotide
gcagttgcctaagaactggtggg

SEQ ID NO: 631 - DNA, 23 bp, Artificial Sequence
  Description of Artificial Sequence: Synthetic oligonucleotide
ggggctccaccctcacgagtggg

SEQ ID NO: 632 - DNA, 23 bp, Artificial Sequence
  Description of Artificial Sequence: Synthetic oligonucleotide
gccttctttatcccctatcgagg

SEQ ID NO: 633 - DNA, 48 bp, Artificial Sequence
  Description of Artificial Sequence: Synthetic oligonucleotide
  CDS (1)..(45)
gaaggaccatttgacgttcagctcctactcagactgttactctggtga

SEQ ID NO: 634 - protein, 15 aa, Artificial Sequence
  Description of Artificial Sequence: Synthetic peptide
EGPFDVQLLLRLLLW

SEQ ID NO: 635 - DNA, 46 bp, Artificial Sequence
  Description of Artificial Sequence: Synthetic oligonucleotide
  CDS (1)..(42)
gaaggaccatttgacgttcagctcctactcagactgtctctggtga

SEQ ID NO: 636 - protein, 14 aa, Artificial Sequence
  Description of Artificial Sequence: Synthetic peptide
EGPFDVQLLLRLSL

SEQ ID NO: 637 - RNA, 20 nt, Artificial Sequence
  Description of Artificial Sequence: Synthetic oligonucleotide
gccuacucagacuguuacuc

SEQ ID NO: 638 - DNA, 19 bp, Artificial Sequence
  Description of Artificial Sequence: Synthetic oligonucleotide
cccaccagttcttaggcaa

SEQ ID NO: 639 - DNA, 20 bp, Artificial Sequence
  Description of Artificial Sequence: Synthetic oligonucleotide
cccaccagttcttaggcaac

SEQ ID NO: 640 - DNA, 20 bp, Artificial Sequence
  Description of Artificial Sequence: Synthetic oligonucleotide
tttgatttccagttcttagg

SEQ ID NO: 641 - DNA, 19 bp, Artificial Sequence
  Description of Artificial Sequence: Synthetic oligonucleotide
attaccatagagttcttag

SEQ ID NO: 642 - DNA, 19 bp, Artificial Sequence
  Description of Artificial Sequence: Synthetic oligonucleotide
gtggataaaggcaacaatg

SEQ ID NO: 643 - DNA, 16 bp, Artificial Sequence
  Description of Artificial Sequence: Synthetic oligonucleotide
cctcgataggggataa

SEQ ID NO: 644 - DNA, 23 bp, Artificial Sequence
  Description of Artificial Sequence: Synthetic oligonucleotide
accaaacccacttaggggataaa

SEQ ID NO: 645 - DNA, 21 bp, Artificial Sequence
  Description of Artificial Sequence: Synthetic oligonucleotide
ggtatcttaaggacctccaag

SEQ ID NO: 646 - DNA, 47 bp, Artificial Sequence
  Description of Artificial Sequence: Synthetic oligonucleotide
taggaagtaaattaatttgaagcttgccaattaatccaaatcttacc

SEQ ID NO: 647 - DNA, 83 bp, Artificial Sequence
  Description of Artificial Sequence: Synthetic primer
tttcctttttgcaaaacccaaaatattttagctcctactcagactgttagagtaggaggagaaggagggctgtggctcttgtg

SEQ ID NO: 648 - DNA, 83 bp, Artificial Sequence
  Description of Artificial Sequence: Synthetic primer
  modified_base (20)..(20): a, c, t, g, unknown or other
  modified_base (31)..(31): a, c, t, g, unknown or other
  modified_base (69)..(69): a, c, t, g, unknown or other
aaaacccccaaaccctcccnctttttcctcntactctaacagtgtgagtaggaggccacacttagctgnggctctagtaagtc

SEQ ID NO: 649 - DNA, 94 bp, Artificial Sequence
  Description of Artificial Sequence: Synthetic primer
  modified_base (50)..(50): a, c, t, g, unknown or other
cttcttttttcctttttgcaaaaacccaaaatattttagctcctactcanaccgttttcggggggtattttgtatttggatgaaacacttgatg

SEQ ID NO: 650 - DNA, 93 bp, Artificial Sequence
  Description of Artificial Sequence: Synthetic primer
tcttcttttttccttcccgcaaaaacccaaaatattttcgctcctactcaggacctggtcgtggggtattttgtatttggatgaaacacttga

SEQ ID NO: 651 - DNA, 104 bp, Artificial Sequence
  Description of Artificial Sequence: Synthetic primer
  modified_base (21)..(22): a, c, t, g, unknown or other
tcaaggaagatggcatttctnntttggagatggcagtttccttagtaaccacaggttgtgtcaccatggccagtaagaaggatgccacacttgtgtgtgtcgct

SEQ ID NO: 652 - DNA, 86 bp, Artificial Sequence
  Description of Artificial Sequence: Synthetic primer
  modified_base (35)..(36): a, c, t, g, unknown or other
  modified_base (42)..(44): a, c, t, g, unknown or other
ttggagatagcagtttccttggtaagtacaggttnntcaccnnnacagtgtgagtaggaggccacacttagctgtggctctagtaa

SEQ ID NO: 653 - DNA, 71 bp, Artificial Sequence
  Description of Artificial Sequence: Synthetic primer
  modified_base (54)..(54): a, c, t, g, unknown or other
  modified_base (61)..(63): a, c, t, g, unknown or other
  modified_base (69)..(69): a, c, t, g, unknown or other
tttctagtttggagatggcagtttccttagtaaccacaggttgtgtcaccaggnctcgagnnntggttntg

SEQ ID NO: 654 - DNA, 87 bp, Artificial Sequence
  Description of Artificial Sequence: Synthetic primer
cagttgccatagtcttcactaaccgcgtcaccagagctcaggacctggtcgtggggtattttgtatttggatgaaacacttgatggt

SEQ ID NO: 655 - DNA, 92 bp, Artificial Sequence
  Description of Artificial Sequence: Synthetic primer
  modified_base (52)..(52): a, c, t, g, unknown or other
  modified_base (59)..(59): a, c, t, g, unknown or other
  modified_base (78)..(78): a, c, t, g, unknown or other
tattgtatcttggtttttcttcactgctggccagtttactaacaatctgaantaagccnattaatccaaatcttaccngacgaaaaatcaaa

SEQ ID NO: 656 - DNA, 89 bp, Artificial Sequence
  Description of Artificial Sequence: Synthetic primer
  modified_base (6)..(6): a, c, t, g, unknown or other
  modified_base (10)..(10): a, c, t, g, unknown or other
  modified_base (19)..(19): a, c, t, g, unknown or other
  modified_base (30)..(30): a, c, t, g, unknown or other
  modified_base (57)..(57): a, c, t, g, unknown or other
atggtntttngtcattgcnggccagttttntaacaatgtgatcaatgccaattaatncaaatcttaccagaggaaaaatcaagccacag

SEQ ID NO: 657 - DNA, 94 bp, Artificial Sequence
  Description of Artificial Sequence: Synthetic primer
  modified_base (93)..(94): a, c, t, g, unknown or other
aataaaaagaaaaaaatatgataaactgctcccagtataaaatacagagctaagacaagaacgtttcattggctgttaaaagtcggaaatcgnn

SEQ ID NO: 658 - DNA, 94 bp, Artificial Sequence
  Description of Artificial Sequence: Synthetic primer
ttctgatttaaaattcccttgaataggaagtaaattaatttgaagcttgccaattaatccaaatcttaccagaggaaaaatcaagccacagata

SEQ ID NO: 659 - DNA, 90 bp, Artificial Sequence
  Description of Artificial Sequence: Synthetic primer
caaaacaagatgggataaaatcttctttctgatttaaaattcccttgaataggaagtaaattactagagctgttcaaggcctgaactcta

SEQ ID NO: 660 - DNA, 96 bp, Artificial Sequence
  Description of Artificial Sequence: Synthetic primer
  modified_base (49)..(49): a, c, t, g, unknown or other
  modified_base (51)..(52): a, c, t, g, unknown or other
  modified_base (54)..(54): a, c, t, g, unknown or other
ctgatttaaaattcccttgaataggaagtaaattactagagctgttcangnncngaactctaggctagcatttccagcccaaaacaaacacagttc

SEQ ID NO: 661 - DNA, 26 bp, Artificial Sequence
  Description of Artificial Sequence: Synthetic oligonucleotide
  modified_base (8)..(26): a, c, t, g, unknown or other
ttgtttgnnnnnnnnnnnnnnnnnnn

SEQ ID NO: 662 - DNA, 24 bp, Artificial Sequence
  Description of Artificial Sequence: Synthetic oligonucleotide
  modified_base (6)..(24): a, c, t, g, unknown or other
caccgnnnnnnnnnnnnnnnnnnn

SEQ ID NO: 663 - DNA, 24 bp, Artificial Sequence
  Description of Artificial Sequence: Synthetic oligonucleotide
  modified_base (6)..(24): a, c, t, g, unknown or other
tcccannnnnnnnnnnnnnnnnnn

SEQ ID NO: 664 - DNA, 24 bp, Artificial Sequence
  Description of Artificial Sequence: Synthetic oligonucleotide
  modified_base (6)..(24): a, c, t, g, unknown or other
cctcgnnnnnnnnnnnnnnnnnnn

SEQ ID NO: 665 - DNA, 26 bp, Artificial Sequence
  Description of Artificial Sequence: Synthetic oligonucleotide
  modified_base (5)..(23): a, c, t, g, unknown or other
aaacnnnnnnnnnnnnnnnnnnncaa

SEQ ID NO: 666 - DNA, 24 bp, Artificial Sequence
  Description of Artificial Sequence: Synthetic oligonucleotide
  modified_base (5)..(23): a, c, t, g, unknown or other
aaacnnnnnnnnnnnnnnnnnnnc

SEQ ID NO: 667 - DNA, 24 bp, Artificial Sequence
  Description of Artificial Sequence: Synthetic oligonucleotide
  modified_base (5)..(23): a, c, t, g, unknown or other
aaacnnnnnnnnnnnnnnnnnnnt

SEQ ID NO: 668 - DNA, 24 bp, Artificial Sequence
  Description of Artificial Sequence: Synthetic oligonucleotide
  modified_base (5)..(23): a, c, t, g, unknown or other
aaacnnnnnnnnnnnnnnnnnnnc

SEQ ID NO: 669 - DNA, 26 bp, Artificial Sequence
  Description of Artificial Sequence: Synthetic oligonucleotide
ttgtttgtcttcgagaagacctgttt

SEQ ID NO: 670 - DNA, 26 bp, Artificial Sequence
  Description of Artificial Sequence: Synthetic oligonucleotide
caccgggtcttcgagaagacctgttt

SEQ ID NO: 671 - DNA, 26 bp, Artificial Sequence
  Description of Artificial Sequence: Synthetic oligonucleotide
tcccaggtcttcgagaagacctgttt

SEQ ID NO: 672 - DNA, 26 bp, Artificial Sequence
  Description of Artificial Sequence: Synthetic oligonucleotide
cctcgggtcttcgagaagacctgttt

SEQ ID NO: 673 - DNA, 25 bp, Artificial Sequence
  Description of Artificial Sequence: Synthetic oligonucleotide
ggcctaccgctaaggctagcctagt

SEQ ID NO: 674 - protein, 1411 aa, Artificial Sequence
  Description of Artificial Sequence: Synthetic polypeptide
MDYKDHDGDYKDHDIDYKDDDDKMAPKKKRKVGRGMDKKYSIGLAIGTNSVGWAVITDEYKVPSKKFKVLGNTDRHSIKKNLIGALLFDSGETAEATRLKRTARRRYTRRKNRICYLQEIFSNEMAKVDDSFFHRLEESFLVEEDKKHERHPIFGNIVDEVAYHEKYPTIYHLRKKLVDSTDKADLRLIYLALAHMIKFRGHFLIEGDLNPDNSDVDKLFIQLVQTYNQLFEENPINASGVDAKAILSARLSKSRRLENLIAQLPGEKKNGLFGNLIALSLGLTPNFKSNFDLAEDAKLQLSKDTYDDDLDNLLAQIGDQYADLFLAAKNLSDAILLSDILRVNTEITKAPLSASMIKRYDEHHQDLTLLKALVRQQLPEKYKEIFFDQSKNGYAGYIDGGASQEEFYKFIKPILEKMDGTEELLVKLNREDLLRKQRTFDNGSIPHQIHLGELHAILRRQEDFYPFLKDNREKIEKILTFRIPYYVGPLARGNSRFAWMTRKSEETITPWNFEEVVDKGASAQSFIERMTNFDKNLPNEKVLPKHSLLYEYFTVYNELTKVKYVTEGMRKPAFLSGEQKKAIVDLLFKTNRKVTVKQLKEDYFKKIECFDSVEISGVEDRFNASLGTYHDLLKIIKDKDFLDNEENEDILEDIVLTLTLFEDREMIEERLKTYAHLFDDKVMKQLKRRRYTGWGRLSRKLINGIRDKQSGKTILDFLKSDGFANRNFMQLIHDDSLTFKEDIQKAQVSGQGDSLHEHIANLAGSPAIKKGILQTVKVVDELVKVMGRHKPENIVIEMARENQTTQKGQKNSRERMKRIEEGIKELGSQILKEHPVENTQLQNEKLYLYYLQNGRDMYVDQELDINRLSDYDVDHIVPQSFLKDDSIDNKVLTRSDKNRGKSDNVPSEEVVKKMKNYWRQLLNAKLITQRKFDNLTKAERGGLSELDKAGFIKRQLVETRQITKHVAQILDSRMNTKYDENDKLIREVKVITLKSKLVSDFRKDFQFYKVREINNYHHAHDAYLNAVVGTALIKKYPKLESEFVYGDYKVYDVRKMIAKSEQEIGKATAKYFFYSNIMNFFKTEITLANGEIRKRPLIETNGETGEIVWDKGRDFATVRKVLSMPQVNIVKKTEVQTGGFSKESILPKRNSDKLIARKKDWDPKKYGGFDSPTVAYSVLVVAKVEKGKSKKLKSVKELLGITIMERSSFEKNPIDFLEAKGYKEVKKDLIIKLPKYSLFELENGRKRMLASAGELQKGNELALPSKYVNFLYLASHYEKLKGSPEDNEQKQLFVEQHKHYLDEIIEQISEFSKRVILADANLDKVLSAYNKHRDKPIREQAENIIHLFTLTNLGAPAAFKYFDTTIDRKRYTSTKEVLDATLIHQSITGLYETRIDLSQLGGDPKKKRKVG

SEQ ID NO: 675 - protein, 1483 aa, Artificial Sequence; identical to SEQ ID NO: 1
  Description of Artificial Sequence: Synthetic polypeptide

SEQ ID NO: 676 - protein, 2048 aa, Artificial Sequence
  Description of Artificial Sequence: Synthetic polypeptide
MDYKDHDGDYKDHDIDYKDDDDKMAPKKKRKVGRGMDKKYSIGLAIGTNSVGWAVITDEYKVPSKKFKVLGNTDRHSIKKNLIGALLFDSGETAEATRLKRTARRRYTRRKNRICYLQEIFSNEMAKVDDSFFHRLEESFLVEEDKKHERHPIFGNIVDEVAYHEKYPTIYHLRKKLVDSTDKADLRLIYLALAHMIKFRGHFLIEGDLNPDNSDVDKLFIQLVQTYNQLFEENPINASGVDAKAILSARLSKSRRLENLIAQLPGEKKNGLFGNLIALSLGLTPNFKSNFDLAEDAKLQLSKDTYDDDLDNLLAQIGDQYADLFLAAKNLSDAILLSDILRVNTEITKAPLSASMIKRYDEHHQDLTLLKALVRQQLPEKYKEIFFDQSKNGYAGYIDGGASQEEFYKFIKPILEKMDGTEELLVKLNREDLLRKQRTFDNGSIPHQIHLGELHAILRRQEDFYPFLKDNREKIEKILTFRIPYYVGPLARGNSRFAWMTRKSEETITPWNFEEVVDKGASAQSFIERMTNFDKNLPNEKVLPKHSLLYEYFTVYNELTKVKYVTEGMRKPAFLSGEQKKAIVDLLFKTNRKVTVKQLKEDYFKKIECFDSVEISGVEDRFNASLGTYHDLLKIIKDKDFLDNEENEDILEDIVLTLTLFEDREMIEERLKTYAHLFDDKVMKQLKRRRYTGWGRLSRKLINGIRDKQSGKTILDFLKSDGFANRNFMQLIHDDSLTFKEDIQKAQVSGQGDSLHEHIANLAGSPAIKKGILQTVKVVDELVKVMGRHKPENIVIEMARENQTTQKGQKNSRERMKRIEEGIKELGSQILKEHPVENTQLQNEKLYLYYLQNGRDMYVDQELDINRLSDYDVDAIVPQSFLKDDSIDNKVLTRSDKNRGKSDNVPSEEVVKKMKNYWRQLLNAKLITQRKFDNLTKAERGGLSELDKAGFIKRQLVETRQITKHVAQILDSRMNTKYDENDKLIREVKVITLKSKLVSDFRKDFQFYKVREINNYHHAHDAYLNAVVGTALIKKYPKLESEFVYGDYKVYDVRKMIAKSEQEIGKATAKYFFYSNIMNFFKTEITLANGEIRKRPLIETNGETGEIVWDKGRDFATVRKVLSMPQVNIVKKTEVQTGGFSKESILPKRNSDKLIARKKDWDPKKYGGFDSPTVAYSVLVVAKVEKGKSKKLKSVKELLGITIMERSSFEKNPIDFLEAKGYKEVKKDLIIKLPKYSLFELENGRKRMLASAGELQKGNELALPSKYVNFLYLASHYEKLKGSPEDNEQKQLFVEQHKHYLDEIIEQISEFSKRVILADANLDKVLSAYNKHRDKPIREQAENIIHLFTLTNLGAPAAFKYFDTTIDRKRYTSTKEVLDATLIHQSITGLYETRIDLSQLGGDPIAGSKASPKKKRKVGRAIFKPEELRQALMPTLEALYRQDPESLPFRQPVDPQLLGIPDYFDIVKSPMDLSTIKRKLDTGQYQEPWQYVDDIWLMFNNAWLYNRKTSRVYKYCSKLSEVFEQEIDPVMQSLGYCCGRKLEFSPQTLCCYGKQLCTIPRDATYYSYQNRYHFCEKCFNEIQGESVSLGDDPSQPQTTINKEQFSKRKNDTLDPELFVECTECGRKMHQICVLHHEIIWPAGFVCDGCLKKSARTRKENKFSAKRLPSTRLGTFLENRVNDFLRRQNHPESGEVTVRVVHASDKTVEVKPGMKARFVDSGEMAESFPYRTKALFAFEEIDGVDLCFFGMHVQEYGSDCPPPNQRRVYISYLDSVHFFRPKCLRTAVYHEILIGYLEYVKKLGYTTGHIWACPPSEGDDYIFHCHPPDQKIPKPKRLQEWYKKMLDKAVSERIVHDYKDIFKQATEDRLTSAKELPYFEGDFWPNVLEESIKELEQEEEERKREENTSNESTDVTKGDSKNAKKKNNKKTSKNKSSLSRGNKKKPGMPNVSNDLSQKLYATMEKHKEVFFVIRLIAGPAANSLPPIVDPDPLIPCDLMDGRDAFLTLARDKHLEFSSLRRAQWSTMCMLVELHTQSQDYPYDVPDYAS

SEQ ID NO: 677 - DNA, 23 bp, Artificial Sequence
  Description of Artificial Sequence: Dystrophin gene reference sequence
  modified_base (1)..(21): a, c, t, g, unknown or other
nnnnnnnnnnnnnnnnnnnnngg

SEQ ID NO: 678 - DNA, 23 bp, Artificial Sequence
  Description of Artificial Sequence: Dystrophin gene reference sequence
  modified_base (2)..(21): a, c, t, g, unknown or other
gnnnnnnnnnnnnnnnnnnnngg

SEQ ID NO: 679 - DNA, 20 bp, Artificial Sequence
  Description of Artificial Sequence: Synthetic oligonucleotide
gtgtagagtaagtcagccta

SEQ ID NO: 680 - DNA, 20 bp, Artificial Sequence
  Description of Artificial Sequence: Synthetic oligonucleotide
gttggacagaacttaccgac

SEQ ID NO: 681 - DNA, 20 bp, Artificial Sequence
  Description of Artificial Sequence: Synthetic oligonucleotide
gtttgcttcgctataaaacg

SEQ ID NO: 682 - DNA, 20 bp, Artificial Sequence
  Description of Artificial Sequence: Synthetic oligonucleotide
gtctgaggatggggccgcaa

SEQ ID NO: 683 - DNA, 20 bp, Artificial Sequence
  Description of Artificial Sequence: Synthetic oligonucleotide
ggatctgtcaaatcgcctgc

SEQ ID NO: 684 - DNA, 20 bp, Artificial Sequence
  Description of Artificial Sequence: Synthetic oligonucleotide
gccaggatggcattgggcag

SEQ ID NO: 685 - DNA, 20 bp, Artificial Sequence
  Description of Artificial Sequence: Synthetic oligonucleotide
gctgaatctgcggtggcagg

SEQ ID NO: 686 - DNA, 20 bp, Artificial Sequence
  Description of Artificial Sequence: Synthetic oligonucleotide
gttcttttgttcttctagcc

SEQ ID NO: 687 - DNA, 20 bp, Artificial Sequence
  Description of Artificial Sequence: Synthetic oligonucleotide
ggaaaagcttgagcaagtca

SEQ ID NO: 688 - DNA, 20 bp, Artificial Sequence
  Description of Artificial Sequence: Synthetic oligonucleotide
ggaagagttgcccctgcgcc

SEQ ID NO: 689 - DNA, 20 bp, Artificial Sequence
  Description of Artificial Sequence: Synthetic oligonucleotide
gacaaatctccagtggataa

SEQ ID NO: 690 - DNA, 20 bp, Artificial Sequence
  Description of Artificial Sequence: Synthetic oligonucleotide
gtgtttctcaggtaaagctc

SEQ ID NO: 691 - DNA, 20 bp, Artificial Sequence
  Description of Artificial Sequence: Synthetic oligonucleotide
ggaaggaccatttgacgtta

SEQ ID NO: 692 - DNA, 20 bp, Artificial Sequence
  Description of Artificial Sequence: Synthetic oligonucleotide
gaactgctatttcagtttcc

SEQ ID NO: 693 - DNA, 20 bp, Artificial Sequence
  Description of Artificial Sequence: Synthetic oligonucleotide
gccagccactcagccagtga

SEQ ID NO: 694 - DNA, 20 bp, Artificial Sequence
  Description of Artificial Sequence: Synthetic oligonucleotide
ggtatgcttttctgttaaag

SEQ ID NO: 695 - DNA, 20 bp, Artificial Sequence
  Description of Artificial Sequence: Synthetic oligonucleotide
gctcctggactgaccactat

SEQ ID NO: 696 - DNA, 23 bp, Artificial Sequence
  Description of Artificial Sequence: Synthetic oligonucleotide
ggaacagaggcgtccccagttgg

SEQ ID NO: 697 - DNA, 20 bp, Artificial Sequence
  Description of Artificial Sequence: Synthetic oligonucleotide
ggaggctagaacaatcatta

SEQ ID NO: 698 - DNA, 20 bp, Artificial Sequence
  Description of Artificial Sequence: Synthetic oligonucleotide
gacaagaacaccttcagaac

SEQ ID NO: 699 - DNA, 20 bp, Artificial Sequence
  Description of Artificial Sequence: Synthetic oligonucleotide
gggtttctgtgattttcttt

SEQ ID NO: 700 - DNA, 20 bp, Artificial Sequence
  Description of Artificial Sequence: Synthetic oligonucleotide
gggccaaagacctccgccag

SEQ ID NO: 701 - DNA, 20 bp, Artificial Sequence
  Description of Artificial Sequence: Synthetic oligonucleotide
gttggagaagcattcataaa

SEQ ID NO: 702 - DNA, 20 bp, Artificial Sequence
  Description of Artificial Sequence: Synthetic oligonucleotide
gtcgctcactcaccctgcaa

SEQ ID NO: 703 - DNA, 20 bp, Artificial Sequence
  Description of Artificial Sequence: Synthetic oligonucleotide
gaaaagagctgatgaaacaa

SEQ ID NO: 704 - DNA, 20 bp, Artificial Sequence
  Description of Artificial Sequence: Synthetic oligonucleotide
gtacacttttcaaaatgctt

SEQ ID NO: 705 - DNA, 20 bp, Artificial Sequence
  Description of Artificial Sequence: Synthetic oligonucleotide
ggagatgatcatcaagcaga

SEQ ID NO: 706 - DNA, 20 bp, Artificial Sequence
  Description of Artificial Sequence: Synthetic oligonucleotide
gctttgaaagagcaataaaa

SEQ ID NO: 707 - DNA, 20 bp, Artificial Sequence
  Description of Artificial Sequence: Synthetic oligonucleotide
gcacaaaagtcaaatcggaa

SEQ ID NO: 708 - DNA, 20 bp, Artificial Sequence
  Description of Artificial Sequence: Synthetic oligonucleotide
gatttcaatataagattcgg

SEQ ID NO: 709 - DNA, 20 bp, Artificial Sequence
  Description of Artificial Sequence: Synthetic oligonucleotide
gcttaagcaatcccgaactc

SEQ ID NO: 710 - DNA, 20 bp, Artificial Sequence
  Description of Artificial Sequence: Synthetic oligonucleotide
gaggccaaacctcggcttac

SEQ ID NO: 711 - DNA, 20 bp, Artificial Sequence
  Description of Artificial Sequence: Synthetic oligonucleotide
gttcgaaaatttcaggtaag

SEQ ID NO: 712 - DNA, 20 bp, Artificial Sequence
  Description of Artificial Sequence: Synthetic oligonucleotide
ggcagaacaggagataacag

SEQ ID NO: 713 - DNA, 20 bp, Artificial Sequence
  Description of Artificial Sequence: Synthetic oligonucleotide
ggcggccctcgcccttctct

SEQ ID NO: 714 - DNA, 20 bp, Artificial Sequence
  Description of Artificial Sequence: Synthetic oligonucleotide
gtagtgatcgtggatacgag

SEQ ID NO: 715 - DNA, 20 bp, Artificial Sequence
  Description of Artificial Sequence: Synthetic oligonucleotide
gtacagccctcggtgtatat

SEQ ID NO: 716 - DNA, 20 bp, Artificial Sequence
  Description of Artificial Sequence: Synthetic oligonucleotide
gggaaggaattaagcccgaa

SEQ ID NO: 717 - DNA, 20 bp, Artificial Sequence
  Description of Artificial Sequence: Synthetic oligonucleotide
gggaacagctttcgtagttg

SEQ ID NO: 718 - DNA, 20 bp, Artificial Sequence
  Description of Artificial Sequence: Synthetic oligonucleotide
gataaagtccagtgtcgatc

SEQ ID NO: 719 - DNA, 20 bp, Artificial Sequence
  Description of Artificial Sequence: Synthetic oligonucleotide
gaaaaccagagcttcggtca

SEQ ID NO: 720 - DNA, 31 bp, Artificial Sequence
  Description of Artificial Sequence: Synthetic oligonucleotide
ggagtcttctgggcaggcttaaaggctaacc

SEQ ID NO: 721 - DNA, 31 bp, Artificial Sequence
  Description of Artificial Sequence: Synthetic oligonucleotide
gtcgggtgagcatgtctttaatctacctcga

SEQ ID NO: 722 - DNA, 20 bp, Artificial Sequence
  Description of Artificial Sequence: Synthetic oligonucleotide
ggtgtcaccagagtaacagt

SEQ ID NO: 723 - DNA, 20 bp, Artificial Sequence
  Description of Artificial Sequence: Synthetic oligonucleotide
gtgatcatcaagcagaaggt

SEQ ID NO: 724 - DNA, 21 bp, Artificial Sequence
  Description of Artificial Sequence: Synthetic oligonucleotide
gaacttcgaaaatttcaggta

SEQ ID NO: 725 - DNA, 21 bp, Artificial Sequence
  Description of Artificial Sequence: Synthetic oligonucleotide
ggaaactcatcaaatatgcgt

SEQ ID NO: 726 - DNA, 21 bp, Artificial Sequence
  Description of Artificial Sequence: Synthetic oligonucleotide
gtcatttacactaacacgcat

SEQ ID NO: 727 - DNA, 21 bp, Artificial Sequence
  Description of Artificial Sequence: Synthetic oligonucleotide
ggaatgaaactcatcaaatat

SEQ ID NO: 728 - DNA, 21 bp, Artificial Sequence
  Description of Artificial Sequence: Synthetic oligonucleotide
gtcatcaatatctttgaagga

SEQ ID NO: 729 - DNA, 21 bp, Artificial Sequence
  Description of Artificial Sequence: Synthetic oligonucleotide
gtgttttcataggaaaaatag

SEQ ID NO: 730 - DNA, 21 bp, Artificial Sequence
  Description of Artificial Sequence: Synthetic oligonucleotide
gaattggaaaatgtgatggga

SEQ ID NO: 731 - DNA, 21 bp, Artificial Sequence
  Description of Artificial Sequence: Synthetic oligonucleotide
gatgatcatcaagcagaaggt

SEQ ID NO: 732 - DNA, 21 bp, Artificial Sequence
  Description of Artificial Sequence: Synthetic oligonucleotide
gagatgatcatcaagcagaag

SEQ ID NO: 733 - DNA, 21 bp, Artificial Sequence
  Description of Artificial Sequence: Synthetic oligonucleotide
gcattttttctcataccttct

SEQ ID NO: 734 - DNA, 21 bp, Artificial Sequence
  Description of Artificial Sequence: Synthetic oligonucleotide
gtcctactcagactgttactc

SEQ ID NO: 735 - DNA, 21 bp, Artificial Sequence
  Description of Artificial Sequence: Synthetic oligonucleotide
gacaggttgtgtcaccagagt

SEQ ID NO: 736 - DNA, 21 bp, Artificial Sequence
  Description of Artificial Sequence: Synthetic oligonucleotide
gttatcattttttctcatacc

SEQ ID NO: 737 - DNA, 21 bp, Artificial Sequence
  Description of Artificial Sequence: Synthetic oligonucleotide
gttgcctaagaactggtggga

SEQ ID NO: 738 - DNA, 21 bp, Artificial Sequence
  Description of Artificial Sequence: Synthetic oligonucleotide
gaaacagttgcctaagaactg

SEQ ID NO: 739 - DNA, 21 bp, Artificial Sequence
  Description of Artificial Sequence: Synthetic oligonucleotide
gtttcccaccagttcttaggc

SEQ ID NO: 740 - DNA, 21 bp, Artificial Sequence
  Description of Artificial Sequence: Synthetic oligonucleotide
gtggctttgatttccctaggg

SEQ ID NO: 741 - DNA, 21 bp, Artificial Sequence
  Description of Artificial Sequence: Synthetic oligonucleotide
gtagggaaatcaaagccaatg

SEQ ID NO: 742 - DNA, 21 bp, Artificial Sequence
  Description of Artificial Sequence: Synthetic oligonucleotide
ggaccctagggaaatcaaagc

SEQ ID NO: 743 - DNA, 21 bp, Artificial Sequence
  Description of Artificial Sequence: Synthetic oligonucleotide
gtgagggctccaccctcacga

SEQ ID NO: 744 - DNA, 21 bp, Artificial Sequence
  Description of Artificial Sequence: Synthetic oligonucleotide
gaaggattgagggctccaccc

SEQ ID NO: 745 - DNA, 21 bp, Artificial Sequence
  Description of Artificial Sequence: Synthetic oligonucleotide
ggctccaccctcacgagtggg

SEQ ID NO: 746 - DNA, 21 bp, Artificial Sequence
  Description of Artificial Sequence: Synthetic oligonucleotide
gtatcccctatcgaggaaacc

SEQ ID NO: 747 - DNA, 21 bp, Artificial Sequence
  Description of Artificial Sequence: Synthetic oligonucleotide
ggataaagaaggcctatttca

SEQ ID NO: 748 - DNA, 21 bp, Artificial Sequence
  Description of Artificial Sequence: Synthetic oligonucleotide
gaggccttctttatcccctat

SEQ ID NO: 749 - DNA, 21 bp, Artificial Sequence
  Description of Artificial Sequence: Synthetic oligonucleotide
gtgagggctccaccctcacga

SEQ ID NO: 750 - DNA, 21 bp, Artificial Sequence
  Description of Artificial Sequence: Synthetic oligonucleotide
ggataaagaaggcctatttca